European Patent Application EP 4 653 458 A1, published November 26, 2025. Title: HUMAN ANTI-HUMAN PLA2R ANTIBODY STANDARD AND USE THEREOF. Applicant: CHENGDU DI'AO PHARMACEUTICAL GROUP CO., LTD. The sequence listing filed with the application follows.

SEQUENCE LISTING (445 sequences)

SEQ ID NO: 1 - protein, 9 aa, synthetic construct
GGSISSGGY

SEQ ID NO: 2 - protein, 7 aa, synthetic construct
GFTFSRY

SEQ ID NO: 3 - protein, 7 aa, synthetic construct
GGTFSSY

SEQ ID NO: 4 - protein, 7 aa, synthetic construct
GFTFSSY

SEQ ID NO: 5 - protein, 7 aa, synthetic construct
GYTFTDY

SEQ ID NO: 6 - protein, 7 aa, synthetic construct
GGTFSSY

SEQ ID NO: 7 - protein, 7 aa, synthetic construct
GGTFSSY

SEQ ID NO: 8 - protein, 7 aa, synthetic construct
GFTFSSY

SEQ ID NO: 9 - protein, 9 aa, synthetic construct
GGSISSGGY

SEQ ID NO: 10 - protein, 9 aa, synthetic construct
GGSISSGGY

SEQ ID NO: 11 - protein, 7 aa, synthetic construct
GGTFSSY

SEQ ID NO: 12 - protein, 7 aa, synthetic construct
GFTFSNY

SEQ ID NO: 13 - protein, 7 aa, synthetic construct
GFTFSSY

SEQ ID NO: 14 - protein, 9 aa, synthetic construct
GGSISSGGY

SEQ ID NO: 15 - protein, 7 aa, synthetic construct
GFTFSSY

SEQ ID NO: 16 - protein, 7 aa, synthetic construct
GFTFSSY

SEQ ID NO: 17 - protein, 7 aa, synthetic construct
GYTFTSY

SEQ ID NO: 18 - protein, 7 aa, synthetic construct
GFTFSSY

SEQ ID NO: 19 - protein, 7 aa, synthetic construct
GDSISNY

SEQ ID NO: 20 - protein, 7 aa, synthetic construct
GFTFSSY

SEQ ID NO: 21 - protein, 7 aa, synthetic construct
GDTFSSF

SEQ ID NO: 22 - protein, 7 aa, synthetic construct
GYTFTSY

SEQ ID NO: 23 - protein, 7 aa, synthetic construct
GFTFSSY

SEQ ID NO: 24 - protein, 8 aa, synthetic construct
GGSISSSN

SEQ ID NO: 25 - protein, 7 aa, synthetic construct
GFTFSSY

SEQ ID NO: 26 - protein, 7 aa, synthetic construct
GGTFSSY

SEQ ID NO: 27 - protein, 7 aa, synthetic construct
GLIFKNY

SEQ ID NO: 28 - protein, 7 aa, synthetic construct
GFTFSSY

SEQ ID NO: 29 - protein, 7 aa, synthetic construct
GFTFSGY

SEQ ID NO: 30 - protein, 7 aa, synthetic construct
GFTFSSY

SEQ ID NO: 31 - protein, 9 aa, synthetic construct
GGSISSGGY

SEQ ID NO: 32 - protein, 9 aa, synthetic construct
GGSISSGGY

SEQ ID NO: 33 - protein, 9 aa, synthetic construct
GGSISSGGY

SEQ ID NO: 34 - protein, 7 aa, synthetic construct
GFTFSSY

SEQ ID NO: 35 - protein, 9 aa, synthetic construct
GGSISSGGY

SEQ ID NO: 36 - protein, 5 aa, synthetic construct
YYSGS

SEQ ID NO: 37 - protein, 6 aa, synthetic construct
SYDGSN

SEQ ID NO: 38 - protein, 6 aa, synthetic construct
IPIFGT

SEQ ID NO: 39 - protein, 6 aa, synthetic construct
SSGSSY

SEQ ID NO: 40 - protein, 6 aa, synthetic construct
DPETGG

SEQ ID NO: 41 - protein, 6 aa, synthetic construct
IPIFGT

SEQ ID NO: 42 - protein, 6 aa, synthetic construct
IPIFGT

SEQ ID NO: 43 - protein, 6 aa, synthetic construct
SGSGGS

SEQ ID NO: 44 - protein, 5 aa, synthetic construct
YYSGS

SEQ ID NO: 45 - protein, 5 aa, synthetic construct
YYSGS

SEQ ID NO: 46 - protein, 6 aa, synthetic construct
IPILGI

SEQ ID NO: 47 - protein, 6 aa, synthetic construct
SYDGSK

SEQ ID NO: 48 - protein, 6 aa, synthetic construct
SYDGSN

SEQ ID NO: 49 - protein, 5 aa, synthetic construct
YYSGS

SEQ ID NO: 50 - protein, 6 aa, synthetic construct
SNDGSN

SEQ ID NO: 51 - protein, 6 aa, synthetic construct
SGSGGS

SEQ ID NO: 52 - protein, 6 aa, synthetic construct
NAGNGN

SEQ ID NO: 53 - protein, 6 aa, synthetic construct
SGSGGS

SEQ ID NO: 54 - protein, 5 aa, synthetic construct
HYSGT

SEQ ID NO: 55 - protein, 6 aa, synthetic construct
SSSSSY

SEQ ID NO: 56 - protein, 6 aa, synthetic construct
IPLFTT

SEQ ID NO: 57 - protein, 6 aa, synthetic construct
NPSGGS

SEQ ID NO: 58 - protein, 6 aa, synthetic construct
SYDGSN

SEQ ID NO: 59 - protein, 5 aa, synthetic construct
YHSGS

SEQ ID NO: 60 - protein, 6 aa, synthetic construct
SGSGGR

SEQ ID NO: 61 - protein, 6 aa, synthetic construct
IPILGI

SEQ ID NO: 62 - protein, 6 aa, synthetic construct
SGNSNY

SEQ ID NO: 63 - protein, 6 aa, synthetic construct
SSSSSY

SEQ ID NO: 64 - protein, 6 aa, synthetic construct
SYDGSN

SEQ ID NO: 65 - protein, 6 aa, synthetic construct
SSSSST

SEQ ID NO: 66 - protein, 5 aa, synthetic construct
YYSGS

SEQ ID NO: 67 - protein, 5 aa, synthetic construct
YYSGS

SEQ ID NO: 68 - protein, 5 aa, synthetic construct
YYSGS

SEQ ID NO: 69 - protein, 6 aa, synthetic construct
SGSGDS

SEQ ID NO: 70 - protein, 5 aa, synthetic construct
YYSGS

SEQ ID NO: 71 - protein, 19 aa, synthetic construct
CARQRRANGYSSSWEFDYW

SEQ ID NO: 72 - protein, 10 aa, synthetic construct
CARGGPTPDW

SEQ ID NO: 73 - protein, 17 aa, synthetic construct
CARDSDFWSGYSSMDVW

SEQ ID NO: 74 - protein, 16 aa, synthetic construct
CARDQGASVTGTHTHW

SEQ ID NO: 75 - protein, 14 aa, synthetic construct
CTTTYGNYWYFDVW

SEQ ID NO: 76 - protein, 14 aa, synthetic construct
CAFTSGSYYYFDYW

SEQ ID NO: 77 - protein, 14 aa, synthetic construct
CARGGGGRGMTSDW

SEQ ID NO: 78 - protein, 22 aa, synthetic construct
CAKGTKMATIRLGYYYYGMDVW

SEQ ID NO: 79 - protein, 16 aa, synthetic construct
CARWGRGGSSWRFDIW

SEQ ID NO: 80 - protein, 15 aa, synthetic construct
CARDSRGRSYGMDVW

SEQ ID NO: 81 - protein, 13 aa, synthetic construct
CATGVGMVRGDPW

SEQ ID NO: 82 - protein, 15 aa, synthetic construct
CATGYSSPWYGMDVW

SEQ ID NO: 83 - protein, 13 aa, synthetic construct
CARAAGHGILDYW

SEQ ID NO: 84 - protein, 20 aa, synthetic construct
CARIHHSTAGPYNNWYFDYW

SEQ ID NO: 85 - protein, 14 aa, synthetic construct
CARLLRGPWNFDLW

SEQ ID NO: 86 - protein, 15 aa, synthetic construct
CATSSGPRIDAFDIW

SEQ ID NO: 87 - protein, 13 aa, synthetic construct
CATSKSVWNFDYW

SEQ ID NO: 88 - protein, 12 aa, synthetic construct
CARSYGNYFTYW

SEQ ID NO: 89 - protein, 22 aa, synthetic construct
CARRGRIAAAGTGYYYYGMDVW

SEQ ID NO: 90 - protein, 12 aa, synthetic construct
CARGRRRDFDYW

SEQ ID NO: 91 - protein, 22 aa, synthetic construct
CARGPERIAAAGYYYYYGMDVW

SEQ ID NO: 92 - protein, 14 aa, synthetic construct
CARGVSRRGAFDIW

SEQ ID NO: 93 - protein, 12 aa, synthetic construct
CARNRYGATDYW

SEQ ID NO: 94 - protein, 20 aa, synthetic construct
CARDDGWRYGSVYYYYMDVW

SEQ ID NO: 95 - protein, 16 aa, synthetic construct
CARVLQYSGTDDLDVW

SEQ ID NO: 96 - protein, 13 aa, synthetic construct
CATGVGMVRGDPW

SEQ ID NO: 97 - protein, 11 aa, synthetic construct
CSSGYFYFDLW

SEQ ID NO: 98 - protein, 17 aa, synthetic construct
CVRRLWEAPGIGPFDVW

SEQ ID NO: 99 - protein, 13 aa, synthetic construct
CARGRGRGVFDYW

SEQ ID NO: 100 - protein, 10 aa, synthetic construct
CARDRTLGYW

SEQ ID NO: 101 - protein, 20 aa, synthetic construct
CARWDRVREGGRFSNAFDIW

SEQ ID NO: 102 - protein, 16 aa, synthetic construct
CARGKRDGYNYYFDYW

SEQ ID NO: 103 - protein, 19 aa, synthetic construct
CARQRRANGYSSSWEFDYW

SEQ ID NO: 104 - protein, 16 aa, synthetic construct
CAKGSRRSGFNLFDYW

SEQ ID NO: 105 - protein, 18 aa, synthetic construct
CARMGRIAASNYYGMDVW

SEQ ID NO: 106 - protein, 11 aa, synthetic construct
RASQGISSALA

SEQ ID NO: 107 - protein, 11 aa, synthetic construct
RASQGIRNYLA

SEQ ID NO: 108 - protein, 16 aa, synthetic construct
RSSQSLVHSDGNTYLN

SEQ ID NO: 109 - protein, 11 aa, synthetic construct
RASQSVSSYLA

SEQ ID NO: 110 - protein, 11 aa, synthetic construct
RASQNIENWLA

SEQ ID NO: 111 - protein, 16 aa, synthetic construct
RSSQSLVHSDGNTYLN

SEQ ID NO: 112 - protein, 11 aa, synthetic construct
RASQDISNYLA

SEQ ID NO: 113 - protein, 16 aa, synthetic construct
RSSQSLLHSNGRNYLD

SEQ ID NO: 114 - protein, 11 aa, synthetic construct
RASQALTYTLA

SEQ ID NO: 115 - protein, 11 aa, synthetic construct
RASQSINNYLN

SEQ ID NO: 116 - protein, 16 aa, synthetic construct
RSSQSLVKSDGNTYLS

SEQ ID NO: 117 - protein, 11 aa, synthetic construct
RASQSVNSYVN

SEQ ID NO: 118 - protein, 11 aa, synthetic construct
RASQSIARRIA

SEQ ID NO: 119 - protein, 11 aa, synthetic construct
RASQGISSYLA

SEQ ID NO: 120 - protein, 12 aa, synthetic construct
RASQSVSSSYLA

SEQ ID NO: 121 - protein, 11 aa, synthetic construct
RASQGIRNSLA

SEQ ID NO: 122 - protein, 11 aa, synthetic construct
RASQGISSYLA

SEQ ID NO: 123 - protein, 11 aa, synthetic construct
RASQSVSSYLA

SEQ ID NO: 124 - protein, 11 aa, synthetic construct
RASQSVSNYLA

SEQ ID NO: 125 - protein, 11 aa, synthetic construct
RASQGIGTFLA

SEQ ID NO: 126 - protein, 12 aa, synthetic construct
RASQSVSSSSLA

SEQ ID NO: 127 - protein, 16 aa, synthetic construct
RSSQSLLHRSGYNYLD

SEQ ID NO: 128 - protein, 11 aa, synthetic construct
RASQGINSWLA

SEQ ID NO: 129 - protein, 11 aa, synthetic construct
RASQSIDDHLN

SEQ ID NO: 130 - protein, 11 aa, synthetic construct
RASQSISSYLN

SEQ ID NO: 131 - protein, 16 aa, synthetic construct
RSSQSLVYSDGNTYLN

SEQ ID NO: 132 - protein, 11 aa, synthetic construct
RASQSISSWLA

SEQ ID NO: 133 - protein, 11 aa, synthetic construct
RASQSISSYLN

SEQ ID NO: 134 - protein, 11 aa, synthetic construct
RASQSVSKYLA

SEQ ID NO: 135 - protein, 11 aa, synthetic construct
RASQGIGRWLA

SEQ ID NO: 136 - protein, 11 aa, synthetic construct
RASQGISTYLA

SEQ ID NO: 137 - protein, 11 aa, synthetic construct
QASQDISNYLN

SEQ ID NO: 138 - protein, 11 aa, synthetic construct
RASQGISSFLA

SEQ ID NO: 139 - protein, 12 aa, synthetic construct
RASQSVSSSYLA

SEQ ID NO: 140 - protein, 11 aa, synthetic construct
RASQGISSQLA

SEQ ID NO: 141 - protein, 7 aa, synthetic construct
DASSLES

SEQ ID NO: 142 - protein, 7 aa, synthetic construct
AASTLQS

SEQ ID NO: 143 - protein, 7 aa, synthetic construct
KVSNRDS

SEQ ID NO: 144 - protein, 7 aa, synthetic construct
DASNRAT

SEQ ID NO: 145 - protein, 7 aa, synthetic construct
ATSRLEN

SEQ ID NO: 146 - protein, 7 aa, synthetic construct
KVSNRDS

SEQ ID NO: 147 - protein, 7 aa, synthetic construct
AASSLQS

SEQ ID NO: 148 - protein, 7 aa, synthetic construct
LGSNRAS

SEQ ID NO: 149 - protein, 7 aa, synthetic construct
DASSLES

SEQ ID NO: 150 - protein, 7 aa, synthetic construct
AASSLQS

SEQ ID NO: 151 - protein, 7 aa, synthetic construct
KVSNRDS

SEQ ID NO: 152 - protein, 7 aa, synthetic construct
AASSVHN

SEQ ID NO: 153 - protein, 7 aa, synthetic construct
DASNRAT

SEQ ID NO: 154 - protein, 7 aa, synthetic construct
AASLLQR

SEQ ID NO: 155 - protein, 7 aa, synthetic construct
GASSRAT

SEQ ID NO: 156 - protein, 7 aa, synthetic construct
AASKLQT

SEQ ID NO: 157 - protein, 7 aa, synthetic construct
DASNRAT

SEQ ID NO: 158 - protein, 7 aa, synthetic construct
DASNRAT

SEQ ID NO: 159 - protein, 7 aa, synthetic construct
GASSRAT

SEQ ID NO: 160 - protein, 7 aa, synthetic construct
ASSTVQR

SEQ ID NO: 161 - protein, 7 aa, synthetic construct
GASSRAT

SEQ ID NO: 162 - protein, 7 aa, synthetic construct
LGSIRAV

SEQ ID NO: 163 - protein, 7 aa, synthetic construct
AASTLQS

SEQ ID NO: 164 - protein, 7 aa, synthetic construct
SASTLQS

SEQ ID NO: 165 - protein, 7 aa, synthetic construct
AASSLQS

SEQ ID NO: 166 - protein, 7 aa, synthetic construct
KVSNRDS

SEQ ID NO: 167 - protein, 7 aa, synthetic construct
EASTLEV

SEQ ID NO: 168 - protein, 7 aa, synthetic construct
AASSLQS

SEQ ID NO: 169 - protein, 7 aa, synthetic construct
DVSNRAT

SEQ ID NO: 170 - protein, 7 aa, synthetic construct
AASNLQS

SEQ ID NO: 171 - protein, 7 aa, synthetic construct
GASTLQS

SEQ ID NO: 172 - protein, 7 aa, synthetic construct
DASSLES

SEQ ID NO: 173 - protein, 7 aa, synthetic construct
AASTLQS

SEQ ID NO: 174 - protein, 7 aa, synthetic construct
GASSRAT

SEQ ID NO: 175 - protein, 7 aa, synthetic construct
AASTLQS

SEQ ID NO: 176 - protein, 11 aa, synthetic construct [sequence omitted]

SEQ ID NO: 177 - protein, 11 aa, synthetic construct [sequence omitted]

SEQ ID NO: 178 - protein, 11 aa, synthetic construct
CMQGTQWPDTF

SEQ ID NO: 179 - protein, 13 aa, synthetic construct [sequence omitted]

SEQ ID NO: 180 - protein, 11 aa, synthetic construct
CHQANGFPWTF

SEQ ID NO: 181 - protein, 13 aa, synthetic construct [sequence omitted]

SEQ ID NO: 182 - protein, 11 aa, synthetic construct
CQQYKRYPFIF

SEQ ID NO: 183 - protein, 11 aa, synthetic construct [sequence omitted]

SEQ ID NO: 184 - protein, 11 aa, synthetic construct [sequence omitted]

SEQ ID NO: 185 - protein, 11 aa, synthetic construct [sequence omitted]

SEQ ID NO: 186 - protein, 11 aa, synthetic construct [sequence omitted]

SEQ ID NO: 187 - protein, 11 aa, synthetic construct [sequence omitted]

SEQ ID NO: 188 - protein, 11 aa, synthetic construct [sequence omitted]

SEQ ID NO: 189 - protein, 11 aa, synthetic construct [sequence omitted]

SEQ ID NO: 190 - protein, 12 aa, synthetic construct [sequence omitted]

SEQ ID NO: 191 - protein, 11 aa, synthetic construct [sequence omitted]

SEQ ID NO: 192 - protein, 11 aa, synthetic construct [sequence omitted]

SEQ ID NO: 193 - protein, 13 aa, synthetic construct [sequence omitted]

SEQ ID NO: 194 - protein, 11 aa, synthetic construct [sequence omitted]

SEQ ID NO: 195 - protein, 11 aa, synthetic construct [sequence omitted]

SEQ ID NO: 196 - protein, 10 aa, synthetic construct [sequence omitted]

SEQ ID NO: 197 - protein, 11 aa, synthetic construct [sequence omitted]

SEQ ID NO: 198 - protein, 11 aa, synthetic construct [sequence omitted]

SEQ ID NO: 199 - protein, 11 aa, synthetic construct [sequence omitted]

SEQ ID NO: 200 - protein, 11 aa, synthetic construct
CQQSYSTPRTF

SEQ ID NO: 201 - protein, 11 aa, synthetic construct [sequence omitted]

SEQ ID NO: 202 - protein, 11 aa, synthetic construct
CQQYHTDSRTF

SEQ ID NO: 203 - protein, 10 aa, synthetic construct [sequence omitted]

SEQ ID NO: 204 - protein, 11 aa, synthetic construct [sequence omitted]

SEQ ID NO: 205 - protein, 11 aa, synthetic construct [sequence omitted]

SEQ ID NO: 206 - protein, 11 aa, synthetic construct [sequence omitted]

SEQ ID NO: 207 - protein, 11 aa, synthetic construct
CQQYRSYPITF

SEQ ID NO: 208 - protein, 11 aa, synthetic construct
CQQFKIYPLTF

SEQ ID NO: 209 - protein, 12 aa, synthetic construct [sequence omitted]

SEQ ID NO: 210 - protein, 11 aa, synthetic construct [sequence omitted]

SEQ ID NO: 211 - protein, 125 aa, synthetic construct
QVQLQQSGPGLVKPSQTLSLTCTVSGGSISSGGYYWSWIRQHPGKGLEWIGYIYYSGSTYYNPSLKSRVTISVDTSKNQFSLKLSSVTAADTAVYYCARQRRANGYSSSWEFDYWGQGTLVTVSS

SEQ ID NO: 212 - protein, 115 aa, synthetic construct
QVQLVQSGGGVVQPGNSLRLSCVASGFTFSRYTIHWVRQAPGKGLEWVAVISYDGSNKYYADSVKGRFTISRDNSKNTLYLQMNSLRAEDTAVYYCARGGPTPDWGQGTLVTVSS

SEQ ID NO: 213 - protein, 122 aa, synthetic construct
QVQLVQSGAEVKKPGSSVKVSCKASGGTFSSYAISWVRQAPGQGLEWMGGIIPIFGTANYAQKFQGRVTMTRDTSTSTVYMELSSLRSEDTAVYYCARDSDFWSGYSSMDVWGQGTTVTVSS

SEQ ID NO: 214 - protein, 121 aa, synthetic construct
QVQLLESGGGLVKPGGSLRLSCAASGFTFSSYSMNWVRQAPGKGLEWVSSISSGSSYIYYADSVKGRFTISRDNAKNSLYLQMNSLRAEDTAVYYCARDQGASVTGTHTHWGQGTLVTVSS

SEQ ID NO: 215 - protein, 119 aa, synthetic construct
EVHLVESGPELVRPGASVTLSCKASGYTFTDYEMHWVKQTPVHGLEWIGAIDPETGGTAYNQKFKGKATLTADKSSSTAYMELRSLTSEDSAVYYCTTTYGNYWYFDVWGAGTLVTVSS

SEQ ID NO: 216 - protein, 119 aa, synthetic construct
EVQLVESGAEVKKPGSSVKVSCKASGGTFSSYAISWVRQAPGQGLEWMGGIIPIFGTANYAQKFQGRVTITADESTSTAYMELSSLRSEDTAVYYCAFTSGSYYYFDYWGQGTLVTVSS

SEQ ID NO: 217 - protein, 119 aa, synthetic construct
QVQLVQSGAEVKKPGSSVKVSCKASGGTFSSYAISWVRQAPGQGLEWMGGIIPIFGTANYAQKFQGRVTITADESTSTAYMELSSLRSEDTAVYYCARGGGGRGMTSDWGQGTLVTVSS

SEQ ID NO: 218 - protein, 127 aa, synthetic construct
QVQLLESGGGLVQPGGSLRLSCAASGFTFSSYAMSWVRQAPGKGLEWVSAISGSGGSTYYADSVKGRFTISRDNSKNTLYLQMNSLRAEDTAVYYCAKGTKMATIRLGYYYYGMDVWGQGTMVTVSS

SEQ ID NO: 219 - protein, 122 aa, synthetic construct
QVQLQESGPGLVKPSQTLSLTCTVSGGSISSGGYYWSWIRQHPGKGLEWIGYIYYSGSTYYNPSLKSRVTISVDTSKNQFSLKLSSVTAADTAVYYCARWGRGGSSWRFDIWGQGTMVTVSS

SEQ ID NO: 220 - protein, 121 aa, synthetic construct
EVQLLESGPGLVKPSQTLSLTCTVSGGSISSGGYYWSWIRQHPGKGLEWIGYIYYSGSTYYNPSLKSRVTISVDTSKNQFSLKLSSVTAADTAVYYCARDSRGRSYGMDVWGQGTMVTVSS

SEQ ID NO: 221 - protein, 118 aa, synthetic construct
QVQLVQSGAEVKKPGSSVKVSCKASGGTFSSYTISWVRQAPGQGLEWMGRIIPILGIANYAQKFQGRVTITADKSTSTAYMELSSLRSEDTAVYYCATGVGMVRGDPWGQGTLVTVSS

SEQ ID NO: 222 - protein, 120 aa, synthetic construct
QVQLVQSGGGVVQPGRSLRLPCAASGFTFSNYAMHWVRQAPGKGLEWVAVISYDGSKKYYADSVKGRFTISRDNSKNTLYLQVNSLRAEDTAVYYCATGYSSPWYGMDVWGQGTTVTVSS

SEQ ID NO: 223 - protein, 118 aa, synthetic construct
EVQLVETGGGVVQPGRSLRLSCAASGFTFSSYAMHWVRQAPGKGLEWVAVISYDGSNKYYADSVKGRFTISRDNSKNTLYLQMNSLRAEDTAVYYCARAAGHGILDYWGQGTLVTVSS

SEQ ID NO: 224 - protein, 126 aa, synthetic construct
RLQLQESGPGLVKPSQTLSLTCTVSGGSISSGGYYWSWIRQHPGKGLEWIGYIYYSGSTYYNPSLKSRVTISVDTSKNQFSLKLSSVTAADTAVYYCARIHHSTAGPYNNWYFDYWGQGTLVTVSS

SEQ ID NO: 225 - protein, 119 aa, synthetic construct
QVQLLDSGGGLVKPGGSLRLSCAASGFTFSSYGMHWVRQAPGKGLEWVAFISNDGSNKYYADSVKGRFTISRDNSKNTLYLQMNSLRAEDTAVYYCARLLRGPWNFDLWGRGTLVTVSS

SEQ ID NO: 226 - protein, 120 aa, synthetic construct
EVQLLESGGGLVQPGGSLRLSCAASGFTFSSYAMSWVRQAPGKGLEWVSAISGSGGSTYYADSVKGRFTISRDNSKNTLYLQMNSLRAEDTAVYYCATSSGPRIDAFDIWGQGTMVTVSS

SEQ ID NO: 227 - protein, 118 aa, synthetic construct
QVQLVQSGAEVKKPGASVKVSCKASGYTFTSYAMHWVRQAPGQRLEWMGWINAGNGNTKYSQKFQGRVTITRDTSASTAYMELSSLRSEDTAVYYCATSKSVWNFDYWGQGTLVTVSS

SEQ ID NO: 228 - protein, 117 aa, synthetic construct
QVQLVQSGGGLVQPGGSLRLSCAASGFTFSSYAMSWVRQAPGKGLEWVSAISGSGGSTYYADSVKGRFTISRDNPKNTLFLQMTSLRSEDTAMYYCARSYGNYFTYWGQGTLVTVSS

SEQ ID NO: 229 - protein, 126 aa, synthetic construct
QVQLLESGPGLVKPSETLSLTCTVSGDSISNYFWSWIRQSPGKGLEWIGYIHYSGTVSYNPSLRSRVTISIDTSKNQFSLKLSSVTAADTAVYYCARRGRIAAAGTGYYYYGMDVWGQGTTVTVSS

SEQ ID NO: 230 - protein, 117 aa, synthetic construct
EVQLVETGGGLVKPGGSLRLSCAASGFTFSSYSMNWVRQAPGKGLEWVSSISSSSSYIYYADSVKGRFTISRDNAKNSLYLQMNSLRAEDTAVYYCARGRRRDFDYWGQGTLVTVSS

SEQ ID NO: 231 - protein, 127 aa, synthetic construct
QVQLVQSGAEVKKPGSSVKVSCKASGDTFSSFAISWVRQAPGQGLEWMGTIIPLFTTPNYAQKFQGRVTITADESTRTAYMELSSLRSEDTAVYYCARGPERIAAAGYYYYYGMDVWGQGTTVTVSS

SEQ ID NO: 232 - protein, 119 aa, synthetic construct
QVQLVQSGAEVKKPGASVKVSCKASGYTFTSYYMHWVRQAPGQGLEWMGIINPSGGSTSYAQKFQGRVTMTRDTSTSTVYMELSSLRSEDTAVYYCARGVSRRGAFDIWGQGTMVTVSS

SEQ ID NO: 233 - protein, 117 aa, synthetic construct
EVQLVETGGGVVQPGRSLRLSCAASGFTFSSYAMHWVRQAPGKGLEWVAVISYDGSNKYYADSVKGRFTISRDNSKNTLYLQMNSLRAEDTAVYYCARNRYGATDYWGQGTLVTVSS

SEQ ID NO: 234 - protein, 125 aa, synthetic construct
QITLKESGPGLVKPSGTLSLTCAVSGGSISSSNWWSWVRQPPGKGLEWIGEIYHSGSTNYNPSLKSRVTISVDKSKNQFSLKLSSVTAADTAVYYCARDDGWRYGSVYYYYMDVWGKGTTVTVSS

SEQ ID NO: 235 - protein, 121 aa, synthetic construct
EVQLLESGGGLVQPGGSLRLSCAASGFTFSSYAMSWVRQAPGKGLEWVSAISGSGGRTYYADSVKGRFTISRDNSKNTLYLQMNSLRAEDTAVYYCARVLQYSGTDDLDVWGRGTLVTVSS

SEQ ID NO: 236 - protein, 118 aa, synthetic construct; identical to SEQ ID NO: 221

SEQ ID NO: 237 - protein, 116 aa, synthetic construct
EVQLLESGGGLVKPGGSLRLSCAASGLIFKNYGMNWVRLAPGKGLEWVASISGNSNYISYADSVKGRFTISRDNANNSLFLQMSSLRADDTAVYYCSSGYFYFDLWGPGTLVTVSS

SEQ ID NO: 238 - protein, 122 aa, synthetic construct
EVQLLESGGGLVKPGGSLRLSCAASGFTFSSYSMNWVRQAPGKGLEWVSSISSSSSYIYYADSVKGRFTISRDNAKNSLYLQMNSLRDGDTAIYYCVRRLWEAPGIGPFDVWGHGTMVTVSS

SEQ ID NO: 239 - protein, 118 aa, synthetic construct
EVQLLESGGGLVQPGGSLKLSCAASGFTFSGYAMHWVRQAPGKGLEWVAVISYDGSNKYYADSVKGRFTISRDNSKNTLYLQMNSLRAEDTAVYYCARGRGRGVFDYWGQGTLVTVSS

SEQ ID NO: 240 - protein, 115 aa, synthetic construct
EVQLLESGGGLVQPGGSLRLSCAASGFTFSSYSMNWVRQAPGKGLEWVSYISSSSSTIYYADSVKGRFTISRDNAKNSLYLQMNSLRDEDTAVYYCARDRTLGYWGQGTLVTVSS

SEQ ID NO: 241 - protein, 126 aa, synthetic construct
QVQLQQWGAGLLKPSQTLSLTCTVSGGSISSGGYYWSWIRQHPGKGLEWIGYIYYSGSTYYNPSLKSRVTISVDTSKNQFSLKLSSVTAADTAVYYCARWDRVREGGRFSNAFDIWGQGTMVTVSS

SEQ ID NO: 242 - protein, 122 aa, synthetic construct
QLQLQESGPGLVKPSQTLSLTCTVSGGSISSGGYYWSWIRQHPGKGLEWIGYIYYSGSTYYNPSLKSRVTISVDTSKNQFSLKLSSVTAADTAVYYCARGKRDGYNYYFDYWGQGTLVTVSS

SEQ ID NO: 243 - protein, 125 aa, synthetic construct; identical to SEQ ID NO: 211

SEQ ID NO: 244 - protein, 121 aa, synthetic construct
EVQLVESGGGLVQPGGSLRLSCAASGFTFSSYAMHWVRQAPGKGLEWVSAISGSGDSTYYADSVKGRFSISRDNSKNTLYLQMNSLRAEDTAVYYCAKGSRRSGFNLFDYWGQGTLVTVSS

SEQ ID NO: 245 - protein, 124 aa, synthetic construct
QLQLQESGPGLVKPSQTLSLTCTVSGGSISSGGYYWSWIRQHPGKGLEWIGYIYYSGSTYYNPSLKSRVTISVDTSKNQFSLKLSSVTAADTAVYYCARMGRIAASNYYGMDVWGQGTTVTVSS

SEQ ID NO: 246 - protein, 107 aa, synthetic construct
DIVMTQSPSSLSASVGDRVTITCRASQGISSALAWYQQKPGKAPKLLIYDASSLESGVPSRFSGSGSGTDFTLTISSLQPEDFATYYCQQFNSYPLTFGGGTKVEIK

SEQ ID NO: 247 - protein, 107 aa, synthetic construct
DIQMTQSPSSLSASVGDRVTITCRASQGIRNYLAWYQQKPGKVPRLLIFAASTLQSGVPSRFSGSGSGTDFTLTISSLQPEDVATYYCQKYYSAPFTFGPGTKVDIK

SEQ ID NO: 248 - protein, 112 aa, synthetic construct
DIVMTQSPLSLPVTLGQPASISCRSSQSLVHSDGNTYLNWFQQRPGQSPRRLIYKVSNRDSGVPDRFSGSGSGTDFTLKISRVEAEDVGVYYCMQGTQWPDTFGQGTKLEIK

SEQ ID NO: 249 - protein, 109 aa, synthetic construct
EIVMTQSPATLSLSPGERATLSCRASQSVSSYLAWYQQKPGQAPRLLIYDASNRATGIPARFSGSGSGTDFTLTISSLEPEDFAVYYCQQRSNWPPMYTFGQGTKLEIK

SEQ ID NO: 250 - protein, 107 aa, synthetic construct
DIQLTQSPSSVSASVGDRVTITCRASQNIENWLAWYQQKPGKAPKLLIYATSRLENDVPSRFSGSRSGTEFILTISSLQPEDFATYYCHQANGFPWTFGPGTKVDIK

SEQ ID NO: 251 - protein, 114 aa, synthetic construct
DVVMTQSPLSLPVTLGQPASISCRSSQSLVHSDGNTYLNWFQQRPGQSPRRLIYKVSNRDSGVPDRFSGSGSGTDFTLKISRVEAEDVGVYYCMQGTHWPPRYTFGQGTKLEIK

SEQ ID NO: 252 - protein, 107 aa, synthetic construct
NIQLTQSPSSLSASVGDRVTITCRASQDISNYLAWFQQKPGKAPKSLIYAASSLQSGVPSRFSGSWSGTDFTLTISSLQPEDIATYYCQQYKRYPFIFGQGTKLEIK

SEQ ID NO: 253 - protein, 112 aa, synthetic construct
DIVMTQSPLSLPVTPGEPASISCRSSQSLLHSNGRNYLDWYLQKPGQSPQLLIYLGSNRASGVSDRFSASGSGTDFTLQISRVEAEDVGIYYCMQALQTPWTFGQGTKVEVK

SEQ ID NO: 254 - protein, 107 aa, synthetic construct
AIQMTQSPSSLSASVGDRVTITCRASQALTYTLAWYQQKPGKAPRLLIHDASSLESGVPSRFSGSGSGTDFTLTITSLQPEDFATYYCQQFRSYPLTFGGGTKVEIK

SEQ ID NO: 255 - protein, 107 aa, synthetic construct
DIQMTQSPSSLSASVGDRVTITCRASQSINNYLNWYQEKPGKAPKLLIYAASSLQSGVPSRFSGSGSGTDFTLTISSLQPEDFATYYCQQSYSYPFTFGPGTKVDIK

SEQ ID NO: 256 - protein, 112 aa, synthetic construct
DIVMTQSPLSLPVTLGQPASISCRSSQSLVKSDGNTYLSWFQQRPGQSPRRLIYKVSNRDSGVPDRFSGSGSGTDFTLKISRVEAEDVGVYYCMQGTHWPPTFGPGTKVDIK

SEQ ID NO: 257 - protein, 107 aa, synthetic construct
NIQMTQSPSSLSASVGDRITITCRASQSVNSYVNWYQQTPGQAPKLLIYAASSVHNGVPVRFSGSRSGTEFILTISSLQPEDFVTYFCQQSFTSPWTFGQGTKLEMK

SEQ ID NO: 258 - protein, 107 aa, synthetic construct
EIVLTQSPATLSLSPGERATLSCRASQSIARRIAWYQQQPGQAPRLLIYDASNRATGIPARFSGSGSGTDFTLTISSLEPEDFAIYYCQQRANWPLTFGPGTKVDIK

SEQ ID NO: 259 - protein, 107 aa, synthetic construct
AIQLTQSPSSLSASVGDRVTITCRASQGISSYLAWYQQKPGKAPKLLIFAASLLQRGVPSRFSGSGFGTDFTLTISGLQPEDFATYFCQQFNTYPITFGGGTKVEIK

SEQ ID NO: 260 - protein, 109 aa, synthetic construct
EIVMTQSPGTLSLSPGERATLSCRASQSVSSSYLAWYQQKPGQAPRLLIYGASSRATGIPDRFSGSGSGTDFTLTISRLEPEDFAVYYCQQYGSSPPITFGQGTRLEIK

SEQ ID NO: 261 - protein, 107 aa, synthetic construct
NIQMTQSPSSLTASVGDRITITCRASQGIRNSLAWYQQKPGTAPKLLVSAASKLQTGVPSRFSGSGSGTDYTLTISSLQTEDFATYYCQQYYGTPPTFGQGTKLEIK

SEQ ID NO: 262 - protein, 107 aa, synthetic construct
EIVLTQSPATLSLSPGERATLSCRASQGISSYLAWYQQKPGQAPRLLIYDASNRATGIPARFSGSGSGTDFTLTISNLEPEDFAVYYCQQRKNWPLTFGGGSKVEIK

SEQ ID NO: 263 - protein, 109 aa, synthetic construct
EIVLTQSPATLSLSPGERATLSCRASQSVSSYLAWYQQKPGQAPRLLIYDASNRATGIPARFSGSGSGTDFTLTISSLEPEDFAVYYCQQRSNWPPELTFGGGTKVEIK

SEQ ID NO: 264 - protein, 107 aa, synthetic construct
EIVMTQSPATLSLSPGERATLSCRASQSVSNYLAWYQQKPGQAPRLLIYGASSRATGIPDRFSGSGSGTDFTLTISRLEPEDFAVYYCQQYGSSLWTFGQGTKVEIK

SEQ ID NO: 265 - protein, 107 aa, synthetic construct
DIQMTQSPSSLPASVGDRVTITCRASQGIGTFLAWYQQHLGKAPKLLISASSTVQRGVPSRFSGSGSGTEFTLTINSLQPEDFATYYCQQLNNYPRTFGQGTKVEIK

SEQ ID NO: 266 - protein, 107 aa, synthetic construct
EIVMTQSPGTLSLSPGQRATLSCRASQSVSSSSLAWYQQKPGQAPRLLIHGASSRATGIPDRFSGSGSGTDFTLTISRLEPEDFAVYYCQQYGTSWTFGQGTKVEIK

SEQ ID NO: 267 - protein, 112 aa, synthetic construct
DVVMTQSPLSLPVTPGEPASISCRSSQSLLHRSGYNYLDWYVQKPGQSPQLLIYLGSIRAVGVPDRFSGSASGTDFTLRISRVEAEDVGIYYCMQALQTPPAFGGGTKVEIK

SEQ ID NO: 268 - protein, 107 aa, synthetic construct
NIQLTQSPSSLSASVGDRVTITCRASQGINSWLAWYQQKPGKAPKLLIYAASTLQSGVPSRFSGSGSGTDFTLTINSLQPEDFATYYCQQLNSFPFTFGPGTKVHIK

SEQ ID NO: 269 - protein, 107 aa, synthetic construct
DIQLTQSPSSLSASVGDRVTITCRASQSIDDHLNWYQQKPGKVPKLLISSASTLQSGAPSRFSGSGYGTDFTLTISSLQVEDFATYYCQQSYSPPQTFGQGTKVEIK

SEQ ID NO: 270 - protein, 107 aa, synthetic construct
DIQLTQSPSSLSASVGDRVTITCRASQSISSYLNWYQQKPGKAPKLLIYAASSLQSGVPSRFSGSGSGTDFTLTISSLQPEDFATYYCQQSYSTPRTFGQGTRLEIK

SEQ ID NO: 271 - protein, 112 aa, synthetic construct
DVVMTQSPLSLPVTLGQPASISCRSSQSLVYSDGNTYLNWFQQRPGQSPRRLIYKVSNRDSGVPDRFSGSGSGTDFTLKISRVEAEDVGVYYCMQGTHWPPTFGQGTKLEIK

SEQ ID NO: 272 - protein, 107 aa, synthetic construct
DIQMTQSPSILSASVGDRVTLTCRASQSISSWLAWYQQTPGKAPRVLIYEASTLEVGVPSRFSGSGSGTDFTLTISSLQPEDFGTYFCQQYHTDSRTFGQGTILEIK

SEQ ID NO: 273 - protein, 106 aa, synthetic construct
DIVMTQSPSSLSASVGDRVTITCRASQSISSYLNWYQQKPGKAPKLLIYAASSLQSGVPSRFSGSGSGTDFTLTISSLQPEDFATYYCQQSYSTLTFGGGTKVEIK

SEQ ID NO: 274 - protein, 107 aa, synthetic construct
EIVLTQSPGTLSLSPGERATLSCRASQSVSKYLAWYQQKPGQAPRLLIYDVSNRATGIPARFSGSGSGTDFTLTISSLEPEDFAVYYCQQRRSWPLTFGGGTKVEIR

SEQ ID NO: 275 - protein, 107 aa, synthetic construct
NIQLTQSPSSVSASVGDRVTISCRASQGIGRWLAWYQQKPGKAPKLLIYAASNLQSGVPSRFSGSGSGTDFTLTISSLQPEDFATYYCQQANSFPRTFGPGTKVDIK

SEQ ID NO: 276 - protein, 107 aa, synthetic construct
NIQLTQSPSSLSASVGDRVTITCRASQGISTYLAWYQQKPGLAPKLLIYGASTLQSGVPSKFSGFGSGRDFTLTISSLQPEDIATYYCQQLNTYPPTFGQGTKLEIK

SEQ ID NO: 277 - protein, 107 aa, synthetic construct
DIVMTQSPSSLSASVGDRVTITCQASQDISNYLNWYQQKPGKAPKLLIYDASSLESGVPSKFSGSRSGTDFTLTISSLQPEDSATYYCQQYRSYPITFGGGTKVEIK

SEQ ID NO: 278 - protein, 107 aa, synthetic construct
DIQLTQSPSSLSASIGDRVTITCRASQGISSFLAWYQQKPGKAPQLLIYAASTLQSGVPSRFSGSGSGTEFTLTISSLQPEDFATYYCQQFKIYPLTFGGGTKVEVK

SEQ ID NO: 279 - protein, 109 aa, synthetic construct; identical to SEQ ID NO: 260

SEQ ID NO: 280 - protein, 107 aa, synthetic construct
DIQLTQSPSFLSASVGDRVTITCRASQGISSQLAWYQQEPGKAPKLLIYAASTLQSGVPSRFSGSGSGTEFTLTISSLQPEDFATYYCQQVNAYPLTFGPGTKVDIK

SEQ ID NO: 281 - protein, 327 aa, synthetic construct
ASTKGPSVFPLAPCSRSTSESTAALGCLVKDYFPEPVTVSWNSGALTSGVHTFPAVLQSSGLYSLSSVVTVPSSSLGTKTYTCNVDHKPSNTKVDKRVESKYGPPCPSCPAPEFLGGPSVFLFPPKPKDTLMISRTPEVTCVVVDVSQEDPEVQFNWYVDGVEVHNAKTKPREEQFNSTYRVVSVLTVLHQDWLNGKEYKCKVSNKGLPSSIEKTISKAKGQPREPQVYTLPPSQEEMTKNQVSLTCLVKGFYPSDIAVEWESNGQPENNYKTTPPVLDSDGSFFLYSRLTVDKSRWQEGNVFSCSVMHEALHNHYTQKSLSLSLGK

SEQ ID NO: 282 - protein, 327 aa, synthetic construct
ASTKGPSVFPLAPCSRSTSESTAALGCLVKDYFPEPVTVSWNSGALTSGVHTFPAVLQSSGLYSLSSVVTVPSSSLGTKTYTCNVDHKPSNTKVDKRVESKYGPPCPPCPAPEFLGGPSVFLFPPKPKDTLMISRTPEVTCVVVDVSQEDPEVQFNWYVDGVEVHNAKTKPREEQFNSTYRVVSVLTVLHQDWLNGKEYKCKVSNKGLPSSIEKTISKAKGQPREPQVYTLPPSQEEMTKNQVSLTCLVKGFYPSDIAVEWESNGQPENNYKTTPPVLDSDGSFFLYSRLTVDKSRWQEGNVFSCSVMHEALHNHYTQKSLSLSLGK

SEQ ID NO: 283 - protein, 452 aa, synthetic construct
QVQLQQSGPGLVKPSQTLSLTCTVSGGSISSGGYYWSWIRQHPGKGLEWIGYIYYSGSTYYNPSLKSRVTISVDTSKNQFSLKLSSVTAADTAVYYCARQRRANGYSSSWEFDYWGQGTLVTVSSASTKGPSVFPLAPCSRSTSESTAALGCLVKDYFPEPVTVSWNSGALTSGVHTFPAVLQSSGLYSLSSVVTVPSSSLGTKTYTCNVDHKPSNTKVDKRVESKYGPPCPSCPAPEFLGGPSVFLFPPKPKDTLMISRTPEVTCVVVDVSQEDPEVQFNWYVDGVEVHNAKTKPREEQFNSTYRVVSVLTVLHQDWLNGKEYKCKVSNKGLPSSIEKTISKAKGQPREPQVYTLPPSQEEMTKNQVSLTCLVKGFYPSDIAVEWESNGQPENNYKTTPPVLDSDGSFFLYSRLTVDKSRWQEGNVFSCSVMHEALHNHYTQKSLSLSLGK

SEQ ID NO: 284 - protein, 442 aa, synthetic construct
QVQLVQSGGGVVQPGNSLRLSCVASGFTFSRYTIHWVRQAPGKGLEWVAVISYDGSNKYYADSVKGRFTISRDNSKNTLYLQMNSLRAEDTAVYYCARGGPTPDWGQGTLVTVSSASTKGPSVFPLAPCSRSTSESTAALGCLVKDYFPEPVTVSWNSGALTSGVHTFPAVLQSSGLYSLSSVVTVPSSSLGTKTYTCNVDHKPSNTKVDKRVESKYGPPCPSCPAPEFLGGPSVFLFPPKPKDTLMISRTPEVTCVVVDVSQEDPEVQFNWYVDGVEVHNAKTKPREEQFNSTYRVVSVLTVLHQDWLNGKEYKCKVSNKGLPSSIEKTISKAKGQPREPQVYTLPPSQEEMTKNQVSLTCLVKGFYPSDIAVEWESNGQPENNYKTTPPVLDSDGSFFLYSRLTVDKSRWQEGNVFSCSVMHEALHNHYTQKSLSLSLGK

SEQ ID NO: 285 - protein, 449 aa, synthetic construct
QVQLVQSGAEVKKPGSSVKVSCKASGGTFSSYAISWVRQAPGQGLEWMGGIIPIFGTANYAQKFQGRVTMTRDTSTSTVYMELSSLRSEDTAVYYCARDSDFWSGYSSMDVWGQGTTVTVSSASTKGPSVFPLAPCSRSTSESTAALGCLVKDYFPEPVTVSWNSGALTSGVHTFPAVLQSSGLYSLSSVVTVPSSSLGTKTYTCNVDHKPSNTKVDKRVESKYGPPCPSCPAPEFLGGPSVFLFPPKPKDTLMISRTPEVTCVVVDVSQEDPEVQFNWYVDGVEVHNAKTKPREEQFNSTYRVVSVLTVLHQDWLNGKEYKCKVSNKGLPSSIEKTISKAKGQPREPQVYTLPPSQEEMTKNQVSLTCLVKGFYPSDIAVEWESNGQPENNYKTTPPVLDSDGSFFLYSRLTVDKSRWQEGNVFSCSVMHEALHNHYTQKSLSLSLGK

SEQ ID NO: 286 - protein, 448 aa, synthetic construct
QVQLLESGGGLVKPGGSLRLSCAASGFTFSSYSMNWVRQAPGKGLEWVSSISSGSSYIYYADSVKGRFTISRDNAKNSLYLQMNSLRAEDTAVYYCARDQGASVTGTHTHWGQGTLVTVSSASTKGPSVFPLAPCSRSTSESTAALGCLVKDYFPEPVTVSWNSGALTSGVHTFPAVLQSSGLYSLSSVVTVPSSSLGTKTYTCNVDHKPSNTKVDKRVESKYGPPCPSCPAPEFLGGPSVFLFPPKPKDTLMISRTPEVTCVVVDVSQEDPEVQFNWYVDGVEVHNAKTKPREEQFNSTYRVVSVLTVLHQDWLNGKEYKCKVSNKGLPSSIEKTISKAKGQPREPQVYTLPPSQEEMTKNQVSLTCLVKGFYPSDIAVEWESNGQPENNYKTTPPVLDSDGSFFLYSRLTVDKSRWQEGNVFSCSVMHEALHNHYTQKSLSLSLGK

SEQ ID NO: 287 - protein, 446 aa, synthetic construct
EVHLVESGPELVRPGASVTLSCKASGYTFTDYEMHWVKQTPVHGLEWIGAIDPETGGTAYNQKFKGKATLTADKSSSTAYMELRSLTSEDSAVYYCTTTYGNYWYFDVWGAGTLVTVSSASTKGPSVFPLAPCSRSTSESTAALGCLVKDYFPEPVTVSWNSGALTSGVHTFPAVLQSSGLYSLSSVVTVPSSSLGTKTYTCNVDHKPSNTKVDKRVESKYGPPCPSCPAPEFLGGPSVFLFPPKPKDTLMISRTPEVTCVVVDVSQEDPEVQFNWYVDGVEVHNAKTKPREEQFNSTYRVVSVLTVLHQDWLNGKEYKCKVSNKGLPSSIEKTISKAKGQPREPQVYTLPPSQEEMTKNQVSLTCLVKGFYPSDIAVEWESNGQPENNYKTTPPVLDSDGSFFLYSRLTVDKSRWQEGNVFSCSVMHEALHNHYTQKSLSLSLGK

SEQ ID NO: 288 - protein, 446 aa, synthetic construct
EVQLVESGAEVKKPGSSVKVSCKASGGTFSSYAISWVRQAPGQGLEWMGGIIPIFGTANYAQKFQGRVTITADESTSTAYMELSSLRSEDTAVYYCAFTSGSYYYFDYWGQGTLVTVSSASTKGPSVFPLAPCSRSTSESTAALGCLVKDYFPEPVTVSWNSGALTSGVHTFPAVLQSSGLYSLSSVVTVPSSSLGTKTYTCNVDHKPSNTKVDKRVESKYGPPCPSCPAPEFLGGPSVFLFPPKPKDTLMISRTPEVTCVVVDVSQEDPEVQFNWYVDGVEVHNAKTKPREEQFNSTYRVVSVLTVLHQDWLNGKEYKCKVSNKGLPSSIEKTISKAKGQPREPQVYTLPPSQEEMTKNQVSLTCLVKGFYPSDIAVEWESNGQPENNYKTTPPVLDSDGSFFLYSRLTVDKSRWQEGNVFSCSVMHEALHNHYTQKSLSLSLGK

SEQ ID NO: 289 - protein, 446 aa, synthetic construct
QVQLVQSGAEVKKPGSSVKVSCKASGGTFSSYAISWVRQAPGQGLEWMGGIIPIFGTANYAQKFQGRVTITADESTSTAYMELSSLRSEDTAVYYCARGGGGRGMTSDWGQGTLVTVSSASTKGPSVFPLAPCSRSTSESTAALGCLVKDYFPEPVTVSWNSGALTSGVHTFPAVLQSSGLYSLSSVVTVPSSSLGTKTYTCNVDHKPSNTKVDKRVESKYGPPCPSCPAPEFLGGPSVFLFPPKPKDTLMISRTPEVTCVVVDVSQEDPEVQFNWYVDGVEVHNAKTKPREEQFNSTYRVVSVLTVLHQDWLNGKEYKCKVSNKGLPSSIEKTISKAKGQPREPQVYTLPPSQEEMTKNQVSLTCLVKGFYPSDIAVEWESNGQPENNYKTTPPVLDSDGSFFLYSRLTVDKSRWQEGNVFSCSVMHEALHNHYTQKSLSLSLGK

SEQ ID NO: 290 - protein, 454 aa, synthetic construct
QVQLLESGGGLVQPGGSLRLSCAASGFTFSSYAMSWVRQAPGKGLEWVSAISGSGGSTYYADSVKGRFTISRDNSKNTLYLQMNSLRAEDTAVYYCAKGTKMATIRLGYYYYGMDVWGQGTMVTVSSASTKGPSVFPLAPCSRSTSESTAALGCLVKDYFPEPVTVSWNSGALTSGVHTFPAVLQSSGLYSLSSVVTVPSSSLGTKTYTCNVDHKPSNTKVDKRVESKYGPPCPSCPAPEFLGGPSVFLFPPKPKDTLMISRTPEVTCVVVDVSQEDPEVQFNWYVDGVEVHNAKTKPREEQFNSTYRVVSVLTVLHQDWLNGKEYKCKVSNKGLPSSIEKTISKAKGQPREPQVYTLPPSQEEMTKNQVSLTCLVKGFYPSDIAVEWESNGQPENNYKTTPPVLDSDGSFFLYSRLTVDKSRWQEGNVFSCSVMHEALHNHYTQKSLSLSLGK

SEQ ID NO: 291 - protein, 449 aa, synthetic construct
QVQLQESGPGLVKPSQTLSLTCTVSGGSISSGGYYWSWIRQHPGKGLEWIGYIYYSGSTYYNPSLKSRVTISVDTSKNQFSLKLSSVTAADTAVYYCARWGRGGSSWRFDIWGQGTMVTVSSASTKGPSVFPLAPCSRSTSESTAALGCLVKDYFPEPVTVSWNSGALTSGVHTFPAVLQSSGLYSLSSVVTVPSSSLGTKTYTCNVDHKPSNTKVDKRVESKYGPPCPSCPAPEFLGGPSVFLFPPKPKDTLMISRTPEVTCVVVDVSQEDPEVQFNWYVDGVEVHNAKTKPREEQFNSTYRVVSVLTVLHQDWLNGKEYKCKVSNKGLPSSIEKTISKAKGQPREPQVYTLPPSQEEMTKNQVSLTCLVKGFYPSDIAVEWESNGQPENNYKTTPPVLDSDGSFFLYSRLTVDKSRWQEGNVFSCSVMHEALHNHYTQKSLSLSLGK

SEQ ID NO: 292 - protein, 448 aa, synthetic construct
EVQLLESGPGLVKPSQTLSLTCTVSGGSISSGGYYWSWIRQHPGKGLEWIGYIYYSGSTYYNPSLKSRVTISVDTSKNQFSLKLSSVTAADTAVYYCARDSRGRSYGMDVWGQGTMVTVSSASTKGPSVFPLAPCSRSTSESTAALGCLVKDYFPEPVTVSWNSGALTSGVHTFPAVLQSSGLYSLSSVVTVPSSSLGTKTYTCNVDHKPSNTKVDKRVESKYGPPCPSCPAPEFLGGPSVFLFPPKPKDTLMISRTPEVTCVVVDVSQEDPEVQFNWYVDGVEVHNAKTKPREEQFNSTYRVVSVLTVLHQDWLNGKEYKCKVSNKGLPSSIEKTISKAKGQPREPQVYTLPPSQEEMTKNQVSLTCLVKGFYPSDIAVEWESNGQPENNYKTTPPVLDSDGSFFLYSRLTVDKSRWQEGNVFSCSVMHEALHNHYTQKSLSLSLGK

SEQ ID NO: 293 - protein, 445 aa, synthetic construct
QVQLVQSGAEVKKPGSSVKVSCKASGGTFSSYTISWVRQAPGQGLEWMGRIIPILGIANYAQKFQGRVTITADKSTSTAYMELSSLRSEDTAVYYCATGVGMVRGDPWGQGTLVTVSSASTKGPSVFPLAPCSRSTSESTAALGCLVKDYFPEPVTVSWNSGALTSGVHTFPAVLQSSGLYSLSSVVTVPSSSLGTKTYTCNVDHKPSNTKVDKRVESKYGPPCPSCPAPEFLGGPSVFLFPPKPKDTLMISRTPEVTCVVVDVSQEDPEVQFNWYVDGVEVHNAKTKPREEQFNSTYRVVSVLTVLHQDWLNGKEYKCKVSNKGLPSSIEKTISKAKGQPREPQVYTLPPSQEEMTKNQVSLTCLVKGFYPSDIAVEWESNGQPENNYKTTPPVLDSDGSFFLYSRLTVDKSRWQEGNVFSCSVMHEALHNHYTQKSLSLSLGK

SEQ ID NO: 294 - protein, 447 aa, synthetic construct
QVQLVQSGGGVVQPGRSLRLPCAASGFTFSNYAMHWVRQAPGKGLEWVAVISYDGSKKYYADSVKGRFTISRDNSKNTLYLQVNSLRAEDTAVYYCATGYSSPWYGMDVWGQGTTVTVSSASTKGPSVFPLAPCSRSTSESTAALGCLVKDYFPEPVTVSWNSGALTSGVHTFPAVLQSSGLYSLSSVVTVPSSSLGTKTYTCNVDHKPSNTKVDKRVESKYGPPCPSCPAPEFLGGPSVFLFPPKPKDTLMISRTPEVTCVVVDVSQEDPEVQFNWYVDGVEVHNAKTKPREEQFNSTYRVVSVLTVLHQDWLNGKEYKCKVSNKGLPSSIEKTISKAKGQPREPQVYTLPPSQEEMTKNQVSLTCLVKGFYPSDIAVEWESNGQPENNYKTTPPVLDSDGSFFLYSRLTVDKSRWQEGNVFSCSVMHEALHNHYTQKSLSLSLGK

SEQ ID NO: 295 - protein, 445 aa, synthetic construct
EVQLVETGGGVVQPGRSLRLSCAASGFTFSSYAMHWVRQAPGKGLEWVAVISYDGSNKYYADSVKGRFTISRDNSKNTLYLQMNSLRAEDTAVYYCARAAGHGILDYWGQGTLVTVSSASTKGPSVFPLAPCSRSTSESTAALGCLVKDYFPEPVTVSWNSGALTSGVHTFPAVLQSSGLYSLSSVVTVPSSSLGTKTYTCNVDHKPSNTKVDKRVESKYGPPCPSCPAPEFLGGPSVFLFPPKPKDTLMISRTPEVTCVVVDVSQEDPEVQFNWYVDGVEVHNAKTKPREEQFNSTYRVVSVLTVLHQDWLNGKEYKCKVSNKGLPSSIEKTISKAKGQPREPQVYTLPPSQEEMTKNQVSLTCLVKGFYPSDIAVEWESNGQPENNYKTTPPVLDSDGSFFLYSRLTVDKSRWQEGNVFSCSVMHEALHNHYTQKSLSLSLGK

SEQ ID NO: 296 - protein, 453 aa, synthetic construct
RLQLQESGPGLVKPSQTLSLTCTVSGGSISSGGYYWSWIRQHPGKGLEWIGYIYYSGSTYYNPSLKSRVTISVDTSKNQFSLKLSSVTAADTAVYYCARIHHSTAGPYNNWYFDYWGQGTLVTVSSASTKGPSVFPLAPCSRSTSESTAALGCLVKDYFPEPVTVSWNSGALTSGVHTFPAVLQSSGLYSLSSVVTVPSSSLGTKTYTCNVDHKPSNTKVDKRVESKYGPPCPSCPAPEFLGGPSVFLFPPKPKDTLMISRTPEVTCVVVDVSQEDPEVQFNWYVDGVEVHNAKTKPREEQFNSTYRVVSVLTVLHQDWLNGKEYKCKVSNKGLPSSIEKTISKAKGQPREPQVYTLPPSQEEMTKNQVSLTCLVKGFYPSDIAVEWESNGQPENNYKTTPPVLDSDGSFFLYSRLTVDKSRWQEGNVFSCSVMHEALHNHYTQKSLSLSLGK

SEQ ID NO: 297 - protein, 446 aa, synthetic construct
QVQLLDSGGGLVKPGGSLRLSCAASGFTFSSYGMHWVRQAPGKGLEWVAFISNDGSNKYYADSVKGRFTISRDNSKNTLYLQMNSLRAEDTAVYYCARLLRGPWNFDLWGRGTLVTVSSASTKGPSVFPLAPCSRSTSESTAALGCLVKDYFPEPVTVSWNSGALTSGVHTFPAVLQSSGLYSLSSVVTVPSSSLGTKTYTCNVDHKPSNTKVDKRVESKYGPPCPSCPAPEFLGGPSVFLFPPKPKDTLMISRTPEVTCVVVDVSQEDPEVQFNWYVDGVEVHNAKTKPREEQFNSTYRVVSVLTVLHQDWLNGKEYKCKVSNKGLPSSIEKTISKAKGQPREPQVYTLPPSQEEMTKNQVSLTCLVKGFYPSDIAVEWESNGQPENNYKTTPPVLDSDGSFFLYSRLTVDKSRWQEGNVFSCSVMHEALHNHYTQKSLSLSLGK

SEQ ID NO: 298 - protein, 447 aa, synthetic construct
EVQLLESGGGLVQPGGSLRLSCAASGFTFSSYAMSWVRQAPGKGLEWVSAISGSGGSTYYADSVKGRFTISRDNSKNTLYLQMNSLRAEDTAVYYCATSSGPRIDAFDIWGQGTMVTVSSASTKGPSVFPLAPCSRSTSESTAALGCLVKDYFPEPVTVSWNSGALTSGVHTFPAVLQSSGLYSLSSVVTVPSSSLGTKTYTCNVDHKPSNTKVDKRVESKYGPPCPSCPAPEFLGGPSVFLFPPKPKDTLMISRTPEVTCVVVDVSQEDPEVQFNWYVDGVEVHNAKTKPREEQFNSTYRVVSVLTVLHQDWLNGKEYKCKVSNKGLPSSIEKTISKAKGQPREPQVYTLPPSQEEMTKNQVSLTCLVKGFYPSDIAVEWESNGQPENNYKTTPPVLDSDGSFFLYSRLTVDKSRWQEGNVFSCSVMHEALHNHYTQKSLSLSLGK

SEQ ID NO: 299 - protein, 445 aa, synthetic construct
QVQLVQSGAEVKKPGASVKVSCKASGYTFTSYAMHWVRQAPGQRLEWMGWINAGNGNTKYSQKFQGRVTITRDTSASTAYMELSSLRSEDTAVYYCATSKSVWNFDYWGQGTLVTVSSASTKGPSVFPLAPCSRSTSESTAALGCLVKDYFPEPVTVSWNSGALTSGVHTFPAVLQSSGLYSLSSVVTVPSSSLGTKTYTCNVDHKPSNTKVDKRVESKYGPPCPSCPAPEFLGGPSVFLFPPKPKDTLMISRTPEVTCVVVDVSQEDPEVQFNWYVDGVEVHNAKTKPREEQFNSTYRVVSVLTVLHQDWLNGKEYKCKVSNKGLPSSIEKTISKAKGQPREPQVYTLPPSQEEMTKNQVSLTCLVKGFYPSDIAVEWESNGQPENNYKTTPPVLDSDGSFFLYSRLTVDKSRWQEGNVFSCSVMHEALHNHYTQKSLSLSLGK

SEQ ID NO: 300 - protein, 444 aa, synthetic construct
QVQLVQSGGGLVQPGGSLRLSCAASGFTFSSYAMSWVRQAPGKGLEWVSAISGSGGSTYYADSVKGRFTISRDNPKNTLFLQMTSLRSEDTAMYYCARSYGNYFTYWGQGTLVTVSSASTKGPSVFPLAPCSRSTSESTAALGCLVKDYFPEPVTVSWNSGALTSGVHTFPAVLQSSGLYSLSSVVTVPSSSLGTKTYTCNVDHKPSNTKVDKRVESKYGPPCPSCPAPEFLGGPSVFLFPPKPKDTLMISRTPEVTCVVVDVSQEDPEVQFNWYVDGVEVHNAKTKPREEQFNSTYRVVSVLTVLHQDWLNGKEYKCKVSNKGLPSSIEKTISKAKGQPREPQVYTLPPSQEEMTKNQVSLTCLVKGFYPSDIAVEWESNGQPENNYKTTPPVLDSDGSFFLYSRLTVDKSRWQEGNVFSCSVMHEALHNHYTQKSLSLSLGK

SEQ ID NO: 301 - protein, 453 aa, synthetic construct
QVQLLESGPGLVKPSETLSLTCTVSGDSISNYFWSWIRQSPGKGLEWIGYIHYSGTVSYNPSLRSRVTISIDTSKNQFSLKLSSVTAADTAVYYCARRGRIAAAGTGYYYYGMDVWGQGTTVTVSSASTKGPSVFPLAPCSRSTSESTAALGCLVKDYFPEPVTVSWNSGALTSGVHTFPAVLQSSGLYSLSSVVTVPSSSLGTKTYTCNVDHKPSNTKVDKRVESKYGPPCPSCPAPEFLGGPSVFLFPPKPKDTLMISRTPEVTCVVVDVSQEDPEVQFNWYVDGVEVHNAKTKPREEQFNSTYRVVSVLTVLHQDWLNGKEYKCKVSNKGLPSSIEKTISKAKGQPREPQVYTLPPSQEEMTKNQVSLTCLVKGFYPSDIAVEWESNGQPENNYKTTPPVLDSDGSFFLYSRLTVDKSRWQEGNVFSCSVMHEALHNHYTQKSLSLSLGK

SEQ ID NO: 302 - protein, 444 aa, synthetic construct
EVQLVETGGGLVKPGGSLRLSCAASGFTFSSYSMNWVRQAPGKGLEWVSSISSSSSYIYYADSVKGRFTISRDNAKNSLYLQMNSLRAEDTAVYYCARGRRRDFDYWGQGTLVTVSSASTKGPSVFPLAPCSRSTSESTAALGCLVKDYFPEPVTVSWNSGALTSGVHTFPAVLQSSGLYSLSSVVTVPSSSLGTKTYTCNVDHKPSNTKVDKRVESKYGPPCPSCPAPEFLGGPSVFLFPPKPKDTLMISRTPEVTCVVVDVSQEDPEVQFNWYVDGVEVHNAKTKPREEQFNSTYRVVSVLTVLHQDWLNGKEYKCKVSNKGLPSSIEKTISKAKGQPREPQVYTLPPSQEEMTKNQVSLTCLVKGFYPSDIAVEWESNGQPENNYKTTPPVLDSDGSFFLYSRLTVDKSRWQEGNVFSCSVMHEALHNHYTQKSLSLSLGK

SEQ ID NO: 303 - protein, 454 aa, synthetic construct
QVQLVQSGAEVKKPGSSVKVSCKASGDTFSSFAISWVRQAPGQGLEWMGTIIPLFTTPNYAQKFQGRVTITADESTRTAYMELSSLRSEDTAVYYCARGPERIAAAGYYYYYGMDVWGQGTTVTVSSASTKGPSVFPLAPCSRSTSESTAALGCLVKDYFPEPVTVSWNSGALTSGVHTFPAVLQSSGLYSLSSVVTVPSSSLGTKTYTCNVDHKPSNTKVDKRVESKYGPPCPSCPAPEFLGGPSVFLFPPKPKDTLMISRTPEVTCVVVDVSQEDPEVQFNWYVDGVEVHNAKTKPREEQFNSTYRVVSVLTVLHQDWLNGKEYKCKVSNKGLPSSIEKTISKAKGQPREPQVYTLPPSQEEMTKNQVSLTCLVKGFYPSDIAVEWESNGQPENNYKTTPPVLDSDGSFFLYSRLTVDKSRWQEGNVFSCSVMHEALHNHYTQKSLSLSLGK

SEQ ID NO: 304 - protein, 446 aa, synthetic construct
QVQLVQSGAEVKKPGASVKVSCKASGYTFTSYYMHWVRQAPGQGLEWMGIINPSGGSTSYAQKFQGRVTMTRDTSTSTVYMELSSLRSEDTAVYYCARGVSRRGAFDIWGQGTMVTVSSASTKGPSVFPLAPCSRSTSESTAALGCLVKDYFPEPVTVSWNSGALTSGVHTFPAVLQSSGLYSLSSVVTVPSSSLGTKTYTCNVDHKPSNTKVDKRVESKYGPPCPSCPAPEFLGGPSVFLFPPKPKDTLMISRTPEVTCVVVDVSQEDPEVQFNWYVDGVEVHNAKTKPREEQFNSTYRVVSVLTVLHQDWLNGKEYKCKVSNKGLPSSIEKTISKAKGQPREPQVYTLPPSQEEMTKNQVSLTCLVKGFYPSDIAVEWESNGQPENNYKTTPPVLDSDGSFFLYSRLTVDKSRWQEGNVFSCSVMHEALHNHYTQKSLSLSLGK

SEQ ID NO: 305 - protein, 444 aa, synthetic construct
EVQLVETGGGVVQPGRSLRLSCAASGFTFSSYAMHWVRQAPGKGLEWVAVISYDGSNKYYADSVKGRFTISRDNSKNTLYLQMNSLRAEDTAVYYCARNRYGATDYWGQGTLVTVSSASTKGPSVFPLAPCSRSTSESTAALGCLVKDYFPEPVTVSWNSGALTSGVHTFPAVLQSSGLYSLSSVVTVPSSSLGTKTYTCNVDHKPSNTKVDKRVESKYGPPCPSCPAPEFLGGPSVFLFPPKPKDTLMISRTPEVTCVVVDVSQEDPEVQFNWYVDGVEVHNAKTKPREEQFNSTYRVVSVLTVLHQDWLNGKEYKCKVSNKGLPSSIEKTISKAKGQPREPQVYTLPPSQEEMTKNQVSLTCLVKGFYPSDIAVEWESNGQPENNYKTTPPVLDSDGSFFLYSRLTVDKSRWQEGNVFSCSVMHEALHNHYTQKSLSLSLGK

SEQ ID NO: 306 - protein, 452 aa, synthetic construct
QITLKESGPGLVKPSGTLSLTCAVSGGSISSSNWWSWVRQPPGKGLEWIGEIYHSGSTNYNPSLKSRVTISVDKSKNQFSLKLSSVTAADTAVYYCARDDGWRYGSVYYYYMDVWGKGTTVTVSSASTKGPSVFPLAPCSRSTSESTAALGCLVKDYFPEPVTVSWNSGALTSGVHTFPAVLQSSGLYSLSSVVTVPSSSLGTKTYTCNVDHKPSNTKVDKRVESKYGPPCPSCPAPEFLGGPSVFLFPPKPKDTLMISRTPEVTCVVVDVSQEDPEVQFNWYVDGVEVHNAKTKPREEQFNSTYRVVSVLTVLHQDWLNGKEYKCKVSNKGLPSSIEKTISKAKGQPREPQVYTLPPSQEEMTKNQVSLTCLVKGFYPSDIAVEWESNGQPENNYKTTPPVLDSDGSFFLYSRLTVDKSRWQEGNVFSCSVMHEALHNHYTQKSLSLSLGK

SEQ ID NO: 307 - protein, 448 aa, synthetic construct
EVQLLESGGGLVQPGGSLRLSCAASGFTFSSYAMSWVRQAPGKGLEWVSAISGSGGRTYYADSVKGRFTISRDNSKNTLYLQMNSLRAEDTAVYYCARVLQYSGTDDLDVWGRGTLVTVSSASTKGPSVFPLAPCSRSTSESTAALGCLVKDYFPEPVTVSWNSGALTSGVHTFPAVLQSSGLYSLSSVVTVPSSSLGTKTYTCNVDHKPSNTKVDKRVESKYGPPCPSCPAPEFLGGPSVFLFPPKPKDTLMISRTPEVTCVVVDVSQEDPEVQFNWYVDGVEVHNAKTKPREEQFNSTYRVVSVLTVLHQDWLNGKEYKCKVSNKGLPSSIEKTISKAKGQPREPQVYTLPPSQEEMTKNQVSLTCLVKGFYPSDIAVEWESNGQPENNYKTTPPVLDSDGSFFLYSRLTVDKSRWQEGNVFSCSVMHEALHNHYTQKSLSLSLGK

SEQ ID NO: 308 - protein, 445 aa, synthetic construct; identical to SEQ ID NO: 293

SEQ ID NO: 309 - protein, 443 aa, synthetic construct
EVQLLESGGGLVKPGGSLRLSCAASGLIFKNYGMNWVRLAPGKGLEWVASISGNSNYISYADSVKGRFTISRDNANNSLFLQMSSLRADDTAVYYCSSGYFYFDLWGPGTLVTVSSASTKGPSVFPLAPCSRSTSESTAALGCLVKDYFPEPVTVSWNSGALTSGVHTFPAVLQSSGLYSLSSVVTVPSSSLGTKTYTCNVDHKPSNTKVDKRVESKYGPPCPSCPAPEFLGGPSVFLFPPKPKDTLMISRTPEVTCVVVDVSQEDPEVQFNWYVDGVEVHNAKTKPREEQFNSTYRVVSVLTVLHQDWLNGKEYKCKVSNKGLPSSIEKTISKAKGQPREPQVYTLPPSQEEMTKNQVSLTCLVKGFYPSDIAVEWESNGQPENNYKTTPPVLDSDGSFFLYSRLTVDKSRWQEGNVFSCSVMHEALHNHYTQKSLSLSLGK

SEQ ID NO: 310 - protein, 449 aa, synthetic construct
EVQLLESGGGLVKPGGSLRLSCAASGFTFSSYSMNWVRQAPGKGLEWVSSISSSSSYIYYADSVKGRFTISRDNAKNSLYLQMNSLRDGDTAIYYCVRRLWEAPGIGPFDVWGHGTMVTVSSASTKGPSVFPLAPCSRSTSESTAALGCLVKDYFPEPVTVSWNSGALTSGVHTFPAVLQSSGLYSLSSVVTVPSSSLGTKTYTCNVDHKPSNTKVDKRVESKYGPPCPSCPAPEFLGGPSVFLFPPKPKDTLMISRTPEVTCVVVDVSQEDPEVQFNWYVDGVEVHNAKTKPREEQFNSTYRVVSVLTVLHQDWLNGKEYKCKVSNKGLPSSIEKTISKAKGQPREPQVYTLPPSQEEMTKNQVSLTCLVKGFYPSDIAVEWESNGQPENNYKTTPPVLDSDGSFFLYSRLTVDKSRWQEGNVFSCSVMHEALHNHYTQKSLSLSLGK

SEQ ID NO: 311 - protein, 445 aa, synthetic construct
EVQLLESGGGLVQPGGSLKLSCAASGFTFSGYAMHWVRQAPGKGLEWVAVISYDGSNKYYADSVKGRFTISRDNSKNTLYLQMNSLRAEDTAVYYCARGRGRGVFDYWGQGTLVTVSSASTKGPSVFPLAPCSRSTSESTAALGCLVKDYFPEPVTVSWNSGALTSGVHTFPAVLQSSGLYSLSSVVTVPSSSLGTKTYTCNVDHKPSNTKVDKRVESKYGPPCPSCPAPEFLGGPSVFLFPPKPKDTLMISRTPEVTCVVVDVSQEDPEVQFNWYVDGVEVHNAKTKPREEQFNSTYRVVSVLTVLHQDWLNGKEYKCKVSNKGLPSSIEKTISKAKGQPREPQVYTLPPSQEEMTKNQVSLTCLVKGFYPSDIAVEWESNGQPENNYKTTPPVLDSDGSFFLYSRLTVDKSRWQEGNVFSCSVMHEALHNHYTQKSLSLSLGK

SEQ ID NO: 312 - protein, 442 aa, synthetic construct
EVQLLESGGGLVQPGGSLRLSCAASGFTFSSYSMNWVRQAPGKGLEWVSYISSSSSTIYYADSVKGRFTISRDNAKNSLYLQMNSLRDEDTAVYYCARDRTLGYWGQGTLVTVSSASTKGPSVFPLAPCSRSTSESTAALGCLVKDYFPEPVTVSWNSGALTSGVHTFPAVLQSSGLYSLSSVVTVPSSSLGTKTYTCNVDHKPSNTKVDKRVESKYGPPCPSCPAPEFLGGPSVFLFPPKPKDTLMISRTPEVTCVVVDVSQEDPEVQFNWYVDGVEVHNAKTKPREEQFNSTYRVVSVLTVLHQDWLNGKEYKCKVSNKGLPSSIEKTISKAKGQPREPQVYTLPPSQEEMTKNQVSLTCLVKGFYPSDIAVEWESNGQPENNYKTTPPVLDSDGSFFLYSRLTVDKSRWQEGNVFSCSVMHEALHNHYTQKSLSLSLGK

SEQ ID NO: 313 - protein, 453 aa, synthetic construct
QVQLQQWGAGLLKPSQTLSLTCTVSGGSISSGGYYWSWIRQHPGKGLEWIGYIYYSGSTYYNPSLKSRVTISVDTSKNQFSLKLSSVTAADTAVYYCARWDRVREGGRFSNAFDIWGQGTMVTVSSASTKGPSVFPLAPCSRSTSESTAALGCLVKDYFPEPVTVSWNSGALTSGVHTFPAVLQSSGLYSLSSVVTVPSSSLGTKTYTCNVDHKPSNTKVDKRVESKYGPPCPSCPAPEFLGGPSVFLFPPKPKDTLMISRTPEVTCVVVDVSQEDPEVQFNWYVDGVEVHNAKTKPREEQFNSTYRVVSVLTVLHQDWLNGKEYKCKVSNKGLPSSIEKTISKAKGQPREPQVYTLPPSQEEMTKNQVSLTCLVKGFYPSDIAVEWESNGQPENNYKTTPPVLDSDGSFFLYSRLTVDKSRWQEGNVFSCSVMHEALHNHYTQKSLSLSLGK

SEQ ID NO: 314 - protein, 449 aa, synthetic construct
QLQLQESGPGLVKPSQTLSLTCTVSGGSISSGGYYWSWIRQHPGKGLEWIGYIYYSGSTYYNPSLKSRVTISVDTSKNQFSLKLSSVTAADTAVYYCARGKRDGYNYYFDYWGQGTLVTVSSASTKGPSVFPLAPCSRSTSESTAALGCLVKDYFPEPVTVSWNSGALTSGVHTFPAVLQSSGLYSLSSVVTVPSSSLGTKTYTCNVDHKPSNTKVDKRVESKYGPPCPSCPAPEFLGGPSVFLFPPKPKDTLMISRTPEVTCVVVDVSQEDPEVQFNWYVDGVEVHNAKTKPREEQFNSTYRVVSVLTVLHQDWLNGKEYKCKVSNKGLPSSIEKTISKAKGQPREPQVYTLPPSQEEMTKNQVSLTCLVKGFYPSDIAVEWESNGQPENNYKTTPPVLDSDGSFFLYSRLTVDKSRWQEGNVFSCSVMHEALHNHYTQKSLSLSLGK

SEQ ID NO: 315 - protein, 452 aa, synthetic construct; identical to SEQ ID NO: 283

SEQ ID NO: 316 - protein, 448 aa, synthetic construct
EVQLVESGGGLVQPGGSLRLSCAASGFTFSSYAMHWVRQAPGKGLEWVSAISGSGDSTYYADSVKGRFSISRDNSKNTLYLQMNSLRAEDTAVYYCAKGSRRSGFNLFDYWGQGTLVTVSSASTKGPSVFPLAPCSRSTSESTAALGCLVKDYFPEPVTVSWNSGALTSGVHTFPAVLQSSGLYSLSSVVTVPSSSLGTKTYTCNVDHKPSNTKVDKRVESKYGPPCPSCPAPEFLGGPSVFLFPPKPKDTLMISRTPEVTCVVVDVSQEDPEVQFNWYVDGVEVHNAKTKPREEQFNSTYRVVSVLTVLHQDWLNGKEYKCKVSNKGLPSSIEKTISKAKGQPREPQVYTLPPSQEEMTKNQVSLTCLVKGFYPSDIAVEWESNGQPENNYKTTPPVLDSDGSFFLYSRLTVDKSRWQEGNVFSCSVMHEALHNHYTQKSLSLSLGK

SEQ ID NO: 317 - protein, 451 aa, synthetic construct
QLQLQESGPGLVKPSQTLSLTCTVSGGSISSGGYYWSWIRQHPGKGLEWIGYIYYSGSTYYNPSLKSRVTISVDTSKNQFSLKLSSVTAADTAVYYCARMGRIAASNYYGMDVWGQGTTVTVSSASTKGPSVFPLAPCSRSTSESTAALGCLVKDYFPEPVTVSWNSGALTSGVHTFPAVLQSSGLYSLSSVVTVPSSSLGTKTYTCNVDHKPSNTKVDKRVESKYGPPCPSCPAPEFLGGPSVFLFPPKPKDTLMISRTPEVTCVVVDVSQEDPEVQFNWYVDGVEVHNAKTKPREEQFNSTYRVVSVLTVLHQDWLNGKEYKCKVSNKGLPSSIEKTISKAKGQPREPQVYTLPPSQEEMTKNQVSLTCLVKGFYPSDIAVEWESNGQPENNYKTTPPVLDSDGSFFLYSRLTVDKSRWQEGNVFSCSVMHEALHNHYTQKSLSLSLGK

SEQ ID NO: 318 - protein, 214 aa, synthetic construct
DIVMTQSPSSLSASVGDRVTITCRASQGISSALAWYQQKPGKAPKLLIYDASSLESGVPSRFSGSGSGTDFTLTISSLQPEDFATYYCQQFNSYPLTFGGGTKVEIKRTVAAPSVFIFPPSDEQLKSGTASVVCLLNNFYPREAKVQWKVDNALQSGNSQESVTEQDSKDSTYSLSSTLTLSKADYEKHKVYACEVTHQGLSSPVTKSFNRGEC

SEQ ID NO: 319 - protein, 214 aa, synthetic construct
DIQMTQSPSSLSASVGDRVTITCRASQGIRNYLAWYQQKPGKVPRLLIFAASTLQSGVPSRFSGSGSGTDFTLTISSLQPEDVATYYCQKYYSAPFTFGPGTKVDIKRTVAAPSVFIFPPSDEQLKSGTASVVCLLNNFYPREAKVQWKVDNALQSGNSQESVTEQDSKDSTYSLSSTLTLSKADYEKHKVYACEVTHQGLSSPVTKSFNRGEC

SEQ ID NO: 320 - protein, 219 aa, synthetic construct
DIVMTQSPLSLPVTLGQPASISCRSSQSLVHSDGNTYLNWFQQRPGQSPRRLIYKVSNRDSGVPDRFSGSGSGTDFTLKISRVEAEDVGVYYCMQGTQWPDTFGQGTKLEIKRTVAAPSVFIFPPSDEQLKSGTASVVCLLNNFYPREAKVQWKVDNALQSGNSQESVTEQDSKDSTYSLSSTLTLSKADYEKHKVYACEVTHQGLSSPVTKSFNRGEC

SEQ ID NO: 321 - protein, 216 aa, synthetic construct
EIVMTQSPATLSLSPGERATLSCRASQSVSSYLAWYQQKPGQAPRLLIYDASNRATGIPARFSGSGSGTDFTLTISSLEPEDFAVYYCQQRSNWPPMYTFGQGTKLEIKRTVAAPSVFIFPPSDEQLKSGTASVVCLLNNFYPREAKVQWKVDNALQSGNSQESVTEQDSKDSTYSLSSTLTLSKADYEKHKVYACEVTHQGLSSPVTKSFNRGEC

SEQ ID NO: 322 - protein, 214 aa, synthetic construct
DIQLTQSPSSVSASVGDRVTITCRASQNIENWLAWYQQKPGKAPKLLIYATSRLENDVPSRFSGSRSGTEFILTISSLQPEDFATYYCHQANGFPWTFGPGTKVDIKRTVAAPSVFIFPPSDEQLKSGTASVVCLLNNFYPREAKVQWKVDNALQSGNSQESVTEQDSKDSTYSLSSTLTLSKADYEKHKVYACEVTHQGLSSPVTKSFNRGEC

SEQ ID NO: 323 - protein, 221 aa, synthetic construct
DVVMTQSPLSLPVTLGQPASISCRSSQSLVHSDGNTYLNWFQQRPGQSPRRLIYKVSNRDSGVPDRFSGSGSGTDFTLKISRVEAEDVGVYYCMQGTHWPPRYTFGQGTKLEIKRTVAAPSVFIFPPSDEQLKSGTASVVCLLNNFYPREAKVQWKVDNALQSGNSQESVTEQDSKDSTYSLSSTLTLSKADYEKHKVYACEVTHQGLSSPVTKSFNRGEC

SEQ ID NO: 324 - protein, 214 aa, synthetic construct
NIQLTQSPSSLSASVGDRVTITCRASQDISNYLAWFQQKPGKAPKSLIYAASSLQSGVPSRFSGSWSGTDFTLTISSLQPEDIATYYCQQYKRYPFIFGQGTKLEIKRTVAAPSVFIFPPSDEQLKSGTASVVCLLNNFYPREAKVQWKVDNALQSGNSQESVTEQDSKDSTYSLSSTLTLSKADYEKHKVYACEVTHQGLSSPVTKSFNRGEC

SEQ ID NO: 325 - protein, 219 aa, synthetic construct
DIVMTQSPLSLPVTPGEPASISCRSSQSLLHSNGRNYLDWYLQKPGQSPQLLIYLGSNRASGVSDRFSASGSGTDFTLQISRVEAEDVGIYYCMQALQTPWTFGQGTKVEVKRTVAAPSVFIFPPSDEQLKSGTASVVCLLNNFYPREAKVQWKVDNALQSGNSQESVTEQDSKDSTYSLSSTLTLSKADYEKHKVYACEVTHQGLSSPVTKSFNRGEC

SEQ ID NO: 326 - protein, 214 aa, synthetic construct
AIQMTQSPSSLSASVGDRVTITCRASQALTYTLAWYQQKPGKAPRLLIHDASSLESGVPSRFSGSGSGTDFTLTITSLQPEDFATYYCQQFRSYPLTFGGGTKVEIKRTVAAPSVFIFPPSDEQLKSGTASVVCLLNNFYPREAKVQWKVDNALQSGNSQESVTEQDSKDSTYSLSSTLTLSKADYEKHKVYACEVTHQGLSSPVTKSFNRGEC

SEQ ID NO: 327 - protein, 214 aa, synthetic construct
DIQMTQSPSSLSASVGDRVTITCRASQSINNYLNWYQEKPGKAPKLLIYAASSLQSGVPSRFSGSGSGTDFTLTISSLQPEDFATYYCQQSYSYPFTFGPGTKVDIKRTVAAPSVFIFPPSDEQLKSGTASVVCLLNNFYPREAKVQWKVDNALQSGNSQESVTEQDSKDSTYSLSSTLTLSKADYEKHKVYACEVTHQGLSSPVTKSFNRGEC

SEQ ID NO: 328 - protein, 219 aa, synthetic construct
DIVMTQSPLSLPVTLGQPASISCRSSQSLVKSDGNTYLSWFQQRPGQSPRRLIYKVSNRDSGVPDRFSGSGSGTDFTLKISRVEAEDVGVYYCMQGTHWPPTFGPGTKVDIKRTVAAPSVFIFPPSDEQLKSGTASVVCLLNNFYPREAKVQWKVDNALQSGNSQESVTEQDSKDSTYSLSSTLTLSKADYEKHKVYACEVTHQGLSSPVTKSFNRGEC

SEQ ID NO: 329 - protein, 214 aa, synthetic construct
NIQMTQSPSSLSASVGDRITITCRASQSVNSYVNWYQQTPGQAPKLLIYAASSVHNGVPVRFSGSRSGTEFILTISSLQPEDFVTYFCQQSFTSPWTFGQGTKLEMKRTVAAPSVFIFPPSDEQLKSGTASVVCLLNNFYPREAKVQWKVDNALQSGNSQESVTEQDSKDSTYSLSSTLTLSKADYEKHKVYACEVTHQGLSSPVTKSFNRGEC

SEQ ID NO: 330 - protein, 214 aa, synthetic construct
EIVLTQSPATLSLSPGERATLSCRASQSIARRIAWYQQQPGQAPRLLIYDASNRATGIPARFSGSGSGTDFTLTISSLEPEDFAIYYCQQRANWPLTFGPGTKVDIKRTVAAPSVFIFPPSDEQLKSGTASVVCLLNNFYPREAKVQWKVDNALQSGNSQESVTEQDSKDSTYSLSSTLTLSKADYEKHKVYACEVTHQGLSSPVTKSFNRGEC

SEQ ID NO: 331 - protein, 214 aa, synthetic construct
AIQLTQSPSSLSASVGDRVTITCRASQGISSYLAWYQQKPGKAPKLLIFAASLLQRGVPSRFSGSGFGTDFTLTISGLQPEDFATYFCQQFNTYPITFGGGTKVEIKRTVAAPSVFIFPPSDEQLKSGTASVVCLLNNFYPREAKVQWKVDNALQSGNSQESVTEQDSKDSTYSLSSTLTLSKADYEKHKVYACEVTHQGLSSPVTKSFNRGEC

SEQ ID NO: 332 - protein, 216 aa, synthetic construct
EIVMTQSPGTLSLSPGERATLSCRASQSVSSSYLAWYQQKPGQAPRLLIYGASSRATGIPDRFSGSGSGTDFTLTISRLEPEDFAVYYCQQYGSSPPITFGQGTRLEIKRTVAAPSVFIFPPSDEQLKSGTASVVCLLNNFYPREAKVQWKVDNALQSGNSQESVTEQDSKDSTYSLSSTLTLSKADYEKHKVYACEVTHQGLSSPVTKSFNRGEC

SEQ ID NO: 333 - protein, 214 aa, synthetic construct
NIQMTQSPSSLTASVGDRITITCRASQGIRNSLAWYQQKPGTAPKLLVSAASKLQTGVPSRFSGSGSGTDYTLTISSLQTEDFATYYCQQYYGTPPTFGQGTKLEIKRTVAAPSVFIFPPSDEQLKSGTASVVCLLNNFYPREAKVQWKVDNALQSGNSQESVTEQDSKDSTYSLSSTLTLSKADYEKHKVYACEVTHQGLSSPVTKSFNRGEC

SEQ ID NO: 334 - protein, 214 aa, synthetic construct
EIVLTQSPATLSLSPGERATLSCRASQGISSYLAWYQQKPGQAPRLLIYDASNRATGIPARFSGSGSGTDFTLTISNLEPEDFAVYYCQQRKNWPLTFGGGSKVEIKRTVAAPSVFIFPPSDEQLKSGTASVVCLLNNFYPREAKVQWKVDNALQSGNSQESVTEQDSKDSTYSLSSTLTLSKADYEKHKVYACEVTHQGLSSPVTKSFNRGEC

SEQ ID NO: 335 - protein, 216 aa, synthetic construct
EIVLTQSPATLSLSPGERATLSCRASQSVSSYLAWYQQKPGQAPRLLIYDASNRATGIPARFSGSGSGTDFTLTISSLEPEDFAVYYCQQRSNWPPELTFGGGTKVEIKRTVAAPSVFIFPPSDEQLKSGTASVVCLLNNFYPREAKVQWKVDNALQSGNSQESVTEQDSKDSTYSLSSTLTLSKADYEKHKVYACEVTHQGLSSPVTKSFNRGEC

SEQ ID NO: 336 - protein, 214 aa, synthetic construct
EIVMTQSPATLSLSPGERATLSCRASQSVSNYLAWYQQKPGQAPRLLIYGASSRATGIPDRFSGSGSGTDFTLTISRLEPEDFAVYYCQQYGSSLWTFGQGTKVEIKRTVAAPSVFIFPPSDEQLKSGTASVVCLLNNFYPREAKVQWKVDNALQSGNSQESVTEQDSKDSTYSLSSTLTLSKADYEKHKVYACEVTHQGLSSPVTKSFNRGEC

SEQ ID NO: 337 - protein, 214 aa, synthetic construct
DIQMTQSPSSLPASVGDRVTITCRASQGIGTFLAWYQQHLGKAPKLLISASSTVQRGVPSRFSGSGSGTEFTLTINSLQPEDFATYYCQQLNNYPRTFGQGTKVEIKRTVAAPSVFIFPPSDEQLKSGTASVVCLLNNFYPREAKVQWKVDNALQSGNSQESVTEQDSKDSTYSLSSTLTLSKADYEKHKVYACEVTHQGLSSPVTKSFNRGEC

SEQ ID NO: 338 - protein, 214 aa, synthetic construct
EIVMTQSPGTLSLSPGQRATLSCRASQSVSSSSLAWYQQKPGQAPRLLIHGASSRATGIPDRFSGSGSGTDFTLTISRLEPEDFAVYYCQQYGTSWTFGQGTKVEIKRTVAAPSVFIFPPSDEQLKSGTASVVCLLNNFYPREAKVQWKVDNALQSGNSQESVTEQDSKDSTYSLSSTLTLSKADYEKHKVYACEVTHQGLSSPVTKSFNRGEC

SEQ ID NO: 339 - protein, 219 aa, synthetic construct
DVVMTQSPLSLPVTPGEPASISCRSSQSLLHRSGYNYLDWYVQKPGQSPQLLIYLGSIRAVGVPDRFSGSASGTDFTLRISRVEAEDVGIYYCMQALQTPPAFGGGTKVEIKRTVAAPSVFIFPPSDEQLKSGTASVVCLLNNFYPREAKVQWKVDNALQSGNSQESVTEQDSKDSTYSLSSTLTLSKADYEKHKVYACEVTHQGLSSPVTKSFNRGEC

SEQ ID NO: 340 - protein, 214 aa, synthetic construct
NIQLTQSPSSLSASVGDRVTITCRASQGINSWLAWYQQKPGKAPKLLIYAASTLQSGVPSRFSGSGSGTDFTLTINSLQPEDFATYYCQQLNSFPFTFGPGTKVHIKRTVAAPSVFIFPPSDEQLKSGTASVVCLLNNFYPREAKVQWKVDNALQSGNSQESVTEQDSKDSTYSLSSTLTLSKADYEKHKVYACEVTHQGLSSPVTKSFNRGEC

SEQ ID NO: 341 - protein, 214 aa, synthetic construct
DIQLTQSPSSLSASVGDRVTITCRASQSIDDHLNWYQQKPGKVPKLLISSASTLQSGAPSRFSGSGYGTDFTLTISSLQVEDFATYYCQQSYSPPQTFGQGTKVEIKRTVAAPSVFIFPPSDEQLKSGTASVVCLLNNFYPREAKVQWKVDNALQSGNSQESVTEQDSKDSTYSLSSTLTLSKADYEKHKVYACEVTHQGLSSPVTKSFNRGEC

SEQ ID NO: 342 - protein, 214 aa, synthetic construct
DIQLTQSPSSLSASVGDRVTITCRASQSISSYLNWYQQKPGKAPKLLIYAASSLQSGVPSRFSGSGSGTDFTLTISSLQPEDFATYYCQQSYSTPRTFGQGTRLEIKRTVAAPSVFIFPPSDEQLKSGTASVVCLLNNFYPREAKVQWKVDNALQSGNSQESVTEQDSKDSTYSLSSTLTLSKADYEKHKVYACEVTHQGLSSPVTKSFNRGEC

SEQ ID NO: 343 - protein, 219 aa, synthetic construct
DVVMTQSPLSLPVTLGQPASISCRSSQSLVYSDGNTYLNWFQQRPGQSPRRLIYKVSNRDSGVPDRFSGSGSGTDFTLKISRVEAEDVGVYYCMQGTHWPPTFGQGTKLEIKRTVAAPSVFIFPPSDEQLKSGTASVVCLLNNFYPREAKVQWKVDNALQSGNSQESVTEQDSKDSTYSLSSTLTLSKADYEKHKVYACEVTHQGLSSPVTKSFNRGEC

SEQ ID NO: 344 - protein, 214 aa, synthetic construct
DIQMTQSPSILSASVGDRVTLTCRASQSISSWLAWYQQTPGKAPRVLIYEASTLEVGVPSRFSGSGSGTDFTLTISSLQPEDFGTYFCQQYHTDSRTFGQGTILEIKRTVAAPSVFIFPPSDEQLKSGTASVVCLLNNFYPREAKVQWKVDNALQSGNSQESVTEQDSKDSTYSLSSTLTLSKADYEKHKVYACEVTHQGLSSPVTKSFNRGEC

SEQ ID NO: 345 - protein, 213 aa, synthetic construct
DIVMTQSPSSLSASVGDRVTITCRASQSISSYLNWYQQKPGKAPKLLIYAASSLQSGVPSRFSGSGSGTDFTLTISSLQPEDFATYYCQQSYSTLTFGGGTKVEIKRTVAAPSVFIFPPSDEQLKSGTASVVCLLNNFYPREAKVQWKVDNALQSGNSQESVTEQDSKDSTYSLSSTLTLSKADYEKHKVYACEVTHQGLSSPVTKSFNRGEC

SEQ ID NO: 346 - protein, 214 aa, synthetic construct
EIVLTQSPGTLSLSPGERATLSCRASQSVSKYLAWYQQKPGQAPRLLIYDVSNRATGIPARFSGSGSGTDFTLTISSLEPEDFAVYYCQQRRSWPLTFGGGTKVEIRRTVAAPSVFIFPPSDEQLKSGTASVVCLLNNFYPREAKVQWKVDNALQSGNSQESVTEQDSKDSTYSLSSTLTLSKADYEKHKVYACEVTHQGLSSPVTKSFNRGEC

SEQ ID NO: 347 - protein, 214 aa, synthetic construct
NIQLTQSPSSVSASVGDRVTISCRASQGIGRWLAWYQQKPGKAPKLLIYAASNLQSGVPSRFSGSGSGTDFTLTISSLQPEDFATYYCQQANSFPRTFGPGTKVDIKRTVAAPSVFIFPPSDEQLKSGTASVVCLLNNFYPREAKVQWKVDNALQSGNSQESVTEQDSKDSTYSLSSTLTLSKADYEKHKVYACEVTHQGLSSPVTKSFNRGEC

SEQ ID NO: 348 - protein, 214 aa, synthetic construct
NIQLTQSPSSLSASVGDRVTITCRASQGISTYLAWYQQKPGLAPKLLIYGASTLQSGVPSKFSGFGSGRDFTLTISSLQPEDIATYYCQQLNTYPPTFGQGTKLEIKRTVAAPSVFIFPPSDEQLKSGTASVVCLLNNFYPREAKVQWKVDNALQSGNSQESVTEQDSKDSTYSLSSTLTLSKADYEKHKVYACEVTHQGLSSPVTKSFNRGEC

SEQ ID NO: 349 - protein, 214 aa, synthetic construct
DIVMTQSPSSLSASVGDRVTITCQASQDISNYLNWYQQKPGKAPKLLIYDASSLESGVPSKFSGSRSGTDFTLTISSLQPEDSATYYCQQYRSYPITFGGGTKVEIKRTVAAPSVFIFPPSDEQLKSGTASVVCLLNNFYPREAKVQWKVDNALQSGNSQESVTEQDSKDSTYSLSSTLTLSKADYEKHKVYACEVTHQGLSSPVTKSFNRGEC

SEQ ID NO: 350 - protein, 214 aa, synthetic construct
DIQLTQSPSSLSASIGDRVTITCRASQGISSFLAWYQQKPGKAPQLLIYAASTLQSGVPSRFSGSGSGTEFTLTISSLQPEDFATYYCQQFKIYPLTFGGGTKVEVKRTVAAPSVFIFPPSDEQLKSGTASVVCLLNNFYPREAKVQWKVDNALQSGNSQESVTEQDSKDSTYSLSSTLTLSKADYEKHKVYACEVTHQGLSSPVTKSFNRGEC

SEQ ID NO: 351 - protein, 216 aa, synthetic construct; identical to SEQ ID NO: 332

SEQ ID NO: 352 - protein, 214 aa, synthetic construct
DIQLTQSPSFLSASVGDRVTITCRASQGISSQLAWYQQEPGKAPKLLIYAASTLQSGVPSRFSGSGSGTEFTLTISSLQPEDFATYYCQQVNAYPLTFGPGTKVDIKRTVAAPSVFIFPPSDEQLKSGTASVVCLLNNFYPREAKVQWKVDNALQSGNSQESVTEQDSKDSTYSLSSTLTLSKADYEKHKVYACEVTHQGLSSPVTKSFNRGEC

SEQ ID NO: 353 - protein, 20 aa, synthetic construct
MLLSPSLLLLLLLGAPRGCA

SEQ ID NO: 354 - DNA, 60 bp, synthetic construct
  source 1..60: mol_type = other DNA
atgctgctgtcgccgtcgctgctgctgctgctgctgctgggggcgccgcggggctgcgcc

SEQ ID NO: 355 - protein, 375 aa, synthetic construct
MLLSPSLLLLLLLGAPRGCAEGVAAALTPERLLEWQDKGIFVIQSESLKKCIQAGKSVLTLENCKQANKHMLWKWVSNHGLFNIGGSGCLGLNFSAPEQPLSLYECDSTLVSLRWRCNRKMITGPLQYSVQVAHDNTVVASRKYIHKWISYGSGGGDICEYLHKDLHTIKGNTHGMPCMFPFQYNHQWHHECTREGREDDLLWCATTSRYERDEKWGFCPDPTSAEVGCDTIWEKDLNSHICYQFNLLSSLSWSEAHSSCQMQGGTLLSITDETEENFIREHMSSKTVEVWMGLNQLDEHAGWQWSDGTPLNYLNWSPEVNFEPFVEDHCGTFSSFMPSAWRSRDCESTLPYICKKYLNHIDHEIVEGGHHHHHH

SEQ ID NO: 356 - DNA, 1125 bp, synthetic construct
  source 1..1125: mol_type = other DNA
atgctgctgtcgccgtcgctgctgctgctgctgctgctgggggcgccgcggggctgcgccgagggtgtggcggcggcgcttacccccgagcggctcctggagtggcaggataaaggaatatttgttatccaaagtgagagtctcaagaaatgcattcaagcaggtaaatcggttctgaccctggagaactgcaagcaagcaaacaagcacatgctgtggaaatgggtttcaaaccatggcctctttaacataggaggcagtggttgcctgggcctgaatttctccgccccagagcagccattaagcttatatgaatgtgactccaccctcgtttccttacggtggcgctgtaacaggaagatgatcacaggcccgctgcagtactctgtccaggtggcgcatgacaacacagtggtggcctcacggaagtatattcataagtggatttcttatgggtcaggtggtggagacatttgtgaatatctacacaaagatttgcatacaatcaaagggaacacccacgggatgccgtgtatgtttcccttccagtataaccatcagtggcatcatgaatgtacccgtgaaggtcgggaagatgacttactgtggtgtgccacgacaagccgttatgaaagagatgaaaagtggggattttgccctgatcccacctctgcagaagtaggttgtgatactatttgggagaaggacctcaattcacacatttgctaccagttcaacctgctttcatctctctcttggagtgaggcacattcttcatgccagatgcaaggaggtacgctgttaagtattacagatgaaactgaagaaaatttcataagggagcacatgagcagtaaaacagtggaggtgtggatgggcctcaatcagctggatgaacacgctggctggcagtggtctgatggaacgccgctcaactatctgaattggagcccagaggtaaattttgagccatttgttgaagatcactgtggaacatttagttcatttatgccaagtgcctggaggagtcgggattgtgagtccaccttgccatatatatgtaaaaaatatctaaaccacattgatcatgaaatagttgaaggaggtcatcaccatcaccatcac

SEQ ID NO: 357 - protein, 107 aa, synthetic construct [sequence omitted]

SEQ ID NO: 358 - protein, 452 aa, synthetic construct
QVQLQQSGPGLVKPSQTLSLTCTVSGGSISSGGYYWSWIRQHPGKGLEWIGYIYYSGSTYYNPSLKSRVTISVDTSKNQFSLKLSSVTAADTAVYYCARQRRANGYSSSWEFDYWGQGTLVTVSSASTKGPSVFPLAPCSRSTSESTAALGCLVKDYFPEPVTVSWNSGALTSGVHTFPAVLQSSGLYSLSSVVTVPSSSLGTKTYTCNVDHKPSNTKVDKRVESKYGPPCPPCPAPEFLGGPSVFLFPPKPKDTLMISRTPEVTCVVVDVSQEDPEVQFNWYVDGVEVHNAKTKPREEQFNSTYRVVSVLTVLHQDWLNGKEYKCKVSNKGLPSSIEKTISKAKGQPREPQVYTLPPSQEEMTKNQVSLTCLVKGFYPSDIAVEWESNGQPENNYKTTPPVLDSDGSFFLYSRLTVDKSRWQEGNVFSCSVMHEALHNHYTQKSLSLSLGK

SEQ ID NO: 359 - protein, 442 aa, synthetic construct
QVQLVQSGGGVVQPGNSLRLSCVASGFTFSRYTIHWVRQAPGKGLEWVAVISYDGSNKYYADSVKGRFTISRDNSKNTLYLQMNSLRAEDTAVYYCARGGPTPDWGQGTLVTVSSASTKGPSVFPLAPCSRSTSESTAALGCLVKDYFPEPVTVSWNSGALTSGVHTFPAVLQSSGLYSLSSVVTVPSSSLGTKTYTCNVDHKPSNTKVDKRVESKYGPPCPPCPAPEFLGGPSVFLFPPKPKDTLMISRTPEVTCVVVDVSQEDPEVQFNWYVDGVEVHNAKTKPREEQFNSTYRVVSVLTVLHQDWLNGKEYKCKVSNKGLPSSIEKTISKAKGQPREPQVYTLPPSQEEMTKNQVSLTCLVKGFYPSDIAVEWESNGQPENNYKTTPPVLDSDGSFFLYSRLTVDKSRWQEGNVFSCSVMHEALHNHYTQKSLSLSLGK

SEQ ID NO: 360 - protein, 448 aa, synthetic construct
QVQLLESGGGLVKPGGSLRLSCAASGFTFSSYSMNWVRQAPGKGLEWVSSISSGSSYIYYADSVKGRFTISRDNAKNSLYLQMNSLRAEDTAVYYCARDQGASVTGTHTHWGQGTLVTVSSASTKGPSVFPLAPCSRSTSESTAALGCLVKDYFPEPVTVSWNSGALTSGVHTFPAVLQSSGLYSLSSVVTVPSSSLGTKTYTCNVDHKPSNTKVDKRVESKYGPPCPPCPAPEFLGGPSVFLFPPKPKDTLMISRTPEVTCVVVDVSQEDPEVQFNWYVDGVEVHNAKTKPREEQFNSTYRVVSVLTVLHQDWLNGKEYKCKVSNKGLPSSIEKTISKAKGQPREPQVYTLPPSQEEMTKNQVSLTCLVKGFYPSDIAVEWESNGQPENNYKTTPPVLDSDGSFFLYSRLTVDKSRWQEGNVFSCSVMHEALHNHYTQKSLSLSLGK

SEQ ID NO: 361 - protein, 445 aa, synthetic construct
QVQLVQSGAEVKKPGSSVKVSCKASGGTFSSYTISWVRQAPGQGLEWMGRIIPILGIANYAQKFQGRVTITADKSTSTAYMELSSLRSEDTAVYYCATGVGMVRGDPWGQGTLVTVSSASTKGPSVFPLAPCSRSTSESTAALGCLVKDYFPEPVTVSWNSGALTSGVHTFPAVLQSSGLYSLSSVVTVPSSSLGTKTYTCNVDHKPSNTKVDKRVESKYGPPCPPCPAPEFLGGPSVFLFPPKPKDTLMISRTPEVTCVVVDVSQEDPEVQFNWYVDGVEVHNAKTKPREEQFNSTYRVVSVLTVLHQDWLNGKEYKCKVSNKGLPSSIEKTISKAKGQPREPQVYTLPPSQEEMTKNQVSLTCLVKGFYPSDIAVEWESNGQPENNYKTTPPVLDSDGSFFLYSRLTVDKSRWQEGNVFSCSVMHEALHNHYTQKSLSLSLGK

SEQ ID NO: 362 - protein, 453 aa, synthetic construct
RLQLQESGPGLVKPSQTLSLTCTVSGGSISSGGYYWSWIRQHPGKGLEWIGYIYYSGSTYYNPSLKSRVTISVDTSKNQFSLKLSSVTAADTAVYYCARIHHSTAGPYNNWYFDYWGQGTLVTVSSASTKGPSVFPLAPCSRSTSESTAALGCLVKDYFPEPVTVSWNSGALTSGVHTFPAVLQSSGLYSLSSVVTVPSSSLGTKTYTCNVDHKPSNTKVDKRVESKYGPPCPPCPAPEFLGGPSVFLFPPKPKDTLMISRTPEVTCVVVDVSQEDPEVQFNWYVDGVEVHNAKTKPREEQFNSTYRVVSVLTVLHQDWLNGKEYKCKVSNKGLPSSIEKTISKAKGQPREPQVYTLPPSQEEMTKNQVSLTCLVKGFYPSDIAVEWESNGQPENNYKTTPPVLDSDGSFFLYSRLTVDKSRWQEGNVFSCSVMHEALHNHYTQKSLSLSLGK

SEQ ID NO: 363 - protein, 446 aa, synthetic construct
QVQLLDSGGGLVKPGGSLRLSCAASGFTFSSYGMHWVRQAPGKGLEWVAFISNDGSNKYYADSVKGRFTISRDNSKNTLYLQMNSLRAEDTAVYYCARLLRGPWNFDLWGRGTLVTVSSASTKGPSVFPLAPCSRSTSESTAALGCLVKDYFPEPVTVSWNSGALTSGVHTFPAVLQSSGLYSLSSVVTVPSSSLGTKTYTCNVDHKPSNTKVDKRVESKYGPPCPPCPAPEFLGGPSVFLFPPKPKDTLMISRTPEVTCVVVDVSQEDPEVQFNWYVDGVEVHNAKTKPREEQFNSTYRVVSVLTVLHQDWLNGKEYKCKVSNKGLPSSIEKTISKAKGQPREPQVYTLPPSQEEMTKNQVSLTCLVKGFYPSDIAVEWESNGQPENNYKTTPPVLDSDGSFFLYSRLTVDKSRWQEGNVFSCSVMHEALHNHYTQKSLSLSLGK

SEQ ID NO: 364 - protein, 445 aa, synthetic construct; identical to SEQ ID NO: 361

SEQ ID NO: 365 - protein, 443 aa, synthetic construct
EVQLLESGGGLVKPGGSLRLSCAASGLIFKNYGMNWVRLAPGKGLEWVASISGNSNYISYADSVKGRFTISRDNANNSLFLQMSSLRADDTAVYYCSSGYFYFDLWGPGTLVTVSSASTKGPSVFPLAPCSRSTSESTAALGCLVKDYFPEPVTVSWNSGALTSGVHTFPAVLQSSGLYSLSSVVTVPSSSLGTKTYTCNVDHKPSNTKVDKRVESKYGPPCPPCPAPEFLGGPSVFLFPPKPKDTLMISRTPEVTCVVVDVSQEDPEVQFNWYVDGVEVHNAKTKPREEQFNSTYRVVSVLTVLHQDWLNGKEYKCKVSNKGLPSSIEKTISKAKGQPREPQVYTLPPSQEEMTKNQVSLTCLVKGFYPSDIAVEWESNGQPENNYKTTPPVLDSDGSFFLYSRLTVDKSRWQEGNVFSCSVMHEALHNHYTQKSLSLSLGK

SEQ ID NO: 366 - protein, 452 aa, synthetic construct; identical to SEQ ID NO: 358

SEQ ID NO: 367 - DNA, 1356 bp, synthetic construct
  source 1..1356: mol_type = other DNA
caggtacagctgcagcagtcgggcccaggactggtgaagccttcacagaccctgtccctcacctgcactgtctctggtggctccatcagcagtggtggttactactggagctggatccgccagcacccagggaagggcctggagtggattgggtacatctattacagtgggagcacctactacaacccgtccctcaagagtcgagttaccatatcagtagacacgtctaagaaccagttctccctgaagctgagctctgtgaccgccgcagacacggctgtgtattactgtgcgagacagaggcgtgccaacgggtatagcagcagctgggaatttgactactggggccagggcaccctggtcaccgtctcatcagcttccaccaagggccccagcgtgttccccctggccccttgttccaggagcacctccgagagcaccgccgctctgggctgcctggtgaaggactacttccctgagcctgtgaccgtgagctggaactccggcgctctgacctccggcgtgcacaccttccccgccgtgctgcagagcagcggcctgtacagcctgagctccgtggtgacagtgcccagctccagcctgggcaccaagacctacacctgcaatgtggatcacaagcccagcaataccaaggtggacaagagggtggagtccaagtacggccctccctgcccctcctgtcctgctcctgagttcctgggcggcccttccgtgttcctgttcccccccaagcccaaggataccctgatgatcagccggacccctgaggtgacatgtgtggtggtggatgtgagccaggaggaccctgaggtgcagttcaactggtacgtggatggcgtggaggtgcacaacgccaagaccaagcctcgggaggagcagttcaatagcacctaccgggtggtgagcgtgctgaccgtgctgcaccaggattggctgaacggcaaggagtacaagtgcaaggtgagcaacaagggcctgcccagcagcatcgagaagaccatctccaaggctaagggccagccacgggagcctcaggtgtacaccctgccccctagccaggaggagatgaccaagaaccaggtgagcctgacctgtctggtgaagggcttctacccctccgatatcgctgtggagtgggagtccaacggccagcccgagaacaactataagaccaccccccctgtgctggacagcgacggcagcttcttcctgtattccaggctgaccgtggacaagagccggtggcaggagggcaatgtgttctcctgcagcgtgatgcacgaggccctgcacaaccactacacccagaagtccctgtccctgtccctcggcaag

SEQ ID NO: 368 - DNA, 1326 bp, synthetic construct
  source 1..1326: mol_type = other DNA
caggtgcagctggtacagtctgggggaggcgtggtccagcctgggaactccctgagactctcctgtgtagcctctggattcaccttcagtaggtacaccatccactgggtccgccaggctccaggcaaggggctggagtgggtggcagttatatcatatgatggaagcaataaatactacgcagactccgtgaagggccgattcaccatctccagagacaattccaagaacacgctgtatctgcaaatgaacagcctgagagctgaggacacggctgtgtattactgtgcgagaggaggcccaactccagactggggccagggcaccctggtcaccgtctcatcagcttccaccaagggccccagcgtgttccccctggccccttgttccaggagcacctccgagagcaccgccgctctgggctgcctggtgaaggactacttccctgagcctgtgaccgtgagctggaactccggcgctctgacctccggcgtgcacaccttccccgccgtgctgcagagcagcggcctgtacagcctgagctccgtggtgacagtgcccagctccagcctgggcaccaagacctacacctgcaatgtggatcacaagcccagcaataccaaggtggacaagagggtggagtccaagtacggccctccctgcccctcctgtcctgctcctgagttcctgggcggcccttccgtgttcctgttcccccccaagcccaaggataccctgatgatcagccggacccctgaggtgacatgtgtggtggtggatgtgagccaggaggaccctgaggtgcagttcaactggtacgtggatggcgtggaggtgcacaacgccaagaccaagcctcgggaggagcagttcaatagcacctaccgggtggtgagcgtgctgaccgtgctgcaccaggattggctgaacggcaaggagtacaagtgcaaggtgagcaacaagggcctgcccagcagcatcgagaagaccatctccaaggctaagggccagccacgggagcctcaggtgtacaccctgccccctagccaggaggagatgaccaagaaccaggtgagcctgacctgtctggtgaagggcttctacccctccgatatcgctgtggagtgggagtccaacggccagcccgagaacaactataagaccaccccccctgtgctggacagcgacggcagcttcttcctgtattccaggctgaccgtggacaagagccggtggcaggagggcaatgtgttctcctgcagcgtgatgcacgaggccctgcacaaccactacacccagaagtccctgtccctgtccctcggcaag

SEQ ID NO: 369 - DNA, 1347 bp, synthetic construct
  source 1..1347: mol_type = other DNA
caggttcagctggtacagtctggggctgaggtgaagaagcctgggtcctcggtgaaggtctcctgcaaggcttctggaggcaccttcagcagctatgctatcagctgggtgcgacaggcccctggacaagggcttgagtggatgggagggatcatccctatctttggtacagcaaactacgcacagaagttccagggcagagtcaccatgaccagggacacgtccacgagcacagtctacatggagctgagcagcctgagatctgaggacacggccgtgtattactgtgcgagagattcggatttttggagtggttattcatcaatggacgtctggggccaagggaccacggtcaccgtctcatcagcttccaccaagggccccagcgtgttccccctggccccttgttccaggagcacctccgagagcaccgccgctctgggctgcctggtgaaggactacttccctgagcctgtgaccgtgagctggaactccggcgctctgacctccggcgtgcacaccttccccgccgtgctgcagagcagcggcctgtacagcctgagctccgtggtgacagtgcccagctccagcctgggcaccaagacctacacctgcaatgtggatcacaagcccagcaataccaaggtggacaagagggtggagtccaagtacggccctccctgcccctcctgtcctgctcctgagttcctgggcggcccttccgtgttcctgttcccccccaagcccaaggataccctgatgatcagccggacccctgaggtgacatgtgtggtggtggatgtgagccaggaggaccctgaggtgcagttcaactggtacgtggatggcgtggaggtgcacaacgccaagaccaagcctcgggaggagcagttcaatagcacctaccgggtggtgagcgtgctgaccgtgctgcaccaggattggctgaacggcaaggagtacaagtgcaaggtgagcaacaagggcctgcccagcagcatcgagaagaccatctccaaggctaagggccagccacgggagcctcaggtgtacaccctgccccctagccaggaggagatgaccaagaaccaggtgagcctgacctgtctggtgaagggcttctacccctccgatatcgctgtggagtgggagtccaacggccagcccgagaacaactataagaccaccccccctgtgctggacagcgacggcagcttcttcctgtattccaggctgaccgtggacaagagccggtggcaggagggcaatgtgttctcctgcagcgtgatgcacgaggccctgcacaaccactacacccagaagtccctgtccctgtccctcggcaag

SEQ ID NO: 370 - DNA, 1344 bp, synthetic construct
  source 1..1344: mol_type = other DNA
caggtgcagctgttggagtctgggggaggcctggtcaagcctggggggtccctgagactctcctgtgcagcctctggattcaccttcagtagctatagcatgaactgggtccgccaggctccagggaaggggctggagtgggtctcatccattagtagtggtagtagttacatatactacgcagactcagtgaagggccgattcaccatctccagagacaacgccaagaactcactgtatctgcaaatgaacagcctgagagccgaggacacggctgtgtattactgtgcgagagatcaaggggcgtccgtaactggaacccacacccactggggccagggaaccctggtcaccgtctcatcagcttccaccaagggccccagcgtgttccccctggccccttgttccaggagcacctccgagagcaccgccgctctgggctgcctggtgaaggactacttccctgagcctgtgaccgtgagctggaactccggcgctctgacctccggcgtgcacaccttccccgccgtgctgcagagcagcggcctgtacagcctgagctccgtggtgacagtgcccagctccagcctgggcaccaagacctacacctgcaatgtggatcacaagcccagcaataccaaggtggacaagagggtggagtccaagtacggccctccctgcccctcctgtcctgctcctgagttcctgggcggcccttccgtgttcctgttcccccccaagcccaaggataccctgatgatcagccggacccctgaggtgacatgtgtggtggtggatgtgagccaggaggaccctgaggtgcagttcaactggtacgtggatggcgtggaggtgcacaacgccaagaccaagcctcgggaggagcagttcaatagcacctaccgggtggtgagcgtgctgaccgtgctgcaccaggattggctgaacggcaaggagtacaagtgcaaggtgagcaacaagggcctgcccagcagcatcgagaagaccatctccaaggctaagggccagccacgggagcctcaggtgtacaccctgccccctagccaggaggagatgaccaagaaccaggtgagcctgacctgtctggtgaagggcttctacccctccgatatcgctgtggagtgggagtccaacggccagcccgagaacaactataagaccaccccccctgtgctggacagcgacggcagcttcttcctgtattccaggctgaccgtggacaagagccggtggcaggagggcaatgtgttctcctgcagcgtgatgcacgaggccctgcacaaccactacacccagaagtccctgtccctgtccctcggcaag

SEQ ID NO: 371 - DNA, 1338 bp, synthetic construct
  source 1..1338: mol_type = other DNA
gaggtgcatctggtggagtctgggcctgagctggtgaggcctggggcttcagtgacgctgtcctgcaaggcttcgggctacacatttactgactatgaaatgcactgggtgaagcagacacctgtgcatggcctggaatggattggagctattgatcctgaaactggtggtactgcctacaatcagaagttcaagggcaaggccacactgactgcagacaaatcctccagcacagcctacatggagctccgcagcctgacatctgaggactctgccgtctattactgtacaaccacttatggtaactactggtacttcgatgtctggggcgcaggaaccctggtcaccgtctcatcagcttccaccaagggccccagcgtgttccccctggccccttgttccaggagcacctccgagagcaccgccgctctgggctgcctggtgaaggactacttccctgagcctgtgaccgtgagctggaactccggcgctctgacctccggcgtgcacaccttccccgccgtgctgcagagcagcggcctgtacagcctgagctccgtggtgacagtgcccagctccagcctgggcaccaagacctacacctgcaatgtggatcacaagcccagcaataccaaggtggacaagagggtggagtccaagtacggccctccctgcccctcctgtcctgctcctgagttcctgggcggcccttccgtgttcctgttcccccccaagcccaaggataccctgatgatcagccggacccctgaggtgacatgtgtggtggtggatgtgagccaggaggaccctgaggtgcagttcaactggtacgtggatggcgtggaggtgcacaacgccaagaccaagcctcgggaggagcagttcaatagcacctaccgggtggtgagcgtgctgaccgtgctgcaccaggattggctgaacggcaaggagtacaagtgcaaggtgagcaacaagggcctgcccagcagcatcgagaagaccatctccaaggctaagggccagccacgggagcctcaggtgtacaccctgccccctagccaggaggagatgaccaagaaccaggtgagcctgacctgtctggtgaagggcttctacccctccgatatcgctgtggagtgggagtccaacggccagcccgagaacaactataagaccaccccccctgtgctggacagcgacggcagcttcttcctgtattccaggctgaccgtggacaagagccggtggcaggagggcaatgtgttctcctgcagcgtgatgcacgaggccctgcacaaccactacacccagaagtccctgtccctgtccctcggcaag

SEQ ID NO: 372 - DNA, 1338 bp, synthetic construct
  source 1..1338: mol_type = other DNA
gaagtgcagctggtggagtctggggctgaggtgaagaagcctgggtcctcggtgaaggtctcctgcaaggcttctggaggcaccttcagcagctatgctatcagctgggtgcgacaggcccctggacaagggcttgagtggatgggagggatcatccctatctttggtacagcaaactacgcacagaagttccagggcagagtcacgattaccgcggacgaatccacgagcacagcctacatggagctgagcagcctgagatctgaggacacggccgtgtattactgtgcgttcaccagtgggagctactactactttgactactggggccagggcaccctggtcaccgtctcatcagcttccaccaagggccccagcgtgttccccctggccccttgttccaggagcacctccgagagcaccgccgctctgggctgcctggtgaaggactacttccctgagcctgtgaccgtgagctggaactccggcgctctgacctccggcgtgcacaccttccccgccgtgctgcagagcagcggcctgtacagcctgagctccgtggtgacagtgcccagctccagcctgggcaccaagacctacacctgcaatgtggatcacaagcccagcaataccaaggtggacaagagggtggagtccaagtacggccctccctgcccctcctgtcctgctcctgagttcctgggcggcccttccgtgttcctgttcccccccaagcccaaggataccctgatgatcagccggacccctgaggtgacatgtgtggtggtggatgtgagccaggaggaccctgaggtgcagttcaactggtacgtggatggcgtggaggtgcacaacgccaagaccaagcctcgggaggagcagttcaatagcacctaccgggtggtgagcgtgctgaccgtgctgcaccaggattggctgaacggcaaggagtacaagtgcaaggtgagcaacaagggcctgcccagcagcatcgagaagaccatctccaaggctaagggccagccacgggagcctcaggtgtacaccctgccccctagccaggaggagatgaccaagaaccaggtgagcctgacctgtctggtgaagggcttctacccctccgatatcgctgtggagtgggagtccaacggccagcccgagaacaactataagaccaccccccctgtgctggacagcgacggcagcttcttcctgtattccaggctgaccgtggacaagagccggtggcaggagggcaatgtgttctcctgcagcgtgatgcacgaggccctgcacaaccactacacccagaagtccctgtccctgtccctcggcaag

SEQ ID NO: 373 - DNA, 1338 bp, synthetic construct
  source 1..1338: mol_type = other DNA
caggtccagcttgtgcaatctggggctgaggtgaagaagcctgggtcctcggtgaaggtctcctgcaaggcttctggaggcaccttcagcagctatgctatcagctgggtgcgacaggcccctggacaagggcttgagtggatgggagggatcatccctatctttggtacagcaaactacgcacagaagttccagggcagagtcacgattaccgcggacgaatccacgagcacagcctacatggagctgagcagcctgagatctgaggacacggccgtgtattactgtgcgagagggggaggggggaggggtatgacgagcgactggggccagggaaccctggtcaccgtctcatcagcttccaccaagggccccagcgtgttccccctggccccttgttccaggagcacctccgagagcaccgccgctctgggctgcctggtgaaggactacttccctgagcctgtgaccgtgagctggaactccggcgctctgacctccggcgtgcacaccttccccgccgtgctgcagagcagcggcctgtacagcctgagctccgtggtgacagtgcccagctccagcctgggcaccaagacctacacctgcaatgtggatcacaagcccagcaataccaaggtggacaagagggtggagtccaagtacggccctccctgcccctcctgtcctgctcctgagttcctgggcggcccttccgtgttcctgttcccccccaagcccaaggataccctgatgatcagccggacccctgaggtgacatgtgtggtggtggatgtgagccaggaggaccctgaggtgcagttcaactggtacgtggatggcgtggaggtgcacaacgccaagaccaagcctcgggaggagcagttcaatagcacctaccgggtggtgagcgtgctgaccgtgctgcaccaggattggctgaacggcaaggagtacaagtgcaaggtgagcaacaagggcctgcccagcagcatcgagaagaccatctccaaggctaagggccagccacgggagcctcaggtgtacaccctgccccctagccaggaggagatgaccaagaaccaggtgagcctgacctgtctggtgaagggcttctacccctccgatatcgctgtggagtgggagtccaacggccagcccgagaacaactataagaccaccccccctgtgctggacagcgacggcagcttcttcctgtattccaggctgaccgtggacaagagccggtggcaggagggcaatgtgttctcctgcagcgtgatgcacgaggccctgcacaaccactacacccagaagtccctgtccctgtccctcggcaag

SEQ ID NO: 374 - DNA, 1362 bp, synthetic construct
  source 1..1362: mol_type = other DNA
caggtgcagctgttggagtctgggggaggcttggtacagcctggggggtccctgagactctcctgtgcagcctctggattcacctttagcagctatgccatgagctgggtccgccaggctccagggaaggggctggagtgggtctcagctattagtggtagtggtggtagcacatactacgcagactccgtgaagggccggttcaccatctccagagacaattccaagaacacgctgtatctgcaaatgaacagcctgagagccgaggacacggccgtatattactgtgcgaaaggaacgaagatggctacaatccgcctcggctactactactacggtatggacgtctggggccaagggacaatggtcaccgtctcatcagcttccaccaagggccccagcgtgttccccctggccccttgttccaggagcacctccgagagcaccgccgctctgggctgcctggtgaaggactacttccctgagcctgtgaccgtgagctggaactccggcgctctgacctccggcgtgcacaccttccccgccgtgctgcagagcagcggcctgtacagcctgagctccgtggtgacagtgcccagctccagcctgggcaccaagacctacacctgcaatgtggatcacaagcccagcaataccaaggtggacaagagggtggagtccaagtacggccctccctgcccctcctgtcctgctcctgagttcctgggcggcccttccgtgttcctgttcccccccaagcccaaggataccctgatgatcagccggacccctgaggtgacatgtgtggtggtggatgtgagccaggaggaccctgaggtgcagttcaactggtacgtggatggcgtggaggtgcacaacgccaagaccaagcctcgggaggagcagttcaatagcacctaccgggtggtgagcgtgctgaccgtgctgcaccaggattggctgaacggcaaggagtacaagtgcaaggtgagcaacaagggcctgcccagcagcatcgagaagaccatctccaaggctaagggccagccacgggagcctcaggtgtacaccctgccccctagccaggaggagatgaccaagaaccaggtgagcctgacctgtctggtgaagggcttctacccctccgatatcgctgtggagtgggagtccaacggccagcccgagaacaactataagaccaccccccctgtgctggacagcgacggcagcttcttcctgtattccaggctgaccgtggacaagagccggtggcaggagggcaatgtgttctcctgcagcgtgatgcacgaggccctgcacaaccactacacccagaagtccctgtccctgtccctcggcaag

SEQ ID NO: 375 - DNA, 1347 bp, synthetic construct
  source 1..1347: mol_type = other DNA
caggtacagctgcaggagtcgggcccaggactggtgaagccttcacagaccctgtccctcacctgcactgtctctggtggctccatcagcagtggtggttactactggagctggatccgccagcacccagggaagggcctggagtggattgggtacatctattacagtgggagcacctactacaacccgtccctcaagagtcgagttaccatatcagtagacacgtctaagaaccagttctccctgaagctgagctctgtgactgccgcggacacggccgtgtattactgtgcgagatgggggcgagggggcagcagctggcggtttgatatctggggccaagggacaatggtcaccgtctcatcagcttccaccaagggccccagcgtgttccccctggccccttgttccaggagcacctccgagagcaccgccgctctgggctgcctggtgaaggactacttccctgagcctgtgaccgtgagctggaactccggcgctctgacctccggcgtgcacaccttccccgccgtgctgcagagcagcggcctgtacagcctgagctccgtggtgacagtgcccagctccagcctgggcaccaagacctacacctgcaatgtggatcacaagcccagcaataccaaggtggacaagagggtggagtccaagtacggccctccctgcccctcctgtcctgctcctgagttcctgggcggcccttccgtgttcctgttcccccccaagcccaaggataccctgatgatcagccggacccctgaggtgacatgtgtggtggtggatgtgagccaggaggaccctgaggtgcagttcaactggtacgtggatggcgtggaggtgcacaacgccaagaccaagcctcgggaggagcagttcaatagcacctaccgggtggtgagcgtgctgaccgtgctgcaccaggattggctgaacggcaaggagtacaagtgcaaggtgagcaacaagggcctgcccagcagcatcgagaagaccatctccaaggctaagggccagccacgggagcctcaggtgtacaccctgccccctagccaggaggagatgaccaagaaccaggtgagcctgacctgtctggtgaagggcttctacccctccgatatcgctgtggagtgggagtccaacggccagcccgagaacaactataagaccaccccccctgtgctggacagcgacggcagcttcttcctgtattccaggctgaccgtggacaagagccggtggcaggagggcaatgtgttctcctgcagcgtgatgcacgaggccctgcacaaccactacacccagaagtccctgtccctgtccctcggcaag

SEQ ID NO: 376 - DNA, 1344 bp, synthetic construct
  source 1..1344: mol_type = other DNA
gaggtgcagctgttggagtctggcccaggactggtgaagccttcacagaccctgtccctcacctgcactgtctctggtggctccatcagcagtggtggttactactggagctggatccgccagcacccagggaagggcctggagtggattgggtacatctattacagtgggagcacctactacaacccgtccctcaagagtcgagttaccatatcagtagacacgtctaagaaccagttctccctgaagctgagctctgtgactgccgcggacacggccgtgtattactgtgcgagagattcgagggggcgaagctacggtatggacgtctggggccaagggacaatggtcaccgtctcatcagcttccaccaagggccccagcgtgttccccctggccccttgttccaggagcacctccgagagcaccgccgctctgggctgcctggtgaaggactacttccctgagcctgtgaccgtgagctggaactccggcgctctgacctccggcgtgcacaccttccccgccgtgctgcagagcagcggcctgtacagcctgagctccgtggtgacagtgcccagctccagcctgggcaccaagacctacacctgcaatgtggatcacaagcccagcaataccaaggtggacaagagggtggagtccaagtacggccctccctgcccctcctgtcctgctcctgagttcctgggcggcccttccgtgttcctgttcccccccaagcccaaggataccctgatgatcagccggacccctgaggtgacatgtgtggtggtggatgtgagccaggaggaccctgaggtgcagttcaactggtacgtggatggcgtggaggtgcacaacgccaagaccaagcctcgggaggagcagttcaatagcacctaccgggtggtgagcgtgctgaccgtgctgcaccaggattggctgaacggcaaggagtacaagtgcaaggtgagcaacaagggcctgcccagcagcatcgagaagaccatctccaaggctaagggccagccacgggagcctcaggtgtacaccctgccccctagccaggaggagatgaccaagaaccaggtgagcctgacctgtctggtgaagggcttctacccctccgatatcgctgtggagtgggagtccaacggccagcccgagaacaactataagaccaccccccctgtgctggacagcgacggcagcttcttcctgtattccaggctgaccgtggacaagagccggtggcaggagggcaatgtgttctcctgcagcgtgatgcacgaggccctgcacaaccactacacccagaagtccctgtccctgtccctcggcaag

SEQ ID NO: 377 - DNA, 1335 bp, synthetic construct
  source 1..1335: mol_type = other DNA
caggtgcagctggtgcaatctggggctgaggtgaagaagcctgggtcctcggtgaaggtctcctgcaaggcttctggaggcaccttcagcagctatactatcagctgggtgcgacaggcccctggacaagggcttgagtggatgggaaggatcatccctatccttggtatagcaaactacgcacagaagttccagggcagagtcacgattaccgcggacaaatccacgagcacagcctacatggagctgagcagcctgagatctgaggacacggccgtgtattactgtgcgacgggggttggtatggttcggggagacccttggggccagggaaccctggtcaccgtctcatcagcttccaccaagggccccagcgtgttccccctggccccttgttccaggagcacctccgagagcaccgccgctctgggctgcctggtgaaggactacttccctgagcctgtgaccgtgagctggaactccggcgctctgacctccggcgtgcacaccttccccgccgtgctgcagagcagcggcctgtacagcctgagctccgtggtgacagtgcccagctccagcctgggcaccaagacctacacctgcaatgtggatcacaagcccagcaataccaaggtggacaagagggtggagtccaagtacggccctccctgcccctcctgtcctgctcctgagttcctgggcggcccttccgtgttcctgttcccccccaagcccaaggataccctgatgatcagccggacccctgaggtgacatgtgtggtggtggatgtgagccaggaggaccctgaggtgcagttcaactggtacgtggatggcgtggaggtgcacaacgccaagaccaagcctcgggaggagcagttcaatagcacctaccgggtggtgagcgtgctgaccgtgctgcaccaggattggctgaacggcaaggagtacaagtgcaaggtgagcaacaagggcctgcccagcagcatcgagaagaccatctccaaggctaagggccagccacgggagcctcaggtgtacaccctgccccctagccaggaggagatgaccaagaaccaggtgagcctgacctgtctggtgaagggcttctacccctccgatatcgctgtggagtgggagtccaacggccagcccgagaacaactataagaccaccccccctgtgctggacagcgacggcagcttcttcctgtattccaggctgaccgtggacaagagccggtggcaggagggcaatgtgttctcctgcagcgtgatgcacgaggccctgcacaaccactacacccagaagtccctgtccctgtccctcggcaag

SEQ ID NO: 378 - DNA, 1341 bp, synthetic construct
  source 1..1341: mol_type = other DNA
caggtgcagctggtgcaatctgggggaggcgtggtccagcctgggaggtccctgagactcccctgtgcagcctctggattcaccttcagtaattatgctatgcactgggtccgccaggctccaggcaaggggctggagtgggtggcagttatatcatatgatggaagtaagaaatactacgcagactccgtgaagggccgattcaccatctccagagacaattccaagaacacgctgtatctgcaagtgaacagcctgagagctgaggacacggctgtgtattactgtgcgaccggttatagcagtccctggtacggtatggacgtctggggccaagggaccacggtcaccgtctcatcagcttccaccaagggccccagcgtgttccccctggccccttgttccaggagcacctccgagagcaccgccgctctgggctgcctggtgaaggactacttccctgagcctgtgaccgtgagctggaactccggcgctctgacctccggcgtgcacaccttccccgccgtgctgcagagcagcggcctgtacagcctgagctccgtggtgacagtgcccagctccagcctgggcaccaagacctacacctgcaatgtggatcacaagcccagcaataccaaggtggacaagagggtggagtccaagtacggccctccctgcccctcctgtcctgctcctgagttcctgggcggcccttccgtgttcctgttcccccccaagcccaaggataccctgatgatcagccggacccctgaggtgacatgtgtggtggtggatgtgagccaggaggaccctgaggtgcagttcaactggtacgtggatggcgtggaggtgcacaacgccaagaccaagcctcgggaggagcagttcaatagcacctaccgggtggtgagcgtgctgaccgtgctgcaccaggattggctgaacggcaaggagtacaagtgcaaggtgagcaacaagggcctgcccagcagcatcgagaagaccatctccaaggctaagggccagccacgggagcctcaggtgtacaccctgccccctagccaggaggagatgaccaagaaccaggtgagcctgacctgtctggtgaagggcttctacccctccgatatcgctgtggagtgggagtccaacggccagcccgagaacaactataagaccaccccccctgtgctggacagcgacggcagcttcttcctgtattccaggctgaccgtggacaagagccggtggcaggagggcaatgtgttctcctgcagcgtgatgcacgaggccctgcacaaccactacacccagaagtccctgtccctgtccctcggcaag

SEQ ID NO: 379 - DNA, 1335 bp, synthetic construct
  source 1..1335: mol_type = other DNA
gaggtgcagctggtggagactgggggaggcgtggtccagcctgggaggtccctgagactctcctgtgcagcctctggattcaccttcagtagctatgctatgcactgggtccgccaggctccaggcaaggggctggagtgggtggcagttatatcatatgatggaagtaataaatactacgcagactccgtgaagggccgattcaccatctccagagacaattccaagaacacgctgtatctgcaaatgaacagcctgagagctgaggacacggctgtgtattactgtgcgagagccgcaggtcacgggattttagactactggggccagggaaccctggtcaccgtctcatcagcttccaccaagggccccagcgtgttccccctggccccttgttccaggagcacctccgagagcaccgccgctctgggctgcctggtgaaggactacttccctgagcctgtgaccgtgagctggaactccggcgctctgacctccggcgtgcacaccttccccgccgtgctgcagagcagcggcctgtacagcctgagctccgtggtgacagtgcccagctccagcctgggcaccaagacctacacctgcaatgtggatcacaagcccagcaataccaaggtggacaagagggtggagtccaagtacggccctccctgcccctcctgtcctgctcctgagttcctgggcggcccttccgtgttcctgttcccccccaagcccaaggataccctgatgatcagccggacccctgaggtgacatgtgtggtggtggatgtgagccaggaggaccctgaggtgcagttcaactggtacgtggatggcgtggaggtgcacaacgccaagaccaagcctcgggaggagcagttcaatagcacctaccgggtggtgagcgtgctgaccgtgctgcaccaggattggctgaacggcaaggagtacaagtgcaaggtgagcaacaagggcctgcccagcagcatcgagaagaccatctccaaggctaagggccagccacgggagcctcaggtgtacaccctgccccctagccaggaggagatgaccaagaaccaggtgagcctgacctgtctggtgaagggcttctacccctccgatatcgctgtggagtgggagtccaacggccagcccgagaacaactataagaccaccccccctgtgctggacagcgacggcagcttcttcctgtattccaggctgaccgtggacaagagccggtggcaggagggcaatgtgttctcctgcagcgtgatgcacgaggccctgcacaaccactacacccagaagtccctgtccctgtccctcggcaag

SEQ ID NO: 380 - DNA, 1359 bp, synthetic construct
  source 1..1359: mol_type = other DNA
cggctgcagctgcaggagtcgggcccaggactggtgaagccttcacagaccctgtccctcacctgcactgtctctggtggctccatcagcagtggtggttactactggagctggatccgccagcacccagggaagggcctggagtggattgggtacatctattacagtgggagcacctactacaacccgtccctcaagagtcgagttaccatatcagtagacacgtctaagaaccagttctccctgaagctgagctctgtgactgccgcggacacggccgtgtattactgtgcgaggattcaccatagtaccgcggggccatacaacaactggtactttgactactggggccagggaaccctggtcaccgtctcatcagcttccaccaagggccccagcgtgttccccctggccccttgttccaggagcacctccgagagcaccgccgctctgggctgcctggtgaaggactacttccctgagcctgtgaccgtgagctggaactccggcgctctgacctccggcgtgcacaccttccccgccgtgctgcagagcagcggcctgtacagcctgagctccgtggtgacagtgcccagctccagcctgggcaccaagacctacacctgcaatgtggatcacaagcccagcaataccaaggtggacaagagggtggagtccaagtacggccctccctgcccctcctgtcctgctcctgagttcctgggcggcccttccgtgttcctgttcccccccaagcccaaggataccctgatgatcagccggacccctgaggtgacatgtgtggtggtggatgtgagccaggaggaccctgaggtgcagttcaactggtacgtggatggcgtggaggtgcacaacgccaagaccaagcctcgggaggagcagttcaatagcacctaccgggtggtgagcgtgctgaccgtgctgcaccaggattggctgaacggcaaggagtacaagtgcaaggtgagcaacaagggcctgcccagcagcatcgagaagaccatctccaaggctaagggccagccacgggagcctcaggtgtacaccctgccccctagccaggaggagatgaccaagaaccaggtgagcctgacctgtctggtgaagggcttctacccctccgatatcgctgtggagtgggagtccaacggccagcccgagaacaactataagaccaccccccctgtgctggacagcgacggcagcttcttcctgtattccaggctgaccgtggacaagagccggtggcaggagggcaatgtgttctcctgcagcgtgatgcacgaggccctgcacaaccactacacccagaagtccctgtccctgtccctcggcaag

SEQ ID NO: 381 - DNA, 1338 bp, synthetic construct
  source 1..1338: mol_type = other DNA
caggtgcagctgttggactctgggggaggcttggtcaagcctggagggtccctgagactctcctgtgcagcctctggattcaccttcagtagttatggcatgcactgggtccgccaggctccaggcaaggggctggagtgggtggcatttatatcaaatgatggaagtaataaatactatgcagactccgtgaagggccgattcaccatctccagagacaattccaagaacacgttgtatctgcaaatgaacagcctgagagctgaggacacggctgtgtattactgtgcgagacttctccgtggaccctggaacttcgatctctggggccgtggcaccctggtcaccgtctcatcagcttccaccaagggccccagcgtgttccccctggccccttgttccaggagcacctccgagagcaccgccgctctgggctgcctggtgaaggactacttccctgagcctgtgaccgtgagctggaactccggcgctctgacctccggcgtgcacaccttccccgccgtgctgcagagcagcggcctgtacagcctgagctccgtggtgacagtgcccagctccagcctgggcaccaagacctacacctgcaatgtggatcacaagcccagcaataccaaggtggacaagagggtggagtccaagtacggccctccctgcccctcctgtcctgctcctgagttcctgggcggcccttccgtgttcctgttcccccccaagcccaaggataccctgatgatcagccggacccctgaggtgacatgtgtggtggtggatgtgagccaggaggaccctgaggtgcagttcaactggtacgtggatggcgtggaggtgcacaacgccaagaccaagcctcgggaggagcagttcaatagcacctaccgggtggtgagcgtgctgaccgtgctgcaccaggattggctgaacggcaaggagtacaagtgcaaggtgagcaacaagggcctgcccagcagcatcgagaagaccatctccaaggctaagggccagccacgggagcctcaggtgtacaccctgccccctagccaggaggagatgaccaagaaccaggtgagcctgacctgtctggtgaagggcttctacccctccgatatcgctgtggagtgggagtccaacggccagcccgagaacaactataagaccaccccccctgtgctggacagcgacggcagcttcttcctgtattccaggctgaccgtggacaagagccggtggcaggagggcaatgtgttctcctgcagcgtgatgcacgaggccctgcacaaccactacacccagaagtccctgtccctgtccctcggcaag

SEQ ID NO: 382 - DNA, 1341 bp, synthetic construct
  source 1..1341: mol_type = other DNA
gaggtgcagctgttggagtctgggggaggcttggtacagcctggggggtccctgagactctcctgtgcagcctctggattcacctttagcagctatgccatgagctgggtccgccaggctccagggaaggggctggagtgggtctcagctattagtggtagtggtggtagcacatactacgcagactccgtgaagggccggttcaccatctccagagacaattccaagaacacgctgtatctgcaaatgaacagcctgagagccgaggacacggccgtatattactgtgcgactagtagtggccctagaattgatgcttttgatatctggggccaagggacaatggtcaccgtctcatcagcttccaccaagggccccagcgtgttccccctggccccttgttccaggagcacctccgagagcaccgccgctctgggctgcctggtgaaggactacttccctgagcctgtgaccgtgagctggaactccggcgctctgacctccggcgtgcacaccttccccgccgtgctgcagagcagcggcctgtacagcctgagctccgtggtgacagtgcccagctccagcctgggcaccaagacctacacctgcaatgtggatcacaagcccagcaataccaaggtggacaagagggtggagtccaagtacggccctccctgcccctcctgtcctgctcctgagttcctgggcggcccttccgtgttcctgttcccccccaagcccaaggataccctgatgatcagccggacccctgaggtgacatgtgtggtggtggatgtgagccaggaggaccctgaggtgcagttcaactggtacgtggatggcgtggaggtgcacaacgccaagaccaagcctcgggaggagcagttcaatagcacctaccgggtggtgagcgtgctgaccgtgctgcaccaggattggctgaacggcaaggagtacaagtgcaaggtgagcaacaagggcctgcccagcagcatcgagaagaccatctccaaggctaagggccagccacgggagcctcaggtgtacaccctgccccctagccaggaggagatgaccaagaaccaggtgagcctgacctgtctggtgaagggcttctacccctccgatatcgctgtggagtgggagtccaacggccagcccgagaacaactataagaccaccccccctgtgctggacagcgacggcagcttcttcctgtattccaggctgaccgtggacaagagccggtggcaggagggcaatgtgttctcctgcagcgtgatgcacgaggccctgcacaaccactacacccagaagtccctgtccctgtccctcggcaag

SEQ ID NO: 383 - DNA, 1335 bp, synthetic construct
  source 1..1335: mol_type = other DNA
caggtgcagctggtacagtctggggctgaggtgaagaagcctggggcctcagtgaaggtttcctgcaaggcttctggatacaccttcactagctatgctatgcattgggtgcgccaggcccccggacaaaggcttgagtggatgggatggatcaacgctggcaatggtaacacaaaatattcacagaagttccagggcagagtcaccattaccagggacacatccgcgagcacagcctacatggagctgagcagcctgagatctgaagacacggctgtgtattactgtgcgaccagtaagtcggtctggaattttgactactggggccagggaaccctggtcaccgtctcatcagcttccaccaagggccccagcgtgttccccctggccccttgttccaggagcacctccgagagcaccgccgctctgggctgcctggtgaaggactacttccctgagcctgtgaccgtgagctggaactccggcgctctgacctccggcgtgcacaccttccccgccgtgctgcagagcagcggcctgtacagcctgagctccgtggtgacagtgcccagctccagcctgggcaccaagacctacacctgcaatgtggatcacaagcccagcaataccaaggtggacaagagggtggagtccaagtacggccctccctgcccctcctgtcctgctcctgagttcctgggcggcccttccgtgttcctgttcccccccaagcccaaggataccctgatgatcagccggacccctgaggtgacatgtgtggtggtggatgtgagccaggaggaccctgaggtgcagttcaactggtacgtggatggcgtggaggtgcacaacgccaagaccaagcctcgggaggagcagttcaatagcacctaccgggtggtgagcgtgctgaccgtgctgcaccaggattggctgaacggcaaggagtacaagtgcaaggtgagcaacaagggcctgcccagcagcatcgagaagaccatctccaaggctaagggccagccacgggagcctcaggtgtacaccctgccccctagccaggaggagatgaccaagaaccaggtgagcctgacctgtctggtgaagggcttctacccctccgatatcgctgtggagtgggagtccaacggccagcccgagaacaactataagaccaccccccctgtgctggacagcgacggcagcttcttcctgtattccaggctgaccgtggacaagagccggtggcaggagggcaatgtgttctcctgcagcgtgatgcacgaggccctgcacaaccactacacccagaagtccctgtccctgtccctcggcaag

SEQ ID NO: 384 - DNA, 1332 bp, synthetic construct
  source 1..1332: mol_type = other DNA
caggtgcagctggtgcagtctgggggaggcttggtacagcctggggggtccctgagactctcctgtgcagcctctggattcacctttagcagctatgccatgagctgggtccgccaggctccagggaaggggctggagtgggtctcagctattagtggtagtggtggtagcacatactacgcagactccgtgaagggccgattcaccatctccagagacaatcccaagaacaccctgttcctgcaaatgaccagtctaaggtctgaggacacggccatgtattattgtgcaagatcctatggtaactactttacttactggggccaagggaccctggtcaccgtctcatcagcttccaccaagggccccagcgtgttccccctggccccttgttccaggagcacctccgagagcaccgccgctctgggctgcctggtgaaggactacttccctgagcctgtgaccgtgagctggaactccggcgctctgacctccggcgtgcacaccttccccgccgtgctgcagagcagcggcctgtacagcctgagctccgtggtgacagtgcccagctccagcctgggcaccaagacctacacctgcaatgtggatcacaagcccagcaataccaaggtggacaagagggtggagtccaagtacggccctccctgcccctcctgtcctgctcctgagttcctgggcggcccttccgtgttcctgttcccccccaagcccaaggataccctgatgatcagccggacccctgaggtgacatgtgtggtggtggatgtgagccaggaggaccctgaggtgcagttcaactggtacgtggatggcgtggaggtgcacaacgccaagaccaagcctcgggaggagcagttcaatagcacctaccgggtggtgagcgtgctgaccgtgctgcaccaggattggctgaacggcaaggagtacaagtgcaaggtgagcaacaagggcctgcccagcagcatcgagaagaccatctccaaggctaagggccagccacgggagcctcaggtgtacaccctgccccctagccaggaggagatgaccaagaaccaggtgagcctgacctgtctggtgaagggcttctacccctccgatatcgctgtggagtgggagtccaacggccagcccgagaacaactataagaccaccccccctgtgctggacagcgacggcagcttcttcctgtattccaggctgaccgtggacaagagccggtggcaggagggcaatgtgttctcctgcagcgtgatgcacgaggccctgcacaaccactacacccagaagtccctgtccctgtccctcggcaag

SEQ ID NO: 385 - DNA, 1359 bp, synthetic construct
  source 1..1359: mol_type = other DNA
caggtgcagctgttggagtctggcccgggactggtgaagccttcggagaccctgtccctcacctgcactgtctctggtgactcgatcagtaattacttctggagctggatccggcagtccccagggaagggcctggagtggattgggtacatccattatagtgggaccgtcagctataacccgtccctcaggagtcgagtcaccatatcaatagacacgtccaagaaccaattctccctgaagctgagctctgtgaccgccgcagacacggccgtgtattactgtgcgaggcgagggcgtatagcagcagctggtacaggctactactactacggtatggacgtctggggccaagggaccacggtcaccgtctcatcagcttccaccaagggccccagcgtgttccccctggccccttgttccaggagcacctccgagagcaccgccgctctgggctgcctggtgaaggactacttccctgagcctgtgaccgtgagctggaactccggcgctctgacctccggcgtgcacaccttccccgccgtgctgcagagcagcggcctgtacagcctgagctccgtggtgacagtgcccagctccagcctgggcaccaagacctacacctgcaatgtggatcacaagcccagcaataccaaggtggacaagagggtggagtccaagtacggccctccctgcccctcctgtcctgctcctgagttcctgggcggcccttccgtgttcctgttcccccccaagcccaaggataccctgatgatcagccggacccctgaggtgacatgtgtggtggtggatgtgagccaggaggaccctgaggtgcagttcaactggtacgtggatggcgtggaggtgcacaacgccaagaccaagcctcgggaggagcagttcaatagcacctaccgggtggtgagcgtgctgaccgtgctgcaccaggattggctgaacggcaaggagtacaagtgcaaggtgagcaacaagggcctgcccagcagcatcgagaagaccatctccaaggctaagggccagccacgggagcctcaggtgtacaccctgccccctagccaggaggagatgaccaagaaccaggtgagcctgacctgtctggtgaagggcttctacccctccgatatcgctgtggagtgggagtccaacggccagcccgagaacaactataagaccaccccccctgtgctggacagcgacggcagcttcttcctgtattccaggctgaccgtggacaagagccggtggcaggagggcaatgtgttctcctgcagcgtgatgcacgaggccctgcacaaccactacacccagaagtccctgtccctgtccctcggcaag

SEQ ID NO: 386 - DNA, 1332 bp, synthetic construct
  source 1..1332: mol_type = other DNA
gaggtgcagctggtggagactgggggaggcctggtcaagcctggggggtccctgagactctcctgtgcagcctctggattcaccttcagtagctatagcatgaactgggtccgccaggctccagggaaggggctggagtgggtctcatccattagtagtagtagtagttacatatactacgcagactcagtgaagggccgattcaccatctccagagacaacgccaagaactcactgtatctgcaaatgaacagcctgagagccgaggacacggctgtgtattactgtgcgagaggtcgcagacgagactttgactactggggccagggcaccctggtcaccgtctcatcagcttccaccaagggccccagcgtgttccccctggccccttgttccaggagcacctccgagagcaccgccgctctgggctgcctggtgaaggactacttccctgagcctgtgaccgtgagctggaactccggcgctctgacctccggcgtgcacaccttccccgccgtgctgcagagcagcggcctgtacagcctgagctccgtggtgacagtgcccagctccagcctgggcaccaagacctacacctgcaatgtggatcacaagcccagcaataccaaggtggacaagagggtggagtccaagtacggccctccctgcccctcctgtcctgctcctgagttcctgggcggcccttccgtgttcctgttcccccccaagcccaaggataccctgatgatcagccggacccctgaggtgacatgtgtggtggtggatgtgagccaggaggaccctgaggtgcagttcaactggtacgtggatggcgtggaggtgcacaacgccaagaccaagcctcgggaggagcagttcaatagcacctaccgggtggtgagcgtgctgaccgtgctgcaccaggattggctgaacggcaaggagtacaagtgcaaggtgagcaacaagggcctgcccagcagcatcgagaagaccatctccaaggctaagggccagccacgggagcctcaggtgtacaccctgccccctagccaggaggagatgaccaagaaccaggtgagcctgacctgtctggtgaagggcttctacccctccgatatcgctgtggagtgggagtccaacggccagcccgagaacaactataagaccaccccccctgtgctggacagcgacggcagcttcttcctgtattccaggctgaccgtggacaagagccggtggcaggagggcaatgtgttctcctgcagcgtgatgcacgaggccctgcacaaccactacacccagaagtccctgtccctgtccctcggcaag

SEQ ID NO: 387 - DNA, 1362 bp, synthetic construct
  source 1..1362: mol_type = other DNA
caggttcagctggtacagtctggggctgaggtgaagaagcctgggtcctcggtaaaggtctcctgcaaggcttctggagacaccttcagcagctttgctatcagctgggtgcgacaggcccctggacaaggccttgagtggatggggacaatcatccctctctttactactccaaactatgcacagaaattccagggcagagtcacgattaccgcggacgaatccacgcgcacagcctacatggagctgagcagcctgagatctgaggacacggccgtgtattactgtgcgagagggcccgaacgtatagcagcagctggctactactactactacggtatggacgtctggggccaagggaccacggtcaccgtctcatcagcttccaccaagggccccagcgtgttccccctggccccttgttccaggagcacctccgagagcaccgccgctctgggctgcctggtgaaggactacttccctgagcctgtgaccgtgagctggaactccggcgctctgacctccggcgtgcacaccttccccgccgtgctgcagagcagcggcctgtacagcctgagctccgtggtgacagtgcccagctccagcctgggcaccaagacctacacctgcaatgtggatcacaagcccagcaataccaaggtggacaagagggtggagtccaagtacggccctccctgcccctcctgtcctgctcctgagttcctgggcggcccttccgtgttcctgttcccccccaagcccaaggataccctgatgatcagccggacccctgaggtgacatgtgtggtggtggatgtgagccaggaggaccctgaggtgcagttcaactggtacgtggatggcgtggaggtgcacaacgccaagaccaagcctcgggaggagcagttcaatagcacctaccgggtggtgagcgtgctgaccgtgctgcaccaggattggctgaacggcaaggagtacaagtgcaaggtgagcaacaagggcctgcccagcagcatcgagaagaccatctccaaggctaagggccagccacgggagcctcaggtgtacaccctgccccctagccaggaggagatgaccaagaaccaggtgagcctgacctgtctggtgaagggcttctacccctccgatatcgctgtggagtgggagtccaacggccagcccgagaacaactataagaccaccccccctgtgctggacagcgacggcagcttcttcctgtattccaggctgaccgtggacaagagccggtggcaggagggcaatgtgttctcctgcagcgtgatgcacgaggccctgcacaaccactacacccagaagtccctgtccctgtccctcggcaag

SEQ ID NO: 388 - DNA, 1338 bp, synthetic construct
  source 1..1338: mol_type = other DNA
caggtacagctggtgcagtctggggctgaggtgaagaagcctggggcctcagtgaaggtttcctgcaaggcatctggatacaccttcaccagctactatatgcactgggtgcgacaggcccctggacaagggcttgagtggatgggaataatcaaccctagtggtggtagcacaagctacgcacagaagttccagggcagagtcaccatgaccagggacacgtccacgagcacagtctacatggagctgagcagcctgagatctgaggacacggccgtgtattactgtgcgagaggggtttcacgaaggggtgcttttgatatctggggccaagggacaatggtcaccgtctcatcagcttccaccaagggccccagcgtgttccccctggccccttgttccaggagcacctccgagagcaccgccgctctgggctgcctggtgaaggactacttccctgagcctgtgaccgtgagctggaactccggcgctctgacctccggcgtgcacaccttccccgccgtgctgcagagcagcggcctgtacagcctgagctccgtggtgacagtgcccagctccagcctgggcaccaagacctacacctgcaatgtggatcacaagcccagcaataccaaggtggacaagagggtggagtccaagtacggccctccctgcccctcctgtcctgctcctgagttcctgggcggcccttccgtgttcctgttcccccccaagcccaaggataccctgatgatcagccggacccctgaggtgacatgtgtggtggtggatgtgagccaggaggaccctgaggtgcagttcaactggtacgtggatggcgtggaggtgcacaacgccaagaccaagcctcgggaggagcagttcaatagcacctaccgggtggtgagcgtgctgaccgtgctgcaccaggattggctgaacggcaaggagtacaagtgcaaggtgagcaacaagggcctgcccagcagcatcgagaagaccatctccaaggctaagggccagccacgggagcctcaggtgtacaccctgccccctagccaggaggagatgaccaagaaccaggtgagcctgacctgtctggtgaagggcttctacccctccgatatcgctgtggagtgggagtccaacggccagcccgagaacaactataagaccaccccccctgtgctggacagcgacggcagcttcttcctgtattccaggctgaccgtggacaagagccggtggcaggagggcaatgtgttctcctgcagcgtgatgcacgaggccctgcacaaccactacacccagaagtccctgtccctgtccctcggcaag

SEQ ID NO: 389 - DNA, 1332 bp, synthetic construct
  source 1..1332: mol_type = other DNA
gaggtgcagctggtggagactgggggaggcgtggtccagcctgggaggtccctgagactctcctgtgcagcctctggattcaccttcagtagctatgctatgcactgggtccgccaggctccaggcaaggggctggagtgggtggcagttatatcatatgatggaagtaataaatactacgcagactccgtgaagggccgattcaccatctccagagacaattccaagaacacgctgtatctgcaaatgaacagcctgagagctgaggacacggctgtgtattactgtgcgagaaatcgatacggggccactgactactggggccagggaaccctggtcaccgtctcatcagcttccaccaagggccccagcgtgttccccctggccccttgttccaggagcacctccgagagcaccgccgctctgggctgcctggtgaaggactacttccctgagcctgtgaccgtgagctggaactccggcgctctgacctccggcgtgcacaccttccccgccgtgctgcagagcagcggcctgtacagcctgagctccgtggtgacagtgcccagctccagcctgggcaccaagacctacacctgcaatgtggatcacaagcccagcaataccaaggtggacaagagggtggagtccaagtacggccctccctgcccctcctgtcctgctcctgagttcctgggcggcccttccgtgttcctgttcccccccaagcccaaggataccctgatgatcagccggacccctgaggtgacatgtgtggtggtggatgtgagccaggaggaccctgaggtgcagttcaactggtacgtggatggcgtggaggtgcacaacgccaagaccaagcctcgggaggagcagttcaatagcacctaccgggtggtgagcgtgctgaccgtgctgcaccaggattggctgaacggcaaggagtacaagtgcaaggtgagcaacaagggcctgcccagcagcatcgagaagaccatctccaaggctaagggccagccacgggagcctcaggtgtacaccctgccccctagccaggaggagatgaccaagaaccaggtgagcctgacctgtctggtgaagggcttctacccctccgatatcgctgtggagtgggagtccaacggccagcccgagaacaactataagaccaccccccctgtgctggacagcgacggcagcttcttcctgtattccaggctgaccgtggacaagagccggtggcaggagggcaatgtgttctcctgcagcgtgatgcacgaggccctgcacaaccactacacccagaagtccctgtccctgtccctcggcaag

SEQ ID NO: 390 - DNA, 1356 bp, synthetic construct
  source 1..1356: mol_type = other DNA
cagatcaccttgaaggagtctggcccaggactggtgaagccttcggggaccctgtccctcacctgcgctgtctctggtggctccatcagcagtagtaactggtggagttgggtccgccagcccccagggaaggggctggagtggattggggaaatctatcatagtgggagcaccaactacaacccgtccctcaagagtcgagtcaccatatcagtagacaagtccaagaaccagttctccctgaagctgagctctgtgaccgccgcggacacggccgtgtattactgtgcgagagatgacgggtggcgttatggttcggtctactactactacatggacgtctggggcaaagggaccacggtcaccgtctcatcagcttccaccaagggccccagcgtgttccccctggccccttgttccaggagcacctccgagagcaccgccgctctgggctgcctggtgaaggactacttccctgagcctgtgaccgtgagctggaactccggcgctctgacctccggcgtgcacaccttccccgccgtgctgcagagcagcggcctgtacagcctgagctccgtggtgacagtgcccagctccagcctgggcaccaagacctacacctgcaatgtggatcacaagcccagcaataccaaggtggacaagagggtggagtccaagtacggccctccctgcccctcctgtcctgctcctgagttcctgggcggcccttccgtgttcctgttcccccccaagcccaaggataccctgatgatcagccggacccctgaggtgacatgtgtggtggtggatgtgagccaggaggaccctgaggtgcagttcaactggtacgtggatggcgtggaggtgcacaacgccaagaccaagcctcgggaggagcagttcaatagcacctaccgggtggtgagcgtgctgaccgtgctgcaccaggattggctgaacggcaaggagtacaagtgcaaggtgagcaacaagggcctgcccagcagcatcgagaagaccatctccaaggctaagggccagccacgggagcctcaggtgtacaccctgccccctagccaggaggagatgaccaagaaccaggtgagcctgacctgtctggtgaagggcttctacccctccgatatcgctgtggagtgggagtccaacggccagcccgagaacaactataagaccaccccccctgtgctggacagcgacggcagcttcttcctgtattccaggctgaccgtggacaagagccggtggcaggagggcaatgtgttctcctgcagcgtgatgcacgaggccctgcacaaccactacacccagaagtccctgtccctgtccctcggcaag

SEQ ID NO: 391 - DNA, 1344 bp, synthetic construct
  source 1..1344: mol_type = other DNA
gaggtgcagctgttggagtctgggggaggcttggtacagcctggggggtccctgagactctcctgtgcagcctctggattcacctttagcagctatgccatgagctgggtccgccaggctccagggaaggggctggagtgggtctcagctattagtggtagtggtggtagaacatactacgcagactccgtgaagggccggttcaccatctccagagacaattccaagaacacgctgtatctgcaaatgaacagcctgagagccgaggacacggccgtatattactgtgcgagagtgttacaatatagcgggaccgacgatttggacgtctggggccgagggaccctggtcaccgtctcatcagcttccaccaagggccccagcgtgttccccctggccccttgttccaggagcacctccgagagcaccgccgctctgggctgcctggtgaaggactacttccctgagcctgtgaccgtgagctggaactccggcgctctgacctccggcgtgcacaccttccccgccgtgctgcagagcagcggcctgtacagcctgagctccgtggtgacagtgcccagctccagcctgggcaccaagacctacacctgcaatgtggatcacaagcccagcaataccaaggtggacaagagggtggagtccaagtacggccctccctgcccctcctgtcctgctcctgagttcctgggcggcccttccgtgttcctgttcccccccaagcccaaggataccctgatgatcagccggacccctgaggtgacatgtgtggtggtggatgtgagccaggaggaccctgaggtgcagttcaactggtacgtggatggcgtggaggtgcacaacgccaagaccaagcctcgggaggagcagttcaatagcacctaccgggtggtgagcgtgctgaccgtgctgcaccaggattggctgaacggcaaggagtacaagtgcaaggtgagcaacaagggcctgcccagcagcatcgagaagaccatctccaaggctaagggccagccacgggagcctcaggtgtacaccctgccccctagccaggaggagatgaccaagaaccaggtgagcctgacctgtctggtgaagggcttctacccctccgatatcgctgtggagtgggagtccaacggccagcccgagaacaactataagaccaccccccctgtgctggacagcgacggcagcttcttcctgtattccaggctgaccgtggacaagagccggtggcaggagggcaatgtgttctcctgcagcgtgatgcacgaggccctgcacaaccactacacccagaagtccctgtccctgtccctcggcaag

SEQ ID NO: 392 - DNA, 1335 bp, synthetic construct; identical to SEQ ID NO: 377
  source 1..1335: mol_type = other DNA

SEQ ID NO: 393 - DNA, 1329 bp, synthetic construct
  source 1..1329: mol_type = other DNA
gaggtgcagctgttggagtctgggggaggcctggtcaagcctggggggtccctgagactctcctgtgcagcctctggactcatcttcaaaaactatggcatgaactgggtccgcctggctccggggaaggggctggagtgggttgcatccattagtggtaatagtaactacatctcgtatgcagactcagtgaagggccgattcaccatctccagagacaacgccaacaactcactgtttctgcagatgagcagcctgagagccgacgacacggctgtctattattgttcgagtggttatttctactttgacctctggggcccgggaaccctggtcaccgtctcatcagcttccaccaagggccccagcgtgttccccctggccccttgttccaggagcacctccgagagcaccgccgctctgggctgcctggtgaaggactacttccctgagcctgtgaccgtgagctggaactccggcgctctgacctccggcgtgcacaccttccccgccgtgctgcagagcagcggcctgtacagcctgagctccgtggtgacagtgcccagctccagcctgggcaccaagacctacacctgcaatgtggatcacaagcccagcaataccaaggtggacaagagggtggagtccaagtacggccctccctgcccctcctgtcctgctcctgagttcctgggcggcccttccgtgttcctgttcccccccaagcccaaggataccctgatgatcagccggacccctgaggtgacatgtgtggtggtggatgtgagccaggaggaccctgaggtgcagttcaactggtacgtggatggcgtggaggtgcacaacgccaagaccaagcctcgggaggagcagttcaatagcacctaccgggtggtgagcgtgctgaccgtgctgcaccaggattggctgaacggcaaggagtacaagtgcaaggtgagcaacaagggcctgcccagcagcatcgagaagaccatctccaaggctaagggccagccacgggagcctcaggtgtacaccctgccccctagccaggaggagatgaccaagaaccaggtgagcctgacctgtctggtgaagggcttctacccctccgatatcgctgtggagtgggagtccaacggccagcccgagaacaactataagaccaccccccctgtgctggacagcgacggcagcttcttcctgtattccaggctgaccgtggacaagagccggtggcaggagggcaatgtgttctcctgcagcgtgatgcacgaggccctgcacaaccactacacccagaagtccctgtccctgtccctcggcaag

SEQ ID NO: 394 - DNA, 1347 bp, synthetic construct
  source 1..1347: mol_type = other DNA
gaggtgcagctgttggagtctgggggaggcctggtcaagcctggggggtccctgagactctcctgtgcagcctctggattcaccttcagtagctatagcatgaactgggtccgccaggctccagggaaggggctggagtgggtctcatccattagtagtagtagtagttacatatactacgcagactcagtgaagggccgattcaccatctccagagacaacgccaagaactcactgtatctgcaaatgaacagcctgagagacggggacacggccatatactactgtgtgagacgcctttgggaagctccggggattgggccttttgatgtctggggccacgggacaatggtcaccgtctcatcagcttccaccaagggccccagcgtgttccccctggccccttgttccaggagcacctccgagagcaccgccgctctgggctgcctggtgaaggactacttccctgagcctgtgaccgtgagctggaactccggcgctctgacctccggcgtgcacaccttccccgccgtgctgcagagcagcggcctgtacagcctgagctccgtggtgacagtgcccagctccagcctgggcaccaagacctacacctgcaatgtggatcacaagcccagcaataccaaggtggacaagagggtggagtccaagtacggccctccctgcccctcctgtcctgctcctgagttcctgggcggcccttccgtgttcctgttcccccccaagcccaaggataccctgatgatcagccggacccctgaggtgacatgtgtggtggtggatgtgagccaggaggaccctgaggtgcagttcaactggtacgtggatggcgtggaggtgcacaacgccaagaccaagcctcgggaggagcagttcaatagcacctaccgggtggtgagcgtgctgaccgtgctgcaccaggattggctgaacggcaaggagtacaagtgcaaggtgagcaacaagggcctgcccagcagcatcgagaagaccatctccaaggctaagggccagccacgggagcctcaggtgtacaccctgccccctagccaggaggagatgaccaagaaccaggtgagcctgacctgtctggtgaagggcttctacccctccgatatcgctgtggagtgggagtccaacggccagcccgagaacaactataagaccaccccccctgtgctggacagcgacggcagcttcttcctgtattccaggctgaccgtggacaagagccggtggcaggagggcaatgtgttctcctgcagcgtgatgcacgaggccctgcacaaccactacacccagaagtccctgtccctgtccctcggcaag

SEQ ID NO: 395 - DNA, 1335 bp, synthetic construct
  source 1..1335: mol_type = other DNA
gaggtgcagctgttggagtctgggggaggcttggtccagcctggggggtccctgaaactctcctgtgcagcctctgggttcaccttcagtggctatgctatgcactgggtccgccaggctccaggcaaggggctggagtgggtggcagttatatcatatgatggaagtaataaatactacgcagactccgtgaagggccgattcaccatctccagagacaattccaagaacacgctgtatctgcaaatgaacagcctgagagctgaggacacggctgtgtattactgtgcgagaggaagggggaggggggtctttgactactggggccagggaaccctggtcaccgtctcatcagcttccaccaagggccccagcgtgttccccctggccccttgttccaggagcacctccgagagcaccgccgctctgggctgcctggtgaaggactacttccctgagcctgtgaccgtgagctggaactccggcgctctgacctccggcgtgcacaccttccccgccgtgctgcagagcagcggcctgtacagcctgagctccgtggtgacagtgcccagctccagcctgggcaccaagacctacacctgcaatgtggatcacaagcccagcaataccaaggtggacaagagggtggagtccaagtacggccctccctgcccctcctgtcctgctcctgagttcctgggcggcccttccgtgttcctgttcccccccaagcccaaggataccctgatgatcagccggacccctgaggtgacatgtgtggtggtggatgtgagccaggaggaccctgaggtgcagttcaactggtacgtggatggcgtggaggtgcacaacgccaagaccaagcctcgggaggagcagttcaatagcacctaccgggtggtgagcgtgctgaccgtgctgcaccaggattggctgaacggcaaggagtacaagtgcaaggtgagcaacaagggcctgcccagcagcatcgagaagaccatctccaaggctaagggccagccacgggagcctcaggtgtacaccctgccccctagccaggaggagatgaccaagaaccaggtgagcctgacctgtctggtgaagggcttctacccctccgatatcgctgtggagtgggagtccaacggccagcccgagaacaactataagaccaccccccctgtgctggacagcgacggcagcttcttcctgtattccaggctgaccgtggacaagagccggtggcaggagggcaatgtgttctcctgcagcgtgatgcacgaggccctgcacaaccactacacccagaagtccctgtccctgtccctcggcaag

SEQ ID NO: 396 - DNA, 1326 bp, synthetic construct
  source 1..1326: mol_type = other DNA
gaggtgcagctgttggagtctgggggaggcttggtacagcctggggggtccctgagactctcctgtgcagcctctggattcaccttcagtagctatagcatgaactgggtccgccaggctccagggaaggggctggagtgggtttcatacattagtagtagtagtagtaccatatactacgcagactctgtgaagggccgattcaccatctccagagacaatgccaagaactcactgtatctgcaaatgaacagcctgagagacgaggacacggctgtgtattactgtgcgagagatcggacgctgggctactggggccagggaaccctggtcaccgtctcatcagcttccaccaagggccccagcgtgttccccctggccccttgttccaggagcacctccgagagcaccgccgctctgggctgcctggtgaaggactacttccctgagcctgtgaccgtgagctggaactccggcgctctgacctccggcgtgcacaccttccccgccgtgctgcagagcagcggcctgtacagcctgagctccgtggtgacagtgcccagctccagcctgggcaccaagacctacacctgcaatgtggatcacaagcccagcaataccaaggtggacaagagggtggagtccaagtacggccctccctgcccctcctgtcctgctcctgagttcctgggcggcccttccgtgttcctgttcccccccaagcccaaggataccctgatgatcagccggacccctgaggtgacatgtgtggtggtggatgtgagccaggaggaccctgaggtgcagttcaactggtacgtggatggcgtggaggtgcacaacgccaagaccaagcctcgggaggagcagttcaatagcacctaccgggtggtgagcgtgctgaccgtgctgcaccaggattggctgaacggcaaggagtacaagtgcaaggtgagcaacaagggcctgcccagcagcatcgagaagaccatctccaaggctaagggccagccacgggagcctcaggtgtacaccctgccccctagccaggaggagatgaccaagaaccaggtgagcctgacctgtctggtgaagggcttctacccctccgatatcgctgtggagtgggagtccaacggccagcccgagaacaactataagaccaccccccctgtgctggacagcgacggcagcttcttcctgtattccaggctgaccgtggacaagagccggtggcaggagggcaatgtgttctcctgcagcgtgatgcacgaggccctgcacaaccactacacccagaagtccctgtccctgtccctcggcaag

SEQ ID NO: 397 - DNA, 1359 bp, synthetic construct
  source 1..1359: mol_type = other DNA
caggtgcagctacagcagtggggcgcaggactgttgaagccttcacagaccctgtccctcacctgcactgtctctggtggctccatcagcagtggtggttactactggagctggatccgccagcacccagggaagggcctggagtggattgggtacatctattacagtgggagcacctactacaacccgtccctcaagagtcgagttaccatatcagtagacacgtctaagaaccagttctccctgaagctgagctctgtgactgccgcggacacggccgtgtattactgtgcgagatgggaccgagtcagagagggaggccggttctcaaatgcttttgatatctggggccaagggacaatggtcaccgtctcatcagcttccaccaagggccccagcgtgttccccctggccccttgttccaggagcacctccgagagcaccgccgctctgggctgcctggtgaaggactacttccctgagcctgtgaccgtgagctggaactccggcgctctgacctccggcgtgcacaccttccccgccgtgctgcagagcagcggcctgtacagcctgagctccgtggtgacagtgcccagctccagcctgggcaccaagacctacacctgcaatgtggatcacaagcccagcaataccaaggtggacaagagggtggagtccaagtacggccctccctgcccctcctgtcctgctcctgagttcctgggcggcccttccgtgttcctgttcccccccaagcccaaggataccctgatgatcagccggacccctgaggtgacatgtgtggtggtggatgtgagccaggaggaccctgaggtgcagttcaactggtacgtggatggcgtggaggtgcacaacgccaagaccaagcctcgggaggagcagttcaatagcacctaccgggtggtgagcgtgctgaccgtgctgcaccaggattggctgaacggcaaggagtacaagtgcaaggtgagcaacaagggcctgcccagcagcatcgagaagaccatctccaaggctaagggccagccacgggagcctcaggtgtacaccctgccccctagccaggaggagatgaccaagaaccaggtgagcctgacctgtctggtgaagggcttctacccctccgatatcgctgtggagtgggagtccaacggccagcccgagaacaactataagaccaccccccctgtgctggacagcgacggcagcttcttcctgtattccaggctgaccgtggacaagagccggtggcaggagggcaatgtgttctcctgcagcgtgatgcacgaggccctgcacaaccactacacccagaagtccctgtccctgtccctcggcaag

SEQ ID NO: 398 - DNA, 1347 bp, synthetic construct
  source 1..1347: mol_type = other DNA
cagctgcagctgcaggagtcgggcccaggactggtgaagccttcacagaccctgtccctcacctgcactgtctctggtggctccatcagcagtggtggttactactggagctggatccgccagcacccagggaagggcctggagtggattgggtacatctattacagtgggagcacctactacaacccgtccctcaagagtcgagttaccatatcagtagacacgtctaagaaccagttctccctgaagctgagctctgtgactgccgcggacacggccgtgtattactgtgcgaggggtaaaagagatggctacaattactactttgactactggggccagggaaccctggtcaccgtctcatcagcttccaccaagggccccagcgtgttccccctggccccttgttccaggagcacctccgagagcaccgccgctctgggctgcctggtgaaggactacttccctgagcctgtgaccgtgagctggaactccggcgctctgacctccggcgtgcacaccttccccgccgtgctgcagagcagcggcctgtacagcctgagctccgtggtgacagtgcccagctccagcctgggcaccaagacctacacctgcaatgtggatcacaagcccagcaataccaaggtggacaagagggtggagtccaagtacggccctccctgcccctcctgtcctgctcctgagttcctgggcggcccttccgtgttcctgttcccccccaagcccaaggataccctgatgatcagccggacccctgaggtgacatgtgtggtggtggatgtgagccaggaggaccctgaggtgcagttcaactggtacgtggatggcgtggaggtgcacaacgccaagaccaagcctcgggaggagcagttcaatagcacctaccgggtggtgagcgtgctgaccgtgctgcaccaggattggctgaacggcaaggagtacaagtgcaaggtgagcaacaagggcctgcccagcagcatcgagaagaccatctccaaggctaagggccagccacgggagcctcaggtgtacaccctgccccctagccaggaggagatgaccaagaaccaggtgagcctgacctgtctggtgaagggcttctacccctccgatatcgctgtggagtgggagtccaacggccagcccgagaacaactataagaccaccccccctgtgctggacagcgacggcagcttcttcctgtattccaggctgaccgtggacaagagccggtggcaggagggcaatgtgttctcctgcagcgtgatgcacgaggccctgcacaaccactacacccagaagtccctgtccctgtccctcggcaag

SEQ ID NO: 399 - DNA, 1356 bp, synthetic construct
  source 1..1356: mol_type = other DNA
caggtacagctgcagcagtcgggcccaggactggtgaagccttcacagaccctgtccctcacctgcactgtctctggtggctccatcagcagtggtggttactactggagctggatccgccagcacccagggaagggcctggagtggattgggtacatctattacagtgggagcacctactacaacccgtccctcaagagtcgagttaccatatcagtagacacgtctaagaaccagttctccctgaagctgagctctgtgaccgccgcagacacggctgtgtattactgtgcgagacagaggcgtgccaacgggtatagcagcagctgggaatttgactactggggccagggaaccctggtcaccgtctcatcagcttccaccaagggccccagcgtgttccccctggccccttgttccaggagcacctccgagagcaccgccgctctgggctgcctggtgaaggactacttccctgagcctgtgaccgtgagctggaactccggcgctctgacctccggcgtgcacaccttccccgccgtgctgcagagcagcggcctgtacagcctgagctccgtggtgacagtgcccagctccagcctgggcaccaagacctacacctgcaatgtggatcacaagcccagcaataccaaggtggacaagagggtggagtccaagtacggccctccctgcccctcctgtcctgctcctgagttcctgggcggcccttccgtgttcctgttcccccccaagcccaaggataccctgatgatcagccggacccctgaggtgacatgtgtggtggtggatgtgagccaggaggaccctgaggtgcagttcaactggtacgtggatggcgtggaggtgcacaacgccaagaccaagcctcgggaggagcagttcaatagcacctaccgggtggtgagcgtgctgaccgtgctgcaccaggattggctgaacggcaaggagtacaagtgcaaggtgagcaacaagggcctgcccagcagcatcgagaagaccatctccaaggctaagggccagccacgggagcctcaggtgtacaccctgccccctagccaggaggagatgaccaagaaccaggtgagcctgacctgtctggtgaagggcttctacccctccgatatcgctgtggagtgggagtccaacggccagcccgagaacaactataagaccaccccccctgtgctggacagcgacggcagcttcttcctgtattccaggctgaccgtggacaagagccggtggcaggagggcaatgtgttctcctgcagcgtgatgcacgaggccctgcacaaccactacacccagaagtccctgtccctgtccctcggcaag

SEQ ID NO: 400 - DNA, 1344 bp, synthetic construct
  source 1..1344: mol_type = other DNA
gaggtacaactggtggagtctgggggcggcttggtccagcctggggggtccctgagactctcctgtgcagcctctggattcaccttcagtagctatgctatgcactgggtccgccaggctccagggaaggggctggagtgggtctcagctattagtggtagtggtgatagcacatactacgcagactccgtgaagggccggttcagcatctccagagacaattccaagaacacgctgtatctgcaaatgaacagcctgagagccgaggacacggccgtatattactgtgcgaaagggagtaggaggagtggcttcaacctttttgactactggggccagggcaccctggtcaccgtctcatcagcttccaccaagggccccagcgtgttccccctggccccttgttccaggagcacctccgagagcaccgccgctctgggctgcctggtgaaggactacttccctgagcctgtgaccgtgagctggaactccggcgctctgacctccggcgtgcacaccttccccgccgtgctgcagagcagcggcctgtacagcctgagctccgtggtgacagtgcccagctccagcctgggcaccaagacctacacctgcaatgtggatcacaagcccagcaataccaaggtggacaagagggtggagtccaagtacggccctccctgcccctcctgtcctgctcctgagttcctgggcggcccttccgtgttcctgttcccccccaagcccaaggataccctgatgatcagccggacccctgaggtgacatgtgtggtggtggatgtgagccaggaggaccctgaggtgcagttcaactggtacgtggatggcgtggaggtgcacaacgccaagaccaagcctcgggaggagcagttcaatagcacctaccgggtggtgagcgtgctgaccgtgctgcaccaggattggctgaacggcaaggagtacaagtgcaaggtgagcaacaagggcctgcccagcagcatcgagaagaccatctccaaggctaagggccagccacgggagcctcaggtgtacaccctgccccctagccaggaggagatgaccaagaaccaggtgagcctgacctgtctggtgaagggcttctacccctccgatatcgctgtggagtgggagtccaacggccagcccgagaacaactataagaccaccccccctgtgctggacagcgacggcagcttcttcctgtattccaggctgaccgtggacaagagccggtggcaggagggcaatgtgttctcctgcagcgtgatgcacgaggccctgcacaaccactacacccagaagtccctgtccctgtccctcggcaag

SEQ ID NO: 401 - DNA, 1353 bp, synthetic construct
  source 1..1353: mol_type = other DNA
cagctgcagctgcaggagtcgggcccaggactggtgaagccttcacagaccctgtccctcacctgcactgtctctggtggctccatcagcagtggtggttactactggagctggatccgccagcacccagggaagggcctggagtggattgggtacatctattacagtgggagcacctactacaacccgtccctcaagagtcgagttaccatatcagtagacacgtctaagaaccagttctccctgaagctgagctctgtgactgccgcggacacggccgtgtattactgtgcgaggatgggccgtatagcagcatccaactactacggtatggacgtctggggccaagggaccacggtcaccgtctcatcagcttccaccaagggccccagcgtgttccccctggccccttgttccaggagcacctccgagagcaccgccgctctgggctgcctggtgaaggactacttccctgagcctgtgaccgtgagctggaactccggcgctctgacctccggcgtgcacaccttccccgccgtgctgcagagcagcggcctgtacagcctgagctccgtggtgacagtgcccagctccagcctgggcaccaagacctacacctgcaatgtggatcacaagcccagcaataccaaggtggacaagagggtggagtccaagtacggccctccctgcccctcctgtcctgctcctgagttcctgggcggcccttccgtgttcctgttcccccccaagcccaaggataccctgatgatcagccggacccctgaggtgacatgtgtggtggtggatgtgagccaggaggaccctgaggtgcagttcaactggtacgtggatggcgtggaggtgcacaacgccaagaccaagcctcgggaggagcagttcaatagcacctaccgggtggtgagcgtgctgaccgtgctgcaccaggattggctgaacggcaaggagtacaagtgcaaggtgagcaacaagggcctgcccagcagcatcgagaagaccatctccaaggctaagggccagccacgggagcctcaggtgtacaccctgccccctagccaggaggagatgaccaagaaccaggtgagcctgacctgtctggtgaagggcttctacccctccgatatcgctgtggagtgggagtccaacggccagcccgagaacaactataagaccaccccccctgtgctggacagcgacggcagcttcttcctgtattccaggctgaccgtggacaagagccggtggcaggagggcaatgtgttctcctgcagcgtgatgcacgaggccctgcacaaccactacacccagaagtccctgtccctgtccctcggcaag

SEQ ID NO: 402 - DNA, 1356 bp, synthetic construct
  source 1..1356: mol_type = other DNA
caggtacagctgcagcagtcgggcccaggactggtgaagccttcacagaccctgtccctcacctgcactgtctctggtggctccatcagcagtggtggttactactggagctggatccgccagcacccagggaagggcctggagtggattgggtacatctattacagtgggagcacctactacaacccgtccctcaagagtcgagttaccatatcagtagacacgtctaagaaccagttctccctgaagctgagctctgtgaccgccgcagacacggctgtgtattactgtgcgagacagaggcgtgccaacgggtatagcagcagctgggaatttgactactggggccagggcaccctggtcaccgtctcatcagcttccaccaagggccccagcgtgttccccctggccccttgttccaggagcacctccgagagcaccgccgctctgggctgcctggtgaaggactacttccctgagcctgtgaccgtgagctggaactccggcgctctgacctccggcgtgcacaccttccccgccgtgctgcagagcagcggcctgtacagcctgagctccgtggtgacagtgcccagctccagcctgggcaccaagacctacacctgcaatgtggatcacaagcccagcaataccaaggtggacaagagggtggagtccaagtacggccctccctgccccccctgtcctgctcctgagttcctgggcggcccttccgtgttcctgttcccccccaagcccaaggataccctgatgatcagccggacccctgaggtgacatgtgtggtggtggatgtgagccaggaggaccctgaggtgcagttcaactggtacgtggatggcgtggaggtgcacaacgccaagaccaagcctcgggaggagcagttcaatagcacctaccgggtggtgagcgtgctgaccgtgctgcaccaggattggctgaacggcaaggagtacaagtgcaaggtgagcaacaagggcctgcccagcagcatcgagaagaccatctccaaggctaagggccagccacgggagcctcaggtgtacaccctgccccctagccaggaggagatgaccaagaaccaggtgagcctgacctgtctggtgaagggcttctacccctccgatatcgctgtggagtgggagtccaacggccagcccgagaacaactataagaccaccccccctgtgctggacagcgacggcagcttcttcctgtattccaggctgaccgtggacaagagccggtggcaggagggcaatgtgttctcctgcagcgtgatgcacgaggccctgcacaaccactacacccagaagtccctgtccctgtccctcggcaag

SEQ ID NO: 403 - DNA, 1326 bp, synthetic construct
  source 1..1326: mol_type = other DNA
caggtgcagctggtacagtctgggggaggcgtggtccagcctgggaactccctgagactctcctgtgtagcctctggattcaccttcagtaggtacaccatccactgggtccgccaggctccaggcaaggggctggagtgggtggcagttatatcatatgatggaagcaataaatactacgcagactccgtgaagggccgattcaccatctccagagacaattccaagaacacgctgtatctgcaaatgaacagcctgagagctgaggacacggctgtgtattactgtgcgagaggaggcccaactccagactggggccagggcaccctggtcaccgtctcatcagcttccaccaagggccccagcgtgttccccctggccccttgttccaggagcacctccgagagcaccgccgctctgggctgcctggtgaaggactacttccctgagcctgtgaccgtgagctggaactccggcgctctgacctccggcgtgcacaccttccccgccgtgctgcagagcagcggcctgtacagcctgagctccgtggtgacagtgcccagctccagcctgggcaccaagacctacacctgcaatgtggatcacaagcccagcaataccaaggtggacaagagggtggagtccaagtacggccctccctgccccccctgtcctgctcctgagttcctgggcggcccttccgtgttcctgttcccccccaagcccaaggataccctgatgatcagccggacccctgaggtgacatgtgtggtggtggatgtgagccaggaggaccctgaggtgcagttcaactggtacgtggatggcgtggaggtgcacaacgccaagaccaagcctcgggaggagcagttcaatagcacctaccgggtggtgagcgtgctgaccgtgctgcaccaggattggctgaacggcaaggagtacaagtgcaaggtgagcaacaagggcctgcccagcagcatcgagaagaccatctccaaggctaagggccagccacgggagcctcaggtgtacaccctgccccctagccaggaggagatgaccaagaaccaggtgagcctgacctgtctggtgaagggcttctacccctccgatatcgctgtggagtgggagtccaacggccagcccgagaacaactataagaccaccccccctgtgctggacagcgacggcagcttcttcctgtattccaggctgaccgtggacaagagccggtggcaggagggcaatgtgttctcctgcagcgtgatgcacgaggccctgcacaaccactacacccagaagtccctgtccctgtccctcggcaag

SEQ ID NO: 404 - DNA, 1344 bp, synthetic construct
  source 1..1344: mol_type = other DNA
caggtgcagctgttggagtctgggggaggcctggtcaagcctggggggtccctgagactctcctgtgcagcctctggattcaccttcagtagctatagcatgaactgggtccgccaggctccagggaaggggctggagtgggtctcatccattagtagtggtagtagttacatatactacgcagactcagtgaagggccgattcaccatctccagagacaacgccaagaactcactgtatctgcaaatgaacagcctgagagccgaggacacggctgtgtattactgtgcgagagatcaaggggcgtccgtaactggaacccacacccactggggccagggaaccctggtcaccgtctcatcagcttccaccaagggccccagcgtgttccccctggccccttgttccaggagcacctccgagagcaccgccgctctgggctgcctggtgaaggactacttccctgagcctgtgaccgtgagctggaactccggcgctctgacctccggcgtgcacaccttccccgccgtgctgcagagcagcggcctgtacagcctgagctccgtggtgacagtgcccagctccagcctgggcaccaagacctacacctgcaatgtggatcacaagcccagcaataccaaggtggacaagagggtggagtccaagtacggccctccctgccccccctgtcctgctcctgagttcctgggcggcccttccgtgttcctgttcccccccaagcccaaggataccctgatgatcagccggacccctgaggtgacatgtgtggtggtggatgtgagccaggaggaccctgaggtgcagttcaactggtacgtggatggcgtggaggtgcacaacgccaagaccaagcctcgggaggagcagttcaatagcacctaccgggtggtgagcgtgctgaccgtgctgcaccaggattggctgaacggcaaggagtacaagtgcaaggtgagcaacaagggcctgcccagcagcatcgagaagaccatctccaaggctaagggccagccacgggagcctcaggtgtacaccctgccccctagccaggaggagatgaccaagaaccaggtgagcctgacctgtctggtgaagggcttctacccctccgatatcgctgtggagtgggagtccaacggccagcccgagaacaactataagaccaccccccctgtgctggacagcgacggcagcttcttcctgtattccaggctgaccgtggacaagagccggtggcaggagggcaatgtgttctcctgcagcgtgatgcacgaggccctgcacaaccactacacccagaagtccctgtccctgtccctcggcaag

SEQ ID NO: 405 - DNA, 1335 bp, synthetic construct
  source 1..1335: mol_type = other DNA
caggtgcagctggtgcaatctggggctgaggtgaagaagcctgggtcctcggtgaaggtctcctgcaaggcttctggaggcaccttcagcagctatactatcagctgggtgcgacaggcccctggacaagggcttgagtggatgggaaggatcatccctatccttggtatagcaaactacgcacagaagttccagggcagagtcacgattaccgcggacaaatccacgagcacagcctacatggagctgagcagcctgagatctgaggacacggccgtgtattactgtgcgacgggggttggtatggttcggggagacccttggggccagggaaccctggtcaccgtctcatcagcttccaccaagggccccagcgtgttccccctggccccttgttccaggagcacctccgagagcaccgccgctctgggctgcctggtgaaggactacttccctgagcctgtgaccgtgagctggaactccggcgctctgacctccggcgtgcacaccttccccgccgtgctgcagagcagcggcctgtacagcctgagctccgtggtgacagtgcccagctccagcctgggcaccaagacctacacctgcaatgtggatcacaagcccagcaataccaaggtggacaagagggtggagtccaagtacggccctccctgccccccctgtcctgctcctgagttcctgggcggcccttccgtgttcctgttcccccccaagcccaaggataccctgatgatcagccggacccctgaggtgacatgtgtggtggtggatgtgagccaggaggaccctgaggtgcagttcaactggtacgtggatggcgtggaggtgcacaacgccaagaccaagcctcgggaggagcagttcaatagcacctaccgggtggtgagcgtgctgaccgtgctgcaccaggattggctgaacggcaaggagtacaagtgcaaggtgagcaacaagggcctgcccagcagcatcgagaagaccatctccaaggctaagggccagccacgggagcctcaggtgtacaccctgccccctagccaggaggagatgaccaagaaccaggtgagcctgacctgtctggtgaagggcttctacccctccgatatcgctgtggagtgggagtccaacggccagcccgagaacaactataagaccaccccccctgtgctggacagcgacggcagcttcttcctgtattccaggctgaccgtggacaagagccggtggcaggagggcaatgtgttctcctgcagcgtgatgcacgaggccctgcacaaccactacacccagaagtccctgtccctgtccctcggcaag

SEQ ID NO: 406 - DNA, 1359 bp, synthetic construct
  source 1..1359: mol_type = other DNA
cggctgcagctgcaggagtcgggcccaggactggtgaagccttcacagaccctgtccctcacctgcactgtctctggtggctccatcagcagtggtggttactactggagctggatccgccagcacccagggaagggcctggagtggattgggtacatctattacagtgggagcacctactacaacccgtccctcaagagtcgagttaccatatcagtagacacgtctaagaaccagttctccctgaagctgagctctgtgactgccgcggacacggccgtgtattactgtgcgaggattcaccatagtaccgcggggccatacaacaactggtactttgactactggggccagggaaccctggtcaccgtctcatcagcttccaccaagggccccagcgtgttccccctggccccttgttccaggagcacctccgagagcaccgccgctctgggctgcctggtgaaggactacttccctgagcctgtgaccgtgagctggaactccggcgctctgacctccggcgtgcacaccttccccgccgtgctgcagagcagcggcctgtacagcctgagctccgtggtgacagtgcccagctccagcctgggcaccaagacctacacctgcaatgtggatcacaagcccagcaataccaaggtggacaagagggtggagtccaagtacggccctccctgccccccctgtcctgctcctgagttcctgggcggcccttccgtgttcctgttcccccccaagcccaaggataccctgatgatcagccggacccctgaggtgacatgtgtggtggtggatgtgagccaggaggaccctgaggtgcagttcaactggtacgtggatggcgtggaggtgcacaacgccaagaccaagcctcgggaggagcagttcaatagcacctaccgggtggtgagcgtgctgaccgtgctgcaccaggattggctgaacggcaaggagtacaagtgcaaggtgagcaacaagggcctgcccagcagcatcgagaagaccatctccaaggctaagggccagccacgggagcctcaggtgtacaccctgccccctagccaggaggagatgaccaagaaccaggtgagcctgacctgtctggtgaagggcttctacccctccgatatcgctgtggagtgggagtccaacggccagcccgagaacaactataagaccaccccccctgtgctggacagcgacggcagcttcttcctgtattccaggctgaccgtggacaagagccggtggcaggagggcaatgtgttctcctgcagcgtgatgcacgaggccctgcacaaccactacacccagaagtccctgtccctgtccctcggcaag

SEQ ID NO: 407 - DNA, 1338 bp, synthetic construct
  source 1..1338: mol_type = other DNA
caggtgcagctgttggactctgggggaggcttggtcaagcctggagggtccctgagactctcctgtgcagcctctggattcaccttcagtagttatggcatgcactgggtccgccaggctccaggcaaggggctggagtgggtggcatttatatcaaatgatggaagtaataaatactatgcagactccgtgaagggccgattcaccatctccagagacaattccaagaacacgttgtatctgcaaatgaacagcctgagagctgaggacacggctgtgtattactgtgcgagacttctccgtggaccctggaacttcgatctctggggccgtggcaccctggtcaccgtctcatcagcttccaccaagggccccagcgtgttccccctggccccttgttccaggagcacctccgagagcaccgccgctctgggctgcctggtgaaggactacttccctgagcctgtgaccgtgagctggaactccggcgctctgacctccggcgtgcacaccttccccgccgtgctgcagagcagcggcctgtacagcctgagctccgtggtgacagtgcccagctccagcctgggcaccaagacctacacctgcaatgtggatcacaagcccagcaataccaaggtggacaagagggtggagtccaagtacggccctccctgccccccctgtcctgctcctgagttcctgggcggcccttccgtgttcctgttcccccccaagcccaaggataccctgatgatcagccggacccctgaggtgacatgtgtggtggtggatgtgagccaggaggaccctgaggtgcagttcaactggtacgtggatggcgtggaggtgcacaacgccaagaccaagcctcgggaggagcagttcaatagcacctaccgggtggtgagcgtgctgaccgtgctgcaccaggattggctgaacggcaaggagtacaagtgcaaggtgagcaacaagggcctgcccagcagcatcgagaagaccatctccaaggctaagggccagccacgggagcctcaggtgtacaccctgccccctagccaggaggagatgaccaagaaccaggtgagcctgacctgtctggtgaagggcttctacccctccgatatcgctgtggagtgggagtccaacggccagcccgagaacaactataagaccaccccccctgtgctggacagcgacggcagcttcttcctgtattccaggctgaccgtggacaagagccggtggcaggagggcaatgtgttctcctgcagcgtgatgcacgaggccctgcacaaccactacacccagaagtccctgtccctgtccctcggcaag

SEQ ID NO: 408 - DNA, 1335 bp, synthetic construct; identical to SEQ ID NO: 405
  source 1..1335: mol_type = other DNA

SEQ ID NO: 409 - DNA, 1329 bp, synthetic construct
  source 1..1329: mol_type = other DNA
gaggtgcagctgttggagtctgggggaggcctggtcaagcctggggggtccctgagactctcctgtgcagcctctggactcatcttcaaaaactatggcatgaactgggtccgcctggctccggggaaggggctggagtgggttgcatccattagtggtaatagtaactacatctcgtatgcagactcagtgaagggccgattcaccatctccagagacaacgccaacaactcactgtttctgcagatgagcagcctgagagccgacgacacggctgtctattattgttcgagtggttatttctactttgacctctggggcccgggaaccctggtcaccgtctcatcagcttccaccaagggccccagcgtgttccccctggccccttgttccaggagcacctccgagagcaccgccgctctgggctgcctggtgaaggactacttccctgagcctgtgaccgtgagctggaactccggcgctctgacctccggcgtgcacaccttccccgccgtgctgcagagcagcggcctgtacagcctgagctccgtggtgacagtgcccagctccagcctgggcaccaagacctacacctgcaatgtggatcacaagcccagcaataccaaggtggacaagagggtggagtccaagtacggccctccctgccccccctgtcctgctcctgagttcctgggcggcccttccgtgttcctgttcccccccaagcccaaggataccctgatgatcagccggacccctgaggtgacatgtgtggtggtggatgtgagccaggaggaccctgaggtgcagttcaactggtacgtggatggcgtggaggtgcacaacgccaagaccaagcctcgggaggagcagttcaatagcacctaccgggtggtgagcgtgctgaccgtgctgcaccaggattggctgaacggcaaggagtacaagtgcaaggtgagcaacaagggcctgcccagcagcatcgagaagaccatctccaaggctaagggccagccacgggagcctcaggtgtacaccctgccccctagccaggaggagatgaccaagaaccaggtgagcctgacctgtctggtgaagggcttctacccctccgatatcgctgtggagtgggagtccaacggccagcccgagaacaactataagaccaccccccctgtgctggacagcgacggcagcttcttcctgtattccaggctgaccgtggacaagagccggtggcaggagggcaatgtgttctcctgcagcgtgatgcacgaggccctgcacaaccactacacccagaagtccctgtccctgtccctcggcaag

SEQ ID NO: 410 - DNA, 1356 bp, synthetic construct
  source 1..1356: mol_type = other DNA
caggtacagctgcagcagtcgggcccaggactggtgaagccttcacagaccctgtccctcacctgcactgtctctggtggctccatcagcagtggtggttactactggagctggatccgccagcacccagggaagggcctggagtggattgggtacatctattacagtgggagcacctactacaacccgtccctcaagagtcgagttaccatatcagtagacacgtctaagaaccagttctccctgaagctgagctctgtgaccgccgcagacacggctgtgtattactgtgcgagacagaggcgtgccaacgggtatagcagcagctgggaatttgactactggggccagggaaccctggtcaccgtctcatcagcttccaccaagggccccagcgtgttccccctggccccttgttccaggagcacctccgagagcaccgccgctctgggctgcctggtgaaggactacttccctgagcctgtgaccgtgagctggaactccggcgctctgacctccggcgtgcacaccttccccgccgtgctgcagagcagcggcctgtacagcctgagctccgtggtgacagtgcccagctccagcctgggcaccaagacctacacctgcaatgtggatcacaagcccagcaataccaaggtggacaagagggtggagtccaagtacggccctccctgccccccctgtcctgctcctgagttcctgggcggcccttccgtgttcctgttcccccccaagcccaaggataccctgatgatcagccggacccctgaggtgacatgtgtggtggtggatgtgagccaggaggaccctgaggtgcagttcaactggtacgtggatggcgtggaggtgcacaacgccaagaccaagcctcgggaggagcagttcaatagcacctaccgggtggtgagcgtgctgaccgtgctgcaccaggattggctgaacggcaaggagtacaagtgcaaggtgagcaacaagggcctgcccagcagcatcgagaagaccatctccaaggctaagggccagccacgggagcctcaggtgtacaccctgccccctagccaggaggagatgaccaagaaccaggtgagcctgacctgtctggtgaagggcttctacccctccgatatcgctgtggagtgggagtccaacggccagcccgagaacaactataagaccaccccccctgtgctggacagcgacggcagcttcttcctgtattccaggctgaccgtggacaagagccggtggcaggagggcaatgtgttctcctgcagcgtgatgcacgaggccctgcacaaccactacacccagaagtccctgtccctgtccctcggcaag

SEQ ID NO: 411 - DNA, 642 bp, synthetic construct
  source 1..642: mol_type = other DNA
gacattgtgatgacccagtctccatcctccctgtctgcatctgtaggagacagagtcaccatcacttgccgggcaagtcagggcattagcagtgctttagcctggtatcagcagaaaccagggaaagctcctaagctcctgatctatgatgcctccagtttggaaagtggggtcccatcaaggttcagcggcagtggatctgggacagatttcactctcaccatcagcagcctgcagcctgaagattttgcaacttattactgtcaacagtttaatagttacccgctcactttcggcggagggaccaaggtggagatcaaaaggaccgtggctgcccccagcgtgttcatcttccctcctagcgacgagcagctgaagagcggcaccgctagcgtggtgtgtctgctgaataacttctatcccagggaggccaaggtgcagtggaaggtggataacgccctgcagagcggcaactcccaggagtccgtgaccgagcaggactccaaggacagcacctactccctgagctccaccctgaccctgtccaaggctgattatgagaagcacaaggtgtatgcttgcgaggtgacacaccagggcctgtccagccctgtgaccaagagcttcaaccggggcgagtgc

SEQ ID NO: 412 - DNA, 642 bp, synthetic construct
  source 1..642: mol_type = other DNA
gacatccagatgacccagtctccatcctccctgtctgcatctgtaggagacagagtcaccatcacttgccgggcgagtcagggcattcgcaattacttagcctggtatcagcagaaaccagggaaagttcctaggctcctgatctttgctgcatccactttacaatccggggtcccatctcgtttcagtggcagtggatctgggacagatttcactctcaccatcagcagcctgcagcctgaagatgttgcaacttattactgtcaaaagtattacagtgcccccttcactttcggccctgggaccaaagtagatatcaaaaggaccgtggctgcccccagcgtgttcatcttccctcctagcgacgagcagctgaagagcggcaccgctagcgtggtgtgtctgctgaataacttctatcccagggaggccaaggtgcagtggaaggtggataacgccctgcagagcggcaactcccaggagtccgtgaccgagcaggactccaaggacagcacctactccctgagctccaccctgaccctgtccaaggctgattatgagaagcacaaggtgtatgcttgcgaggtgacacaccagggcctgtccagccctgtgaccaagagcttcaaccggggcgagtgc

SEQ ID NO: 413 - DNA, 657 bp, synthetic construct
  source 1..657: mol_type = other DNA
gatattgtgatgactcagtctccactctccctgcccgtcacccttggacagccggcctccatctcctgcaggtctagtcaaagcctcgtacacagtgatggaaacacctacttgaattggtttcagcagaggccaggccaatctccaaggcgcctaatttataaggtttctaaccgggactctggggtcccagacagattcagcggcagtgggtcaggcactgatttcacactgaaaatcagcagggtggaggctgaagatgttggggtttattactgcatgcaaggtacacagtggccggacacttttggccaggggaccaagctggagatcaaaaggaccgtggctgcccccagcgtgttcatcttccctcctagcgacgagcagctgaagagcggcaccgctagcgtggtgtgtctgctgaataacttctatcccagggaggccaaggtgcagtggaaggtggataacgccctgcagagcggcaactcccaggagtccgtgaccgagcaggactccaaggacagcacctactccctgagctccaccctgaccctgtccaaggctgattatgagaagcacaaggtgtatgcttgcgaggtgacacaccagggcctgtccagccctgtgaccaagagcttcaaccggggcgagtgc

SEQ ID NO: 414 - DNA, 648 bp, synthetic construct
  source 1..648: mol_type = other DNA
gaaattgtaatgacacagtctccagccaccctgtctttgtctccaggggaaagagccaccctctcctgcagggccagtcagagtgttagcagctacttagcctggtaccaacagaaacctggccaggctcccaggctcctcatctatgatgcatccaacagggccactggcatcccagccaggttcagtggcagtgggtctgggacagacttcactctcaccatcagcagcctagagcctgaagattttgcagtttattactgtcagcagcgtagcaactggcctccgatgtacacttttggccaggggaccaagctggagatcaaaaggaccgtggctgcccccagcgtgttcatcttccctcctagcgacgagcagctgaagagcggcaccgctagcgtggtgtgtctgctgaataacttctatcccagggaggccaaggtgcagtggaaggtggataacgccctgcagagcggcaactcccaggagtccgtgaccgagcaggactccaaggacagcacctactccctgagctccaccctgaccctgtccaaggctgattatgagaagcacaaggtgtatgcttgcgaggtgacacaccagggcctgtccagccctgtgaccaagagcttcaaccggggcgagtgc

SEQ ID NO: 415 - DNA, 642 bp, synthetic construct
  source 1..642: mol_type = other DNA
gacatccagttgacccagtctccatcttctgtgtctgcatctgtgggggacagagtcaccatcacttgtcgggcgagtcagaatattgagaattggttggcctggtatcaacagaagccagggaaagcccctaaactcctgatctatgcaacatcccgtttggagaatgatgtcccatcaaggttcagcggcagtcggtctgggacagagttcattctcactatcagcagcctacagcctgaggattttgcaacttattattgccatcaggctaatggtttcccgtggacgttcggcccagggaccaaggtggatatcaaaaggaccgtggctgcccccagcgtgttcatcttccctcctagcgacgagcagctgaagagcggcaccgctagcgtggtgtgtctgctgaataacttctatcccagggaggccaaggtgcagtggaaggtggataacgccctgcagagcggcaactcccaggagtccgtgaccgagcaggactccaaggacagcacctactccctgagctccaccctgaccctgtccaaggctgattatgagaagcacaaggtgtatgcttgcgaggtgacacaccagggcctgtccagccctgtgaccaagagcttcaaccggggcgagtgc

SEQ ID NO: 416 - DNA, 663 bp, synthetic construct
  source 1..663: mol_type = other DNA
gatgttgtgatgactcagtctccactctccctgcccgtcacccttggacagccggcctccatctcctgcaggtctagtcaaagcctcgtacacagtgatggaaacacctacttgaattggtttcagcagaggccaggccaatctccaaggcgcctaatttataaggtttctaaccgggactctggggtcccagacagattcagcggcagtgggtcaggcactgatttcacactgaaaatcagcagggtggaggctgaggatgttggggtttattactgcatgcaaggtacacactggcctccgaggtacacttttggccaggggaccaagctggagatcaaaaggaccgtggctgcccccagcgtgttcatcttccctcctagcgacgagcagctgaagagcggcaccgctagcgtggtgtgtctgctgaataacttctatcccagggaggccaaggtgcagtggaaggtggataacgccctgcagagcggcaactcccaggagtccgtgaccgagcaggactccaaggacagcacctactccctgagctccaccctgaccctgtccaaggctgattatgagaagcacaaggtgtatgcttgcgaggtgacacaccagggcctgtccagccctgtgaccaagagcttcaaccggggcgagtgc

SEQ ID NO: 417 - DNA, 642 bp, synthetic construct
  source 1..642: mol_type = other DNA
aacatccagttgacccagtctccatcctcactgtctgcatctgtaggagacagagtcaccatcacttgtcgggcgagtcaggacattagcaattatttagcctggtttcagcagaaaccagggaaagcccctaagtccctgatctatgctgcatccagtttgcaaagtggggtcccatcaaggttcagcggcagttggtctgggacagatttcactctcaccatcagcagcctgcagcctgaagatattgcaacgtattactgccaacagtataagcgttaccctttcatttttggccaggggaccaagctggagatcaaaaggaccgtggctgcccccagcgtgttcatcttccctcctagcgacgagcagctgaagagcggcaccgctagcgtggtgtgtctgctgaataacttctatcccagggaggccaaggtgcagtggaaggtggataacgccctgcagagcggcaactcccaggagtccgtgaccgagcaggactccaaggacagcacctactccctgagctccaccctgaccctgtccaaggctgattatgagaagcacaaggtgtatgcttgcgaggtgacacaccagggcctgtccagccctgtgaccaagagcttcaaccggggcgagtgc

SEQ ID NO: 418 - DNA, 657 bp, synthetic construct
  source 1..657: mol_type = other DNA
gatattgtgatgactcagtctccactctccctgcccgtcacccctggagagccggcctccatctcctgcaggtctagtcagagcctcctgcatagtaatggacgcaactatttggattggtacctgcagaagccagggcagtctccacagctcctgatctatttgggttctaatcgggcctccggggtctctgacaggttcagtgccagtggatcaggcacagattttacactgcaaatcagcagagtggaggctgaggacgttgggatttattactgcatgcaagctctacaaactccgtggacgttcggccaagggaccaaggtggaagtcaaaaggaccgtggctgcccccagcgtgttcatcttccctcctagcgacgagcagctgaagagcggcaccgctagcgtggtgtgtctgctgaataacttctatcccagggaggccaaggtgcagtggaaggtggataacgccctgcagagcggcaactcccaggagtccgtgaccgagcaggactccaaggacagcacctactccctgagctccaccctgaccctgtccaaggctgattatgagaagcacaaggtgtatgcttgcgaggtgacacaccagggcctgtccagccctgtgaccaagagcttcaaccggggcgagtgc

SEQ ID NO: 419 - DNA, 642 bp, synthetic construct
  source 1..642: mol_type = other DNA
gccatccagatgacccagtctccatcctccctgtctgcatctgtaggagacagagtcaccatcacttgccgggcaagtcaggcccttacctatactttagcctggtatcagcagaaaccaggcaaagctcccaggctcctgatccatgatgcctccagtttggaaagtggagtcccttcaaggttcagcggcagtggatctgggacagatttcactctcaccatcaccagcctgcagcctgaagattttgcaacctattactgtcaacagttcaggagttacccgctcactttcggcggagggaccaaggtggagatcaaaaggaccgtggctgcccccagcgtgttcatcttccctcctagcgacgagcagctgaagagcggcaccgctagcgtggtgtgtctgctgaataacttctatcccagggaggccaaggtgcagtggaaggtggataacgccctgcagagcggcaactcccaggagtccgtgaccgagcaggactccaaggacagcacctactccctgagctccaccctgaccctgtccaaggctgattatgagaagcacaaggtgtatgcttgcgaggtgacacaccagggcctgtccagccctgtgaccaagagcttcaaccggggcgagtgc

SEQ ID NO: 420 - DNA, 642 bp, synthetic construct
  source 1..642: mol_type = other DNA
gacatccagatgacccagtctccatcgtccctgtctgcatctgtaggagacagagtcaccatcacttgccgggcaagtcagagcattaacaactatttaaattggtatcaggagaaaccagggaaagcccctaagctcctgatctatgctgcatccagtttgcaaagtggggtcccatcaaggttcagtggcagtggatctgggacagacttcactctcaccatcagcagtctgcaacctgaagattttgcaacttactactgtcaacagagttacagttacccattcactttcggccctgggaccaaagtggatatcaaaaggaccgtggctgcccccagcgtgttcatcttccctcctagcgacgagcagctgaagagcggcaccgctagcgtggtgtgtctgctgaataacttctatcccagggaggccaaggtgcagtggaaggtggataacgccctgcagagcggcaactcccaggagtccgtgaccgagcaggactccaaggacagcacctactccctgagctccaccctgaccctgtccaaggctgattatgagaagcacaaggtgtatgcttgcgaggtgacacaccagggcctgtccagccctgtgaccaagagcttcaaccggggcgagtgc

SEQ ID NO: 421 - DNA, 657 bp, synthetic construct
  source 1..657: mol_type = other DNA
gatattgtgatgactcagtctccactctccctgcccgtcacccttggacagccggcctccatctcctgcaggtctagtcaaagcctcgtaaagagtgatggaaacacctacttgagttggtttcagcagaggccaggccaatctccaaggcgcctaatttataaggtttctaaccgggactctggggtcccagacagattcagcggcagtgggtcaggcactgacttcacactgaaaatcagcagggtggaggctgaggatgttggggtttattactgcatgcaaggtacacactggccacccactttcggccctgggaccaaagtggatatcaaaaggaccgtggctgcccccagcgtgttcatcttccctcctagcgacgagcagctgaagagcggcaccgctagcgtggtgtgtctgctgaataacttctatcccagggaggccaaggtgcagtggaaggtggataacgccctgcagagcggcaactcccaggagtccgtgaccgagcaggactccaaggacagcacctactccctgagctccaccctgaccctgtccaaggctgattatgagaagcacaaggtgtatgcttgcgaggtgacacaccagggcctgtccagccctgtgaccaagagcttcaaccggggcgagtgc

SEQ ID NO: 422 - DNA, 642 bp, synthetic construct
  source 1..642: mol_type = other DNA
aacatccagatgacccagtctccttcctccctgtctgcctctgtgggggacagaatcaccatcacttgccgggcaagtcagagcgtcaatagttatgtgaattggtatcagcagacaccagggcaagcccctaaactcctcatttacgctgcatcgagtgtgcacaatggggtcccagtgaggttcagtggcagtagatctgggacagagttcattctcaccatcagcagtctgcaacctgaagattttgtcacttatttttgtcaacagagtttcactagtccgtggacattcggccaggggaccaaactggaaatgaaaaggaccgtggctgcccccagcgtgttcatcttccctcctagcgacgagcagctgaagagcggcaccgctagcgtggtgtgtctgctgaataacttctatcccagggaggccaaggtgcagtggaaggtggataacgccctgcagagcggcaactcccaggagtccgtgaccgagcaggactccaaggacagcacctactccctgagctccaccctgaccctgtccaaggctgattatgagaagcacaaggtgtatgcttgcgaggtgacacaccagggcctgtccagccctgtgaccaagagcttcaaccggggcgagtgc

SEQ ID NO: 423 - DNA, 642 bp, synthetic construct
  source 1..642: mol_type = other DNA
gaaattgtgttgacacagtctccagccaccctgtctttgtctccaggggaaagagccaccctctcctgcagggccagccagagtattgcccgccgcatagcctggtaccaacagcaacctggccaggctcccaggctcctcatctatgatgcatccaacagggccactggcatcccagccaggttcagtggcagtgggtctgggacagacttcactctcaccatcagcagcctagagcctgaagattttgcaatttattactgtcaacaacgtgccaactggcctctcactttcggccctgggaccaaagtggatatcaaaaggaccgtggctgcccccagcgtgttcatcttccctcctagcgacgagcagctgaagagcggcaccgctagcgtggtgtgtctgctgaataacttctatcccagggaggccaaggtgcagtggaaggtggataacgccctgcagagcggcaactcccaggagtccgtgaccgagcaggactccaaggacagcacctactccctgagctccaccctgaccctgtccaaggctgattatgagaagcacaaggtgtatgcttgcgaggtgacacaccagggcctgtccagccctgtgaccaagagcttcaaccggggcgagtgc

SEQ ID NO: 424 - DNA, 642 bp, synthetic construct
  source 1..642: mol_type = other DNA
gccatccagttgacccagtctccatcctcgctgtctgcatcggtcggagacagagtcaccatcacttgccgggccagtcagggcattagcagttatttagcctggtatcagcaaaaaccagggaaagcccctaagctcctaatctttgctgcatcgcttttacaaaggggggtcccatcaaggttcagcggcagtggatttgggacagatttcactctcaccatcagcggcctgcagcctgaagattttgcgacttatttctgtcaacagtttaatacttacccgatcactttcggcggggggaccaaggtggagatcaaaaggaccgtggctgcccccagcgtgttcatcttccctcctagcgacgagcagctgaagagcggcaccgctagcgtggtgtgtctgctgaataacttctatcccagggaggccaaggtgcagtggaaggtggataacgccctgcagagcggcaactcccaggagtccgtgaccgagcaggactccaaggacagcacctactccctgagctccaccctgaccctgtccaaggctgattatgagaagcacaaggtgtatgcttgcgaggtgacacaccagggcctgtccagccctgtgaccaagagcttcaaccggggcgagtgc

SEQ ID NO: 425 - DNA, 648 bp, synthetic construct
  source 1..648: mol_type = other DNA
gaaattgtgatgacgcagtctccaggcaccctgtctttgtctccaggggaaagagccaccctctcctgcagggccagtcagagtgttagcagcagctacttagcctggtaccagcagaaacctggccaggctcccaggctcctcatctatggtgcatccagcagggccactggcatcccagacaggttcagtggcagtgggtctgggacagacttcactctcaccatcagcagactggagcctgaagattttgcagtgtattactgtcagcagtatggtagctcacctccgatcaccttcggccaagggacacgactggagattaaaaggaccgtggctgcccccagcgtgttcatcttccctcctagcgacgagcagctgaagagcggcaccgctagcgtggtgtgtctgctgaataacttctatcccagggaggccaaggtgcagtggaaggtggataacgccctgcagagcggcaactcccaggagtccgtgaccgagcaggactccaaggacagcacctactccctgagctccaccctgaccctgtccaaggctgattatgagaagcacaaggtgtatgcttgcgaggtgacacaccagggcctgtccagccctgtgaccaagagcttcaaccggggcgagtgc

SEQ ID NO: 426 - DNA, 642 bp, synthetic construct
  source 1..642: mol_type = other DNA
aacatccagatgacccagtctccatcctccctgactgcatctgtaggagacagaatcaccatcacttgccgggcgagtcagggcattcgaaactctttagcctggtatcagcagaaaccagggacagcccctaagctcctggtctctgctgcatccaagttacaaactggggtcccttccaggttcagtggcagcggatctgggacggattacactctcaccatcagcagcctgcagactgaagattttgcaacttattactgtcaacaatattacggaacccctcccacttttggccaggggaccaagctggagatcaaaaggaccgtggctgcccccagcgtgttcatcttccctcctagcgacgagcagctgaagagcggcaccgctagcgtggtgtgtctgctgaataacttctatcccagggaggccaaggtgcagtggaaggtggataacgccctgcagagcggcaactcccaggagtccgtgaccgagcaggactccaaggacagcacctactccctgagctccaccctgaccctgtccaaggctgattatgagaagcacaaggtgtatgcttgcgaggtgacacaccagggcctgtccagccctgtgaccaagagcttcaaccggggcgagtgc

SEQ ID NO: 427 - DNA, 642 bp, synthetic construct
  source 1..642: mol_type = other DNA
gaaattgtgttgacacagtctccagccaccctgtctttgtctccaggggaaagagccaccctctcctgcagggccagtcagggtattagcagctacttagcctggtaccaacagaaacctggccaggctcccagactcctcatttatgatgcatccaatagggccactggcatcccagccaggttcagtggcagtgggtctgggacagacttcactctcaccatcagcaacctagagcctgaagattttgcagtttattactgtcagcagcgtaaaaactggcctctcactttcggcggagggtccaaggtggagatcaaaaggaccgtggctgcccccagcgtgttcatcttccctcctagcgacgagcagctgaagagcggcaccgctagcgtggtgtgtctgctgaataacttctatcccagggaggccaaggtgcagtggaaggtggataacgccctgcagagcggcaactcccaggagtccgtgaccgagcaggactccaaggacagcacctactccctgagctccaccctgaccctgtccaaggctgattatgagaagcacaaggtgtatgcttgcgaggtgacacaccagggcctgtccagccctgtgaccaagagcttcaaccggggcgagtgc

SEQ ID NO: 428 - DNA, 648 bp, synthetic construct
  source 1..648: mol_type = other DNA
gaaattgtgttgacacagtctccagccaccctgtctttgtctccaggggaaagagccaccctctcctgcagggccagtcagagtgttagcagctacttagcctggtaccaacagaaacctggccaggctcccaggctcctcatctatgatgcatccaacagggccactggcatcccagccaggttcagtggcagtgggtctgggacagacttcactctcaccatcagcagcctagagcctgaagattttgcagtttattactgtcagcagcgtagcaactggcctccggagctcactttcggcggagggaccaaggtggagatcaaaaggaccgtggctgcccccagcgtgttcatcttccctcctagcgacgagcagctgaagagcggcaccgctagcgtggtgtgtctgctgaataacttctatcccagggaggccaaggtgcagtggaaggtggataacgccctgcagagcggcaactcccaggagtccgtgaccgagcaggactccaaggacagcacctactccctgagctccaccctgaccctgtccaaggctgattatgagaagcacaaggtgtatgcttgcgaggtgacacaccagggcctgtccagccctgtgaccaagagcttcaaccggggcgagtgc

SEQ ID NO: 429 - DNA, 642 bp, synthetic construct
  source 1..642: mol_type = other DNA
gaaattgtgatgacacagtctccagccaccctgtctttgtctccaggggaaagagccaccctctcctgcagggccagtcagagtgttagcaactacttagcctggtaccagcagaaacctggccaggctcccaggctcctcatctatggtgcatccagcagggccactggcatcccagacaggttcagtggcagtgggtctgggacagacttcactctcaccatcagcagactggagcctgaagattttgcagtgtattactgtcagcagtatggtagctcactttggacgttcggccaagggaccaaggtggaaatcaaaaggaccgtggctgcccccagcgtgttcatcttccctcctagcgacgagcagctgaagagcggcaccgctagcgtggtgtgtctgctgaataacttctatcccagggaggccaaggtgcagtggaaggtggataacgccctgcagagcggcaactcccaggagtccgtgaccgagcaggactccaaggacagcacctactccctgagctccaccctgaccctgtccaaggctgattatgagaagcacaaggtgtatgcttgcgaggtgacacaccagggcctgtccagccctgtgaccaagagcttcaaccggggcgagtgc

SEQ ID NO: 430 - DNA, 642 bp, synthetic construct
  source 1..642: mol_type = other DNA
gacatccagatgacccagtctccctcctccctgcctgcatctgtgggagacagagtcaccatcacttgccgggccagtcagggcattggcacttttttagcctggtatcagcaacacttggggaaagcccctaaactcctgatctctgctagttccactgttcagcgtggggtcccatccaggttcagcggcagtggatctgggacagagttcactctcaccatcaacagcctgcagcctgaagattttgcaacttattactgtcagcagcttaataattaccctcggacgttcggccaagggaccaaagtggaaatcaagaggaccgtggctgcccccagcgtgttcatcttccctcctagcgacgagcagctgaagagcggcaccgctagcgtggtgtgtctgctgaataacttctatcccagggaggccaaggtgcagtggaaggtggataacgccctgcagagcggcaactcccaggagtccgtgaccgagcaggactccaaggacagcacctactccctgagctccaccctgaccctgtccaaggctgattatgagaagcacaaggtgtatgcttgcgaggtgacacaccagggcctgtccagccctgtgaccaagagcttcaaccggggcgagtgc

SEQ ID NO: 431 - DNA, 642 bp, synthetic construct
  source 1..642: mol_type = other DNA
gaaattgtgatgacgcagtctccaggcaccctgtctttgtctccagggcaaagagccaccctctcctgcagggccagtcagagtgttagcagcagctccttagcctggtatcaacagaaacctggccaggctcccaggctcctcatccacggtgcctccagcagggccactggtatcccagacaggttcagtggcagtgggtctgggacagacttcactctcaccatcagcagactggagcctgaagattttgcagtgtattactgtcagcagtatggtacctcgtggacgttcggccaagggaccaaggtggaaatcaaaaggaccgtggctgcccccagcgtgttcatcttccctcctagcgacgagcagctgaagagcggcaccgctagcgtggtgtgtctgctgaataacttctatcccagggaggccaaggtgcagtggaaggtggataacgccctgcagagcggcaactcccaggagtccgtgaccgagcaggactccaaggacagcacctactccctgagctccaccctgaccctgtccaaggctgattatgagaagcacaaggtgtatgcttgcgaggtgacacaccagggcctgtccagccctgtgaccaagagcttcaaccggggcgagtgc

SEQ ID NO: 432 - DNA, 657 bp, synthetic construct
  source 1..657: mol_type = other DNA
gatgttgtgatgactcagtctccactctccctgcccgtcacccctggagagccggcctccatctcctgcaggtctagtcagagcctcctgcataggagtggatacaactatttggattggtacgtgcagaagccagggcagtctccacagctcctgatctatttggggtctattcgagcggtcggggtccccgacaggttcagtggcagcgcatcaggcacagattttacactgagaatcagcagagtggaggctgaggatgttgggatttattactgcatgcaagctctacaaactcctccggctttcggcggggggaccaaggtggagatcaaaaggaccgtggctgcccccagcgtgttcatcttccctcctagcgacgagcagctgaagagcggcaccgctagcgtggtgtgtctgctgaataacttctatcccagggaggccaaggtgcagtggaaggtggataacgccctgcagagcggcaactcccaggagtccgtgaccgagcaggactccaaggacagcacctactccctgagctccaccctgaccctgtccaaggctgattatgagaagcacaaggtgtatgcttgcgaggtgacacaccagggcctgtccagccctgtgaccaagagcttcaaccggggcgagtgc

SEQ ID NO: 433 - DNA, 642 bp, synthetic construct
  source 1..642: mol_type = other DNA
aacatccagttgacccagtctccatcctccctgtctgcatctgtaggagacagagtcaccatcacttgtcgggcgagtcagggtattaacagctggttagcctggtatcagcagaaaccagggaaagcccctaagctccttatctatgctgcatccactttgcaaagtggggtcccatcaagattcagcggcagtggatctgggacagatttcactctcaccatcaacagcctgcagcctgaggattttgcaacttattattgtcagcagcttaacagtttcccattcacttttggccctgggaccaaagtgcatatcaaaaggaccgtggctgcccccagcgtgttcatcttccctcctagcgacgagcagctgaagagcggcaccgctagcgtggtgtgtctgctgaataacttctatcccagggaggccaaggtgcagtggaaggtggataacgccctgcagagcggcaactcccaggagtccgtgaccgagcaggactccaaggacagcacctactccctgagctccaccctgaccctgtccaaggctgattatgagaagcacaaggtgtatgcttgcgaggtgacacaccagggcctgtccagccctgtgaccaagagcttcaaccggggcgagtgc

SEQ ID NO: 434 - DNA, 642 bp, synthetic construct
  source 1..642: mol_type = other DNA
gacatccagttgacccagtctccatcttccctgtctgcatctgtaggagacagagtcaccatcacttgccgggcaagtcagagcattgacgaccatttaaactggtatcagcaaaagccagggaaagtccccaagctcctcataagtagtgcatcgacattgcagagtggggccccatcgaggttcagtggcagtggatatgggacagatttcaccctcaccatcagcagtctgcaagtcgaagattttgcaacttactactgtcaacagagttacagtccccctcagacgttcggccaggggaccaaggtggaaatcaagaggaccgtggctgcccccagcgtgttcatcttccctcctagcgacgagcagctgaagagcggcaccgctagcgtggtgtgtctgctgaataacttctatcccagggaggccaaggtgcagtggaaggtggataacgccctgcagagcggcaactcccaggagtccgtgaccgagcaggactccaaggacagcacctactccctgagctccaccctgaccctgtccaaggctgattatgagaagcacaaggtgtatgcttgcgaggtgacacaccagggcctgtccagccctgtgaccaagagcttcaaccggggcgagtgc

SEQ ID NO: 435 - DNA, 642 bp, synthetic construct
  source 1..642: mol_type = other DNA
gacatccagttgacccagtctccatcctccctgtctgcatctgtaggagacagagtcaccatcacttgccgggcaagtcagagcattagcagctatttaaattggtatcagcagaaaccagggaaagcccctaagctcctgatctatgctgcatccagtttgcaaagtggggtcccatcaaggttcagtggcagtggatctgggacagatttcactctcaccatcagcagtctgcaacctgaagattttgcaacttactactgtcaacagagttacagtacccctcggaccttcggccaagggacacgactggagattaaaaggaccgtggctgcccccagcgtgttcatcttccctcctagcgacgagcagctgaagagcggcaccgctagcgtggtgtgtctgctgaataacttctatcccagggaggccaaggtgcagtggaaggtggataacgccctgcagagcggcaactcccaggagtccgtgaccgagcaggactccaaggacagcacctactccctgagctccaccctgaccctgtccaaggctgattatgagaagcacaaggtgtatgcttgcgaggtgacacaccagggcctgtccagccctgtgaccaagagcttcaaccggggcgagtgc

SEQ ID NO: 436 - DNA, 657 bp, synthetic construct
  source 1..657: mol_type = other DNA
gatgttgtgatgactcagtctccactctccctgcccgtcacccttggacagccggcctccatctcctgcaggtctagtcaaagcctcgtatacagtgatggaaacacctacttgaattggtttcagcagaggccaggccaatctccaaggcgcctaatttataaggtttctaaccgggactctggggtcccagacagattcagcggcagtgggtcaggcactgatttcacactgaaaatcagcagggtggaggctgaggatgttggggtttattactgcatgcaaggtacacactggcctcccacttttggccaggggaccaagctggagatcaaaaggaccgtggctgcccccagcgtgttcatcttccctcctagcgacgagcagctgaagagcggcaccgctagcgtggtgtgtctgctgaataacttctatcccagggaggccaaggtgcagtggaaggtggataacgccctgcagagcggcaactcccaggagtccgtgaccgagcaggactccaaggacagcacctactccctgagctccaccctgaccctgtccaaggctgattatgagaagcacaaggtgtatgcttgcgaggtgacacaccagggcctgtccagccctgtgaccaagagcttcaaccggggcgagtgc

SEQ ID NO: 437 - DNA, 642 bp, synthetic construct
  source 1..642: mol_type = other DNA
gacatccagatgacccagtctccctctatcctgtctgcatctgtaggagacagagtcaccctcacttgccgggccagtcaaagtattagttcctggttggcctggtatcaacagacaccaggaaaagcccctagggtcctgatttatgaggcgtcaactttagaggttggggtcccatcaaggttcagcggcagtggatctgggacagacttcactctcaccatcagcagcctgcagcctgaagattttggaacttacttctgccaacaataccatactgattcgaggacttttggacaggggaccatcctagagatcaaaaggaccgtggctgcccccagcgtgttcatcttccctcctagcgacgagcagctgaagagcggcaccgctagcgtggtgtgtctgctgaataacttctatcccagggaggccaaggtgcagtggaaggtggataacgccctgcagagcggcaactcccaggagtccgtgaccgagcaggactccaaggacagcacctactccctgagctccaccctgaccctgtccaaggctgattatgagaagcacaaggtgtatgcttgcgaggtgacacaccagggcctgtccagccctgtgaccaagagcttcaaccggggcgagtgc

SEQ ID NO: 438 - DNA, 639 bp, synthetic construct
  source 1..639: mol_type = other DNA
gacatcgtgatgacccagtctccatcctccctgtctgcatctgtaggagacagagtcaccatcacttgccgggcaagtcagagcattagcagctatttaaattggtatcagcagaaaccagggaaagcccctaagctcctgatctatgctgcatccagtttgcaaagtggggtcccatcaaggttcagtggcagtggatctgggacagatttcactctcaccatcagcagtctgcaacctgaagattttgcaacttactactgtcaacagagttacagtaccctcactttcggcggagggaccaaggtggagatcaaaaggaccgtggctgcccccagcgtgttcatcttccctcctagcgacgagcagctgaagagcggcaccgctagcgtggtgtgtctgctgaataacttctatcccagggaggccaaggtgcagtggaaggtggataacgccctgcagagcggcaactcccaggagtccgtgaccgagcaggactccaaggacagcacctactccctgagctccaccctgaccctgtccaaggctgattatgagaagcacaaggtgtatgcttgcgaggtgacacaccagggcctgtccagccctgtgaccaagagcttcaaccggggcgagtgc

SEQ ID NO: 439 - DNA, 642 bp, synthetic construct
  source 1..642: mol_type = other DNA
gaaattgtattgacacagtctccaggcaccctgtctttgtctccaggggaaagagccaccctctcctgcagggccagtcagagtgttagcaagtacctagcctggtaccaacagaaacctggccaggctcccaggctccttatctatgatgtttccaacagggccactggcatcccagccagattcagtggcagtgggtctgggacagacttcactctcaccatcagcagcctagagcctgaagattttgcagtttattactgtcagcagcggcgcagctggcctctcactttcggcggagggaccaaggtggagatcagaaggaccgtggctgcccccagcgtgttcatcttccctcctagcgacgagcagctgaagagcggcaccgctagcgtggtgtgtctgctgaataacttctatcccagggaggccaaggtgcagtggaaggtggataacgccctgcagagcggcaactcccaggagtccgtgaccgagcaggactccaaggacagcacctactccctgagctccaccctgaccctgtccaaggctgattatgagaagcacaaggtgtatgcttgcgaggtgacacaccagggcctgtccagccctgtgaccaagagcttcaaccggggcgagtgc

SEQ ID NO: 440 - DNA, 642 bp, synthetic construct
  source 1..642: mol_type = other DNA
aacatccagttgacccagtctccatcttctgtgtctgcatctgtaggagacagagtcaccatctcttgtcgggcgagtcagggtattggcagatggttagcctggtatcagcagaaaccagggaaagcccctaaactcctgatctatgctgcatccaatttgcaaagtggggtcccatcaaggttcagtggcagtggatctgggacagatttcactctcaccatcagcagcctgcagcctgaagatttcgcaacttactattgtcaacaggctaacagtttccctcgtactttcggccctgggaccaaagtggatatcaaaaggaccgtggctgcccccagcgtgttcatcttccctcctagcgacgagcagctgaagagcggcaccgctagcgtggtgtgtctgctgaataacttctatcccagggaggccaaggtgcagtggaaggtggataacgccctgcagagcggcaactcccaggagtccgtgaccgagcaggactccaaggacagcacctactccctgagctccaccctgaccctgtccaaggctgattatgagaagcacaaggtgtatgcttgcgaggtgacacaccagggcctgtccagccctgtgaccaagagcttcaaccggggcgagtgc

SEQ ID NO: 441 - DNA, 642 bp, synthetic construct
  source 1..642: mol_type = other DNA
aacatccagttgacccagtctccatcctccctgtctgcatctgtaggagacagagtcaccatcacttgtcgggccagtcagggcattagcacttatttagcctggtatcagcaaaaaccagggttggcccctaagctcctgatctatggtgcatccactttgcaaagtggggtcccatcaaaattcagcggctttggatctgggagagatttcactctcaccatcagcagcctgcagcctgaagatattgcaacttactactgtcaacaacttaatacttatcctcccacttttggccaggggaccaagctggagatcaaaaggaccgtggctgcccccagcgtgttcatcttccctcctagcgacgagcagctgaagagcggcaccgctagcgtggtgtgtctgctgaataacttctatcccagggaggccaaggtgcagtggaaggtggataacgccctgcagagcggcaactcccaggagtccgtgaccgagcaggactccaaggacagcacctactccctgagctccaccctgaccctgtccaaggctgattatgagaagcacaaggtgtatgcttgcgaggtgacacaccagggcctgtccagccctgtgaccaagagcttcaaccggggcgagtgc

SEQ ID NO: 442 - DNA, 642 bp, synthetic construct
  source 1..642: mol_type = other DNA
gacattgtgatgacccagtctccatcctccctgtctgcatctgtaggagacagagtcaccatcacttgccaggcgagtcaggacattagcaactatttaaattggtatcagcagaaaccagggaaagcccctaagctcctgatctacgatgcatccagtttggaaagcggggtcccatcaaagttcagcggcagtagatctgggacagatttcactctcaccatcagcagcctgcagcctgaagattctgcaacttattactgccaacagtataggagttacccgatcactttcggcggagggaccaaggtggagatcaaaaggaccgtggctgcccccagcgtgttcatcttccctcctagcgacgagcagctgaagagcggcaccgctagcgtggtgtgtctgctgaataacttctatcccagggaggccaaggtgcagtggaaggtggataacgccctgcagagcggcaactcccaggagtccgtgaccgagcaggactccaaggacagcacctactccctgagctccaccctgaccctgtccaaggctgattatgagaagcacaaggtgtatgcttgcgaggtgacacaccagggcctgtccagccctgtgaccaagagcttcaaccggggcgagtgc

SEQ ID NO: 443 - DNA, 642 bp, synthetic construct
  source 1..642: mol_type = other DNA
gacatccagttgacccagtctccatcctccctgtctgcatctataggagacagagtcaccatcacttgccgggccagtcagggcattagcagttttttagcctggtatcagcaaaaaccagggaaagccccacagctcctgatctatgctgcgtccactttgcaaagtggggtcccatcaaggttcagcggcagtgggtctgggacagaattcactctcacaatcagcagcctgcagcctgaagattttgcaacttattactgtcaacaatttaaaatttatcctctcactttcggcggagggaccaaggtggaggtcaaaaggaccgtggctgcccccagcgtgttcatcttccctcctagcgacgagcagctgaagagcggcaccgctagcgtggtgtgtctgctgaataacttctatcccagggaggccaaggtgcagtggaaggtggataacgccctgcagagcggcaactcccaggagtccgtgaccgagcaggactccaaggacagcacctactccctgagctccaccctgaccctgtccaaggctgattatgagaagcacaaggtgtatgcttgcgaggtgacacaccagggcctgtccagccctgtgaccaagagcttcaaccggggcgagtgc

SEQ ID NO: 444 - DNA, 648 bp, synthetic construct
  source 1..648: mol_type = other DNA
gaaatagtgatgacgcagtctccaggcaccctgtctttgtctccaggggaaagagccaccctctcctgcagggccagtcagagtgttagcagcagctacttagcctggtaccagcagaaacctggccaggctcccaggctcctcatctatggtgcatccagcagggccactggcatcccagacaggttcagtggcagtgggtctgggacagacttcactctcaccatcagcagactggagcctgaagattttgcagtgtattactgtcagcagtatggtagctcacctccgatcaccttcggccaagggacacgactggagattaaaaggaccgtggctgcccccagcgtgttcatcttccctcctagcgacgagcagctgaagagcggcaccgctagcgtggtgtgtctgctgaataacttctatcccagggaggccaaggtgcagtggaaggtggataacgccctgcagagcggcaactcccaggagtccgtgaccgagcaggactccaaggacagcacctactccctgagctccaccctgaccctgtccaaggctgattatgagaagcacaaggtgtatgcttgcgaggtgacacaccagggcctgtccagccctgtgaccaagagcttcaaccggggcgagtgc

SEQ ID NO: 445 - DNA, 642 bp, synthetic construct
  source 1..642: mol_type = other DNA
gacatccagttgacccagtctccatccttcctgtctgcatctgttggagacagagtcactatcacttgccgggccagtcagggcattagtagtcagttagcctggtatcaacaagagccagggaaagcccctaagctcctgatctatgctgcatccactttgcaaagtggggtcccatcaaggttcagcggcagtgggtctgggacagagtttactctcacaatcagcagcctgcagcctgaagattttgcaacttattactgtcaacaggtcaatgcttaccctctcactttcggccctgggaccaaagtggatatcaaaaggaccgtggctgcccccagcgtgttcatcttccctcctagcgacgagcagctgaagagcggcaccgctagcgtggtgtgtctgctgaataacttctatcccagggaggccaaggtgcagtggaaggtggataacgccctgcagagcggcaactcccaggagtccgtgaccgagcaggactccaaggacagcacctactccctgagctccaccctgaccctgtccaaggctgattatgagaagcacaaggtgtatgcttgcgaggtgacacaccagggcctgtccagccctgtgaccaagagcttcaaccggggcgagtgc